European Patent Application EP 4 481 049 A2, published December 25, 2024. Title: VARIANTS OF CPF1 (CAS12A) WITH ALTERED PAM SPECIFICITY. Applicant: The General Hospital Corporation. Application WO PCT/US2018/028919, filed April 23, 2018. The sequence listing filed with the application follows.

SEQUENCE LISTING (586 sequences)

SEQ ID NO: 1 - DNA, 27 bp, synthetic construct
  misc_feature 1..27: note = Description of Artificial Sequence: Synthetic oligonucleotide
  modified_base 4: mod_base = OTHER; note = a, c, t, g, unknown or other
  modified_base 25: mod_base = OTHER; note = a, c, t, g, unknown or other
  source 1..27: mol_type = other DNA
tttngacctaccgctcgaatagcgngg

SEQ ID NO: 2 - protein, 1307 aa, Acidaminococcus sp.
MTQFEGFTNLYQVSKTLRFELIPQGKTLKHIQEQGFIEEDKARNDHYKELKPIIDRIYKTYADQCLQLVQLDWENLSAAIDSYRKEKTEETRNALIEEQATYRNAIHDYFIGRTDNLTDAINKRHAEIYKGLFKAELFNGKVLKQLGTVTTTEHENALLRSFDKFTTYFSGFYENRKNVFSAEDISTAIPHRIVQDNFPKFKENCHIFTRLITAVPSLREHFENVKKAIGIFVSTSIEEVFSFPFYNQLLTQTQIDLYNQLLGGISREAGTEKIKGLNEVLNLAIQKNDETAHIIASLPHRFIPLFKQILSDRNTLSFILEEFKSDEEVIQSFCKYKTLLRNENVLETAEALFNELNSIDLTHIFISHKKLETISSALCDHWDTLRNALYERRISELTGKITKSAKEKVQRSLKHEDINLQEIISAAGKELSEAFKQKTSEILSHAHAALDQPLPTTLKKQEEKEILKSQLDSLLGLYHLLDWFAVDESNEVDPEFSARLTGIKLEMEPSLSFYNKARNYATKKPYSVEKFKLNFQMPTLASGWDVNKEKNNGAILFVKNGLYYLGIMPKQKGRYKALSFEPTEKTSEGFDKMYYDYFPDAAKMIPKCSTQLKAVTAHFQTHTTPILLSNNFIEPLEITKEIYDLNNPEKEPKKFQTAYAKKTGDQKGYREALCKWIDFTRDFLSKYTKTTSIDLSSLRPSSQYKDLGEYYAELNPLLYHISFQRIAEKEIMDAVETGKLYLFQIYNKDFAKGHHGKPNLHTLYWTGLFSPENLAKTSIKLNGQAELFYRPKSRMKRMAHRLGEKMLNKKLKDQKTPIPDTLYQELYDYVNHRLSHDLSDEARALLPNVITKEVSHEIIKDRRFTSDKFFFHVPITLNYQAANSPSKFNQRVNAYLKEHPETPIIGIDRGERNLIYITVIDSTGKILEQRSLNTIQQFDYQKKLDNREKERVAARQAWSVVGTIKDLKQGYLSQVIHEIVDLMIHYQAVVVLENLNFGFKSKRTGIAEKAVYQQFEKMLIDKLNCLVLKDYPAEKVGGVLNPYQLTDQFTSFAKMGTQSGFLFYVPAPYTSKIDPLTGFVDPFVWKTIKNHESRKHFLEGFDFLHYDVKTGDFILHFKMNRNLSFQRGLPGFMPAWDIVFEKNETQFDAKGTPFIAGKRIVPVIENHRFTGRYRDLYPANELIALLEEKGIVFRDGSNILPKLLENDDSHAIDTMVALIRSVLQMRNSNAATGEDYINSPVRDLNGVCFDSRFQNPEWPMDADANGAYHIALKGQLLLNHLKESKDLKLQNGISNQDWLAYIQELRN

SEQ ID NO: 3 - protein, 1246 aa, Lachnospiraceae bacterium
MLKNVGIDRLDVEKGRKNMSKLEKFTNCYSLSKTLRFKAIPVGKTQENIDNKRLLVEDEKRAEDYKGVKKLLDRYYLSFINDVLHSIKLKNLNNYISLFRKKTRTEKENKELENLEINLRKEIAKAFKGNEGYKSLFKKDIIETILPEFLDDKDEIALVNSFNGFTTAFTGFFDNRENMFSEEAKSTSIAFRCINENLTRYISNMDIFEKVDAIFDKHEVQEIKEKILNSDYDVEDFFEGEFFNFVLTQEGIDVYNAIIGGFVTESGEKIKGLNEYINLYNQKTKQKLPKFKPLYKQVLSDRESLSFYGEGYTSDEEVLEVFRNTLNKNSEIFSSIKKLEKLFKNFDEYSSAGIFVKNGPAISTISKDIFGEWNVIRDKWNAEYDDIHLKKKAVVTEKYEDDRRKSFKKIGSFSLEQLQEYADADLSVVEKLKEIIIQKVDEIYKVYGSSEKLFDADFVLEKSLKKNDAVVAIMKDLLDSVKSFENYIKAFFGEGKETNRDESFYGDFVLAYDILLKVDHIYDAIRNYVTQKPYSKDKFKLYFQNPQFMGGWDKDKETDYRATILRYGSKYYLAIMDKKYAKCLQKIDKDDVNGNYEKINYKLLPGPNKMLPKVFFSKKWMAYYNPSEDIQKIYKNGTFKKGDMFNLNDCHKLIDFFKDSISRYPKWSNAYDFNFSETEKYKDIAGFYREVEEQGYKVSFESASKKEVDKLVEEGKLYMFQIYNKDFSDKSHGTPNLHTMYFKLLFDENNHGQIRLSGGAELFMRRASLKKEELVVHPANSPIANKNPDNPKKTTTLSYDVYKDKRFSEDQYELHIPIAINKCPKNIFKINTEVRVLLKHDDNPYVIGIDRGERNLLYIVVVDGKGNIVEQYSLNEIINNFNGIRIKTDYHSLLDKKEKERFEARQNWTSIENIKELKAGYISQVVHKICELVEKYDAVIALEDLNSGFKNSRVKVEKQVYQKFEKMLIDKLNYMVDKKSNPCATGGALKGYQITNKFESFKSMSTQNGFIFYIPAWLTSKIDPSTGFVNLLKTKYTSIADSKKFISSFDRIMYVPEEDLFEFALDYKNFSRTDADYIKKWKLYSYGNRIRIFRNPKKNNVFDWEEVCLTSAYKELFNKYGINYQQGDIRALLCEQSDKAFYSSFMALMSLMLQMRNSITGRTDVDFLISPVKNSDGIFYDSRNYEAQENAILPKNADANGAYNIARKVLWAIGQFKKAEDEKLDKVKIAISNKEWLEYAQTSVKH

SEQ ID NO: 4 - protein, 1300 aa, Francisella tularensis
MSIYQEFVNKYSLSKTLRFELIPQGKTLENIKARGLILDDEKRAKDYKKAKQIIDKYHQFFIEEILSSVCISEDLLQNYSDVYFKLKKSDDDNLQKDFKSAKDTIKKQISEYIKDSEKFKNLFNQNLIDAKKGQESDLILWLKQSKDNGIELFKANSDITDIDEALEIIKSFKGWTTYFKGFHENRKNVYSSNDIPTSIIYRIVDDNLPKFLENKAKYESLKDKAPEAINYEQIKKDLAEELTFDIDYKTSEVNQRVFSLDEVFEIANFNNYLNQSGITKFNTIIGGKFVNGENTKRKGINEYINLYSQQINDKTLKKYKMSVLFKQILSDTESKSFVIDKLEDDSDVVTTMQSFYEQIAAFKTVEEKSIKETLSLLFDDLKAQKLDLSKIYFKNDKSLTDLSQQVFDDYSVIGTAVLEYITQQIAPKNLDNPSKKEQELIAKKTEKAKYLSLETIKLALEEFNKHRDIDKQCRFEEILANFAAIPMIFDEIAQNKDNLAQISIKYQNQGKKDLLQASAEDDVKAIKDLLDQTNNLLHKLKIFHISQSEDKANILDKDEHFYLVFEECYFELANIVPLYNKIRNYITQKPYSDEKFKLNFENSTLANGWDKNKEPDNTAILFIKDDKYYLGVMNKKNNKIFDDKAIKENKGEGYKKIVYKLLPGANKMLPKVFFSAKSIKFYNPSEDILRIRNHSTHTKNGSPQKGYEKFEFNIEDCRKFIDFYKQSISKHPEWKDFGFRFSDTQRYNSIDEFYREVENQGYKLTFENISESYIDSVVNQGKLYLFQIYNKDFSAYSKGRPNLHTLYWKALFDERNLQDVVYKLNGEAELFYRKQSIPKKITHPAKEAIANKNKDNPKKESVFEYDLIKDKRFTEDKFFFHCPITINFKSSGANKFNDEINLLLKEKANDVHILSIDRGERHLAYYTLVDGKGNIIKQDTFNIIGNDRMKTNYHDKLAAIEKDRDSARKDWKKINNIKEMKEGYLSQVVHEIAKLVIEYNAIVVFEDLNFGFKRGRFKVEKQVYQKLEKMLIEKLNYLVFKDNEFDKTGGVLRAYQLTAPFETFKKMGKQTGIIYYVPAGFTSKICPVTGFVNQLYPKYESVSKSQEFFSKFDKICYNLDKGYFEFSFDYKNFGDKAAKGKWTIASFGSRLINFRNSDKNHNWDTREVYPTKELEKLLKDYSIEYGHGECIKAAICGESDKKFFAKLTSVLNTILQMRNSKTGTELDYLISPVADVNGNFFDSRQAPKNMPQDADANGAYHIGLKGLMLLGRIKNNQEGKKLNLVIKNEEYFEFVQNRNN

SEQ ID NO: 5 - DNA, 81 bp, synthetic construct
  misc_feature 1..81: note = Description of Artificial Sequence: Synthetic oligonucleotide
  source 1..81: mol_type = other DNA
tacccatacgatgttccagattacgcttatccctacgacgtgcctgattatgcatacccatatgatgtccccgactatgcc

SEQ ID NO: 6 - DNA, 4059 bp, synthetic construct
  misc_feature 1..4059: note = Description of Artificial Sequence: Synthetic polynucleotide
  source 1..4059: mol_type = other DNA
atgacacagttcgagggctttaccaacctgtatcaggtgagcaagacactgcggtttgagctgatcccacagggcaagaccctgaagcacatccaggagcagggcttcatcgaggaggacaaggcccgcaatgatcactacaaggagctgaagcccatcatcgatcggatctacaagacctatgccgaccagtgcctgcagctggtgcagctggattgggagaacctgagcgccgccatcgactcctatagaaaggagaaaaccgaggagacaaggaacgccctgatcgaggagcaggccacatatcgcaatgccatccacgactacttcatcggccggacagacaacctgaccgatgccatcaataagagacacgccgagatctacaagggcctgttcaaggccgagctgtttaatggcaaggtgctgaagcagctgggcaccgtgaccacaaccgagcacgagaacgccctgctgcggagcttcgacaagtttacaacctacttctccggcttttatgagaacaggaagaacgtgttcagcgccgaggatatcagcacagccatcccacaccgcatcgtgcaggacaacttccccaagtttaaggagaattgtcacatcttcacacgcctgatcaccgccgtgcccagcctgcgggagcactttgagaacgtgaagaaggccatcggcatcttcgtgagcacctccatcgaggaggtgttttccttccctttttataaccagctgctgacacagacccagatcgacctgtataaccagctgctgggaggaatctctcgggaggcaggcaccgagaagatcaagggcctgaacgaggtgctgaatctggccatccagaagaatgatgagacagcccacatcatcgcctccctgccacacagattcatccccctgtttaagcagatcctgtccgataggaacaccctgtctttcatcctggaggagtttaagagcgacgaggaagtgatccagtccttctgcaagtacaagacactgctgagaaacgagaacgtgctggagacagccgaggccctgtttaacgagctgaacagcatcgacctgacacacatcttcatcagccacaagaagctggagacaatcagcagcgccctgtgcgaccactgggatacactgaggaatgccctgtatgagcggagaatctccgagctgacaggcaagatcaccaagtctgccaaggagaaggtgcagcgcagcctgaagcacgaggatatcaacctgcaggagatcatctctgccgcaggcaaggagctgagcgaggccttcaagcagaaaaccagcgagatcctgtcccacgcacacgccgccctggatcagccactgcctacaaccctgaagaagcaggaggagaaggagatcctgaagtctcagctggacagcctgctgggcctgtaccacctgctggactggtttgccgtggatgagtccaacgaggtggaccccgagttctctgcccggctgaccggcatcaagctggagatggagccttctctgagcttctacaacaaggccagaaattatgccaccaagaagccctactccgtggagaagttcaagctgaactttcagatgcctacactggcctctggctgggacgtgaataaggagaagaacaatggcgccatcctgtttgtgaagaacggcctgtactatctgggcatcatgccaaagcagaagggcaggtataaggccctgagcttcgagcccacagagaaaaccagcgagggctttgataagatgtactatgactacttccctgatgccgccaagatgatcccaaagtgcagcacccagctgaaggccgtgacagcccactttcagacccacacaacccccatcctgctgtccaacaatttcatcgagcctctggagatcacaaaggagatctacgacctgaacaatcctgagaaggagccaaagaagtttcagacagcctacgccaagaaaaccggcgaccagaagggctacagagaggccctgtgcaagtggatcgacttcacaagggattttctgtccaagtataccaagacaacctctatcgatctgtctagcctgcggccatcctctcagtataaggacctgggcgagtactatgccgagctgaatcccctgctgtaccacatcagcttccagagaatcgccgagaaggagatcatggatgccgtggagacaggcaagctgtacctgttccagatctataacaaggactttgccaagggccaccacggcaagcctaatctgcacacactgtattggaccggcctgttttctccagagaacctggccaagacaagcatcaagctgaatggccaggccgagctgttctaccgccctaagtccaggatgaagaggatggcacaccggctgggagagaagatgctgaacaagaagctgaaggatcagaaaaccccaatccccgacaccctgtaccaggagctgtacgactatgtgaatcacagactgtcccacgacctgtctgatgaggccagggccctgctgcccaacgtgatcaccaaggaggtgtctcacgagatcatcaaggataggcgctttaccagcgacaagttctttttccacgtgcctatcacactgaactatcaggccgccaattccccatctaagttcaaccagagggtgaatgcctacctgaaggagcaccccgagacacctatcatcggcatcgatcggggcgagagaaacctgatctatatcacagtgatcgactccaccggcaagatcctggagcagcggagcctgaacaccatccagcagtttgattaccagaagaagctggacaacagggagaaggagagggtggcagcaaggcaggcctggtctgtggtgggcacaatcaaggatctgaagcagggctatctgagccaggtcatccacgagatcgtggacctgatgatccactaccaggccgtggtggtgctggagaacctgaatttcggctttaagagcaagaggaccggcatcgccgagaaggccgtgtaccagcagttcgagaagatgctgatcgataagctgaattgcctggtgctgaaggactatccagcagagaaagtgggaggcgtgctgaacccataccagctgacagaccagttcacctcctttgccaagatgggcacccagtctggcttcctgttttacgtgcctgccccatatacatctaagatcgatcccctgaccggcttcgtggaccccttcgtgtggaaaaccatcaagaatcacgagagccgcaagcacttcctggagggcttcgactttctgcactacgacgtgaaaaccggcgacttcatcctgcactttaagatgaacagaaatctgtccttccagaggggcctgcccggctttatgcctgcatgggatatcgtgttcgagaagaacgagacacagtttgacgccaagggcacccctttcatcgccggcaagagaatcgtgccagtgatcgagaatcacagattcaccggcagataccgggacctgtatcctgccaacgagctgatcgccctgctggaggagaagggcatcgtgttcagggatggctccaacatcctgccaaagctgctggagaatgacgattctcacgccatcgacaccatggtggccctgatccgcagcgtgctgcagatgcggaactccaatgccgccacaggcgaggactatatcaacagccccgtgcgcgatctgaatggcgtgtgcttcgactcccggtttcagaacccagagtggcccatggacgccgatgccaatggcgcctaccacatcgccctgaagggccagctgctgctgaatcacctgaaggagagcaaggatctgaagctgcagaacggcatctccaatcaggactggctggcctacatccaggagctgcgcaacaaaaggccggcggccacgaaaaaggccggccaggcaaaaaagaaaaagggatcctacccatacgatgttccagattacgcttatccctacgacgtgcctgattatgcatacccatatgatgtccccgactatgcctaa

SEQ ID NO: 7 - protein, 16 aa, unidentified
  REGION 1..16: note = Description of Unknown: Nucleoplasmin NLS peptide
KRPAATKKAGQAKKKK

SEQ ID NO: 8 - protein, 27 aa, synthetic construct
  REGION 1..27: note = Description of Artificial Sequence: Synthetic peptide
YPYDVPDYAYPYDVPDYAYPYDVPDYA

SEQ ID NO: 9 - protein, 1352 aa, synthetic construct
  REGION 1..1352: note = Description of Artificial Sequence: Synthetic polypeptide
MTQFEGFTNLYQVSKTLRFELIPQGKTLKHIQEQGFIEEDKARNDHYKELKPIIDRIYKTYADQCLQLVQLDWENLSAAIDSYRKEKTEETRNALIEEQATYRNAIHDYFIGRTDNLTDAINKRHAEIYKGLFKAELFNGKVLKQLGTVTTTEHENALLRSFDKFTTYFSGFYENRKNVFSAEDISTAIPHRIVQDNFPKFKENCHIFTRLITAVPSLREHFENVKKAIGIFVSTSIEEVFSFPFYNQLLTQTQIDLYNQLLGGISREAGTEKIKGLNEVLNLAIQKNDETAHIIASLPHRFIPLFKQILSDRNTLSFILEEFKSDEEVIQSFCKYKTLLRNENVLETAEALFNELNSIDLTHIFISHKKLETISSALCDHWDTLRNALYERRISELTGKITKSAKEKVQRSLKHEDINLQEIISAAGKELSEAFKQKTSEILSHAHAALDQPLPTTLKKQEEKEILKSQLDSLLGLYHLLDWFAVDESNEVDPEFSARLTGIKLEMEPSLSFYNKARNYATKKPYSVEKFKLNFQMPTLASGWDVNKEKNNGAILFVKNGLYYLGIMPKQKGRYKALSFEPTEKTSEGFDKMYYDYFPDAAKMIPKCSTQLKAVTAHFQTHTTPILLSNNFIEPLEITKEIYDLNNPEKEPKKFQTAYAKKTGDQKGYREALCKWIDFTRDFLSKYTKTTSIDLSSLRPSSQYKDLGEYYAELNPLLYHISFQRIAEKEIMDAVETGKLYLFQIYNKDFAKGHHGKPNLHTLYWTGLFSPENLAKTSIKLNGQAELFYRPKSRMKRMAHRLGEKMLNKKLKDQKTPIPDTLYQELYDYVNHRLSHDLSDEARALLPNVITKEVSHEIIKDRRFTSDKFFFHVPITLNYQAANSPSKFNQRVNAYLKEHPETPIIGIDRGERNLIYITVIDSTGKILEQRSLNTIQQFDYQKKLDNREKERVAARQAWSVVGTIKDLKQGYLSQVIHEIVDLMIHYQAVVVLENLNFGFKSKRTGIAEKAVYQQFEKMLIDKLNCLVLKDYPAEKVGGVLNPYQLTDQFTSFAKMGTQSGFLFYVPAPYTSKIDPLTGFVDPFVWKTIKNHESRKHFLEGFDFLHYDVKTGDFILHFKMNRNLSFQRGLPGFMPAWDIVFEKNETQFDAKGTPFIAGKRIVPVIENHRFTGRYRDLYPANELIALLEEKGIVFRDGSNILPKLLENDDSHAIDTMVALIRSVLQMRNSNAATGEDYINSPVRDLNGVCFDSRFQNPEWPMDADANGAYHIALKGQLLLNHLKESKDLKLQNGISNQDWLAYIQELRNKRPAATKKAGQAKKKKGSYPYDVPDYAYPYDVPDYAYPYDVPDYA

SEQ ID NO: 10 - DNA, 3822 bp, synthetic construct
  misc_feature 1..3822: note = Description of Artificial Sequence: Synthetic polynucleotide
  source 1..3822: mol_type = other DNA
atgagcaagctggagaagtttacaaactgctactccctgtctaagaccctgaggttcaaggccatccctgtgggcaagacccaggagaacatcgacaataagcggctgctggtggaggacgagaagagagccgaggattataagggcgtgaagaagctgctggatcgctactatctgtcttttatcaacgacgtgctgcacagcatcaagctgaagaatctgaacaattacatcagcctgttccggaagaaaaccagaaccgagaaggagaataaggagctggagaacctggagatcaatctgcggaaggagatcgccaaggccttcaagggcaacgagggctacaagtccctgtttaagaaggatatcatcgagacaatcctgccagagttcctggacgataaggacgagatcgccctggtgaacagcttcaatggctttaccacagccttcaccggcttctttgataacagagagaatatgttttccgaggaggccaagagcacatccatcgccttcaggtgtatcaacgagaatctgacccgctacatctctaatatggacatcttcgagaaggtggacgccatctttgataagcacgaggtgcaggagatcaaggagaagatcctgaacagcgactatgatgtggaggatttctttgagggcgagttctttaactttgtgctgacacaggagggcatcgacgtgtataacgccatcatcggcggcttcgtgaccgagagcggcgagaagatcaagggcctgaacgagtacatcaacctgtataatcagaaaaccaagcagaagctgcctaagtttaagccactgtataagcaggtgctgagcgatcgggagtctctgagcttctacggcgagggctatacatccgatgaggaggtgctggaggtgtttagaaacaccctgaacaagaacagcgagatcttcagctccatcaagaagctggagaagctgttcaagaattttgacgagtactctagcgccggcatctttgtgaagaacggccccgccatcagcacaatctccaaggatatcttcggcgagtggaacgtgatccgggacaagtggaatgccgagtatgacgatatccacctgaagaagaaggccgtggtgaccgagaagtacgaggacgatcggagaaagtccttcaagaagatcggctccttttctctggagcagctgcaggagtacgccgacgccgatctgtctgtggtggagaagctgaaggagatcatcatccagaaggtggatgagatctacaaggtgtatggctcctctgagaagctgttcgacgccgattttgtgctggagaagagcctgaagaagaacgacgccgtggtggccatcatgaaggacctgctggattctgtgaagagcttcgagaattacatcaaggccttctttggcgagggcaaggagacaaacagggacgagtccttctatggcgattttgtgctggcctacgacatcctgctgaaggtggaccacatctacgatgccatccgcaattatgtgacccagaagccctactctaaggataagttcaagctgtattttcagaaccctcagttcatgggcggctgggacaaggataaggagacagactatcgggccaccatcctgagatacggctccaagtactatctggccatcatggataagaagtacgccaagtgcctgcagaagatcgacaaggacgatgtgaacggcaattacgagaagatcaactataagctgctgcccggccctaataagatgctgccaaaggtgttcttttctaagaagtggatggcctactataaccccagcgaggacatccagaagatctacaagaatggcacattcaagaagggcgatatgtttaacctgaatgactgtcacaagctgatcgacttctttaaggatagcatctcccggtatccaaagtggtccaatgcctacgatttcaacttttctgagacagagaagtataaggacatcgccggcttttacagagaggtggaggagcagggctataaggtgagcttcgagtctgccagcaagaaggaggtggataagctggtggaggagggcaagctgtatatgttccagatctataacaaggacttttccgataagtctcacggcacacccaatctgcacaccatgtacttcaagctgctgtttgacgagaacaatcacggacagatcaggctgagcggaggagcagagctgttcatgaggcgcgcctccctgaagaaggaggagctggtggtgcacccagccaactcccctatcgccaacaagaatccagataatcccaagaaaaccacaaccctgtcctacgacgtgtataaggataagaggttttctgaggaccagtacgagctgcacatcccaatcgccatcaataagtgccccaagaacatcttcaagatcaatacagaggtgcgcgtgctgctgaagcacgacgataacccctatgtgatcggcatcgataggggcgagcgcaatctgctgtatatcgtggtggtggacggcaagggcaacatcgtggagcagtattccctgaacgagatcatcaacaacttcaacggcatcaggatcaagacagattaccactctctgctggacaagaaggagaaggagaggttcgaggcccgccagaactggacctccatcgagaatatcaaggagctgaaggccggctatatctctcaggtggtgcacaagatctgcgagctggtggagaagtacgatgccgtgatcgccctggaggacctgaactctggctttaagaatagccgcgtgaaggtggagaagcaggtgtatcagaagttcgagaagatgctgatcgataagctgaactacatggtggacaagaagtctaatccttgtgcaacaggcggcgccctgaagggctatcagatcaccaataagttcgagagctttaagtccatgtctacccagaacggcttcatcttttacatccctgcctggctgacatccaagatcgatccatctaccggctttgtgaacctgctgaaaaccaagtataccagcatcgccgattccaagaagttcatcagctcctttgacaggatcatgtacgtgcccgaggaggatctgttcgagtttgccctggactataagaacttctctcgcacagacgccgattacatcaagaagtggaagctgtactcctacggcaaccggatcagaatcttccggaatcctaagaagaacaacgtgttcgactgggaggaggtgtgcctgaccagcgcctataaggagctgttcaacaagtacggcatcaattatcagcagggcgatatcagagccctgctgtgcgagcagtccgacaaggccttctactctagctttatggccctgatgagcctgatgctgcagatgcggaacagcatcacaggccgcaccgacgtggattttctgatcagccctgtgaagaactccgacggcatcttctacgatagccggaactatgaggcccaggagaatgccatcctgccaaagaacgccgacgccaatggcgcctataacatcgccagaaaggtgctgtgggccatcggccagttcaagaaggccgaggacgagaagctggataaggtgaagatcgccatctctaacaaggagtggctggagtacgcccagaccagcgtgaagcacaaaaggccggcggccacgaaaaaggccggccaggcaaaaaagaaaaagggatcctacccatacgatgttccagattacgcttatccctacgacgtgcctgattatgcatacccatatgatgtccccgactatgcctaa

SEQ ID NO: 11 - protein, 1273 aa, synthetic construct
  REGION 1..1273: note = Description of Artificial Sequence: Synthetic polypeptide
MSKLEKFTNCYSLSKTLRFKAIPVGKTQENIDNKRLLVEDEKRAEDYKGVKKLLDRYYLSFINDVLHSIKLKNLNNYISLFRKKTRTEKENKELENLEINLRKEIAKAFKGNEGYKSLFKKDIIETILPEFLDDKDEIALVNSFNGFTTAFTGFFDNRENMFSEEAKSTSIAFRCINENLTRYISNMDIFEKVDAIFDKHEVQEIKEKILNSDYDVEDFFEGEFFNFVLTQEGIDVYNAIIGGFVTESGEKIKGLNEYINLYNQKTKQKLPKFKPLYKQVLSDRESLSFYGEGYTSDEEVLEVFRNTLNKNSEIFSSIKKLEKLFKNFDEYSSAGIFVKNGPAISTISKDIFGEWNVIRDKWNAEYDDIHLKKKAVVTEKYEDDRRKSFKKIGSFSLEQLQEYADADLSVVEKLKEIIIQKVDEIYKVYGSSEKLFDADFVLEKSLKKNDAVVAIMKDLLDSVKSFENYIKAFFGEGKETNRDESFYGDFVLAYDILLKVDHIYDAIRNYVTQKPYSKDKFKLYFQNPQFMGGWDKDKETDYRATILRYGSKYYLAIMDKKYAKCLQKIDKDDVNGNYEKINYKLLPGPNKMLPKVFFSKKWMAYYNPSEDIQKIYKNGTFKKGDMFNLNDCHKLIDFFKDSISRYPKWSNAYDFNFSETEKYKDIAGFYREVEEQGYKVSFESASKKEVDKLVEEGKLYMFQIYNKDFSDKSHGTPNLHTMYFKLLFDENNHGQIRLSGGAELFMRRASLKKEELVVHPANSPIANKNPDNPKKTTTLSYDVYKDKRFSEDQYELHIPIAINKCPKNIFKINTEVRVLLKHDDNPYVIGIDRGERNLLYIVVVDGKGNIVEQYSLNEIINNFNGIRIKTDYHSLLDKKEKERFEARQNWTSIENIKELKAGYISQVVHKICELVEKYDAVIALEDLNSGFKNSRVKVEKQVYQKFEKMLIDKLNYMVDKKSNPCATGGALKGYQITNKFESFKSMSTQNGFIFYIPAWLTSKIDPSTGFVNLLKTKYTSIADSKKFISSFDRIMYVPEEDLFEFALDYKNFSRTDADYIKKWKLYSYGNRIRIFRNPKKNNVFDWEEVCLTSAYKELFNKYGINYQQGDIRALLCEQSDKAFYSSFMALMSLMLQMRNSITGRTDVDFLISPVKNSDGIFYDSRNYEAQENAILPKNADANGAYNIARKVLWAIGQFKKAEDEKLDKVKIAISNKEWLEYAQTSVKHKRPAATKKAGQAKKKKGSYPYDVPDYAYPYDVPDYAYPYDVPDYA

SEQ ID NO: 12 - protein, 4 aa, synthetic construct
  REGION 1..4: note = Description of Artificial Sequence: Synthetic peptide
GGGS

SEQ ID NO: 13 - protein, 5 aa, synthetic construct
  REGION 1..5: note = Description of Artificial Sequence: Synthetic peptide
GGGGS

SEQ ID NO: 14-15 - skipped (2 entries)

SEQ ID NO: 16 - protein, 7 aa, Simian virus 40
PKKKRRV

SEQ ID NO: 17 - DNA, 4038 bp, synthetic construct
  misc_feature 1..4038: note = Description of Artificial Sequence: Synthetic polynucleotide
  source 1..4038: mol_type = other DNA
atgagcatctaccaggagttcgtcaacaagtattcactgagtaagacactgcggttcgagctgatcccacagggcaagacactggagaacatcaaggcccgaggcctgattctggacgatgagaagcgggcaaaagactataagaaagccaagcagatcattgataaataccaccagttctttatcgaggaaattctgagctccgtgtgcatcagtgaggatctgctgcagaattactcagacgtgtacttcaagctgaagaagagcgacgatgacaacctgcagaaggacttcaagtccgccaaggacaccatcaagaaacagattagcgagtacatcaaggactccgaaaagtttaaaaatctgttcaaccagaatctgatcgatgctaagaaaggccaggagtccgacctgatcctgtggctgaaacagtctaaggacaatgggattgaactgttcaaggctaactccgatatcactgatattgacgaggcactggaaatcatcaagagcttcaagggatggaccacatactttaaaggcttccacgagaaccgcaagaacgtgtactccagcaacgacattcctacctccatcatctaccgaatcgtcgatgacaatctgccaaagttcctggagaacaaggccaaatatgaatctctgaaggacaaagctcccgaggcaattaattacgaacagatcaagaaagatctggctgaggaactgacattcgatatcgactataagactagcgaggtgaaccagagggtcttttccctggacgaggtgtttgaaatcgccaatttcaacaattacctgaaccagtccggcattactaaattcaataccatcattggcgggaagtttgtgaacggggagaataccaagcgcaagggaattaacgaatacatcaatctgtatagccagcagatcaacgacaaaactctgaagaaatacaagatgtctgtgctgttcaaacagatcctgagtgataccgagtccaagtcttttgtcattgataaactggaagatgactcagacgtggtcactaccatgcagagcttttatgagcagatcgccgctttcaagacagtggaggaaaaatctattaaggaaactctgagtctgctgttcgatgacctgaaagcccagaagctggacctgagtaagatctacttcaaaaacgataagagtctgacagacctgtcacagcaggtgtttgatgactattccgtgattgggaccgccgtcctggagtacattacacagcagatcgctccaaagaacctggataatccctctaagaaagagcaggaactgatcgctaagaaaaccgagaaggcaaaatatctgagtctggaaacaattaagctggcactggaggagttcaacaagcacagggatattgacaaacagtgccgctttgaggaaatcctggccaacttcgcagccatccccatgatttttgatgagatcgcccagaacaaagacaatctggctcagatcagtattaagtaccagaaccagggcaagaaagacctgctgcaggcttcagcagaagatgacgtgaaagccatcaaggatctgctggaccagaccaacaatctgctgcacaagctgaaaatcttccatattagtcagtcagaggataaggctaatatcctggataaagacgaacacttctacctggtgttcgaggaatgttacttcgagctggcaaacattgtccccctgtataacaagattaggaactacatcacacagaagccttactctgacgagaagtttaaactgaacttcgaaaatagtaccctggccaacgggtgggataagaacaaggagcctgacaacacagctatcctgttcatcaaggatgacaagtactatctgggagtgatgaataagaaaaacaataagatcttcgatgacaaagccattaaggagaacaaaggggaaggatacaagaaaatcgtgtataagctgctgcccggcgcaaataagatgctgcctaaggtgttcttcagcgccaagagtatcaaattctacaacccatccgaggacatcctgcggattagaaatcactcaacacatactaagaacgggagcccccagaagggatatgagaaatttgagttcaacatcgaggattgcaggaagtttattgacttctacaagcagagcatctccaaacaccctgaatggaaggattttggcttccggttttccgacacacagagatataactctatcgacgagttctaccgcgaggtggaaaatcaggggtataagctgacttttgagaacatttctgaaagttacatcgacagcgtggtcaatcagggaaagctgtacctgttccagatctataacaaagatttttcagcatacagcaagggcagaccaaacctgcatacactgtactggaaggccctgttcgatgagaggaatctgcaggacgtggtctataaactgaacggagaggccgaactgttttaccggaagcagtctattcctaagaaaatcactcacccagctaaggaggccatcgctaacaagaacaaggacaatcctaagaaagagagcgtgttcgaatacgatctgattaaggacaagcggttcaccgaagataagttctttttccattgtccaatcaccattaacttcaagtcaagcggcgctaacaagttcaacgacgagatcaatctgctgctgaaggaaaaagcaaacgatgtgcacatcctgagcattgaccgaggagagcggcatctggcctactataccctggtggatggcaaagggaatatcattaagcaggatacattcaacatcattggcaatgaccggatgaaaaccaactaccacgataaactggctgcaatcgagaaggatagagactcagctaggaaggactggaagaaaatcaacaacattaaggagatgaaggaaggctatctgagccaggtggtccatgagattgcaaagctggtcatcgaatacaatgccattgtggtgttcgaggatctgaacttcggctttaagagggggcgctttaaggtggaaaaacaggtctatcagaagctggagaaaatgctgatcgaaaagctgaattacctggtgtttaaagataacgagttcgacaagaccggaggcgtcctgagagcctaccagctgacagctccctttgaaactttcaagaaaatgggaaaacagacaggcatcatctactatgtgccagccggattcacttccaagatctgccccgtgaccggctttgtcaaccagctgtaccctaaatatgagtcagtgagcaagtcccaggaatttttcagcaagttcgataagatctgttataatctggacaaggggtacttcgagttttccttcgattacaagaacttcggcgacaaggccgctaaggggaaatggaccattgcctccttcggatctcgcctgatcaactttcgaaattccgataaaaaccacaattgggacactagggaggtgtacccaaccaaggagctggaaaagctgctgaaagactactctatcgagtatggacatggcgaatgcatcaaggcagccatctgtggcgagagtgataagaaatttttcgccaagctgacctcagtgctgaatacaatcctgcagatgcggaactcaaagaccgggacagaactggactatctgattagccccgtggctgatgtcaacggaaacttcttcgacagcagacaggcacccaaaaatatgcctcaggatgcagacgccaacggggcctaccacatcgggctgaagggactgatgctgctgggccggatcaagaacaatcaggaggggaagaagctgaacctggtcattaagaacgaggaatacttcgagtttgtccagaatagaaataacaaaaggccggcggccacgaaaaaggccggccaggcaaaaaagaaaaagggatcctacccatacgatgttccagattacgcttatccctacgacgtgcctgattatgcatacccatatgatgtccccgactatgcctaa

SEQ ID NO: 18 - protein, 1345 aa, synthetic construct
  REGION 1..1345: note = Description of Artificial Sequence: Synthetic polypeptide
MSIYQEFVNKYSLSKTLRFELIPQGKTLENIKARGLILDDEKRAKDYKKAKQIIDKYHQFFIEEILSSVCISEDLLQNYSDVYFKLKKSDDDNLQKDFKSAKDTIKKQISEYIKDSEKFKNLFNQNLIDAKKGQESDLILWLKQSKDNGIELFKANSDITDIDEALEIIKSFKGWTTYFKGFHENRKNVYSSNDIPTSIIYRIVDDNLPKFLENKAKYESLKDKAPEAINYEQIKKDLAEELTFDIDYKTSEVNQRVFSLDEVFEIANFNNYLNQSGITKFNTIIGGKFVNGENTKRKGINEYINLYSQQINDKTLKKYKMSVLFKQILSDTESKSFVIDKLEDDSDVVTTMQSFYEQIAAFKTVEEKSIKETLSLLFDDLKAQKLDLSKIYFKNDKSLTDLSQQVFDDYSVIGTAVLEYITQQIAPKNLDNPSKKEQELIAKKTEKAKYLSLETIKLALEEFNKHRDIDKQCRFEEILANFAAIPMIFDEIAQNKDNLAQISIKYQNQGKKDLLQASAEDDVKAIKDLLDQTNNLLHKLKIFHISQSEDKANILDKDEHFYLVFEECYFELANIVPLYNKIRNYITQKPYSDEKFKLNFENSTLANGWDKNKEPDNTAILFIKDDKYYLGVMNKKNNKIFDDKAIKENKGEGYKKIVYKLLPGANKMLPKVFFSAKSIKFYNPSEDILRIRNHSTHTKNGSPQKGYEKFEFNIEDCRKFIDFYKQSISKHPEWKDFGFRFSDTQRYNSIDEFYREVENQGYKLTFENISESYIDSVVNQGKLYLFQIYNKDFSAYSKGRPNLHTLYWKALFDERNLQDVVYKLNGEAELFYRKQSIPKKITHPAKEAIANKNKDNPKKESVFEYDLIKDKRFTEDKFFFHCPITINFKSSGANKFNDEINLLLKEKANDVHILSIDRGERHLAYYTLVDGKGNIIKQDTFNIIGNDRMKTNYHDKLAAIEKDRDSARKDWKKINNIKEMKEGYLSQVVHEIAKLVIEYNAIVVFEDLNFGFKRGRFKVEKQVYQKLEKMLIEKLNYLVFKDNEFDKTGGVLRAYQLTAPFETFKKMGKQTGIIYYVPAGFTSKICPVTGFVNQLYPKYESVSKSQEFFSKFDKICYNLDKGYFEFSFDYKNFGDKAAKGKWTIASFGSRLINFRNSDKNHNWDTREVYPTKELEKLLKDYSIEYGHGECIKAAICGESDKKFFAKLTSVLNTILQMRNSKTGTELDYLISPVADVNGNFFDSRQAPKNMPQDADANGAYHIGLKGLMLLGRIKNNQEGKKLNLVIKNEEYFEFVQNRNNKRPAATKKAGQAKKKKGSYPYDVPDYAYPYDVPDYAYPYDVPDYA

SEQ ID NO: 19 - DNA, 21 bp, Simian virus 40
  source 1..21: mol_type = other DNA
ccaaagaaaaagaggaaagtc

SEQ ID NO: 20 - DNA, 21 bp, Simian virus 40
  source 1..21: mol_type = other DNA
cctaaaaagaaacgaaaggtt

SEQ ID NO: 21 - DNA, 48 bp, unidentified
  misc_feature 1..48: note = Description of Unknown: Nucleoplasmin NLS peptide
  source 1..48: mol_type = other DNA
aaaaggccggcggccacgaaaaaggccggccaggcaaaaaagaaaaag

SEQ ID NO: 22 - DNA, 21 bp, Simian virus 40
  source 1..21: mol_type = other DNA
cccaagaagaagaggaaagtc

SEQ ID NO: 23 - DNA, 93 bp, synthetic construct
  misc_feature 1..93: note = Description of Artificial Sequence: Synthetic oligonucleotide
  source 1..93: mol_type = other DNA
tctggtggttcttctggtggttctagcggcagcgagactcccgggacctcagagtccgccacacccgaaagttccggagggagtagcggcggg

SEQ ID NO: 24 - protein, 7 aa, Simian virus 40
PKKKRKV

SEQ ID NO: 25 - protein, 31 aa, synthetic construct
  REGION 1..31: note = Description of Artificial Sequence: Synthetic polypeptide
SGGSSGGSSGSETPGTSESATPESSGGSSGG

SEQ ID NO: 26 - DNA, 24 bp, synthetic construct
  misc_feature 1..24: note = Description of Artificial Sequence: Synthetic oligonucleotide
  source 1..24: mol_type = other DNA
aaccagtggaggcaagagggcggc

SEQ ID NO: 27 - DNA, 24 bp, synthetic construct
  misc_feature 1..24: note = Description of Artificial Sequence: Synthetic oligonucleotide
  source 1..24: mol_type = other DNA
aaccaagacaggtcactgtttcag

SEQ ID NO: 28 - DNA, 24 bp, synthetic construct
  misc_feature 1..24: note = Description of Artificial Sequence: Synthetic oligonucleotide
  source 1..24: mol_type = other DNA
aaccacaccttcacctgggccagg

SEQ ID NO: 29 - DNA, 24 bp, synthetic construct
  misc_feature 1..24: note = Description of Artificial Sequence: Synthetic oligonucleotide
  source 1..24: mol_type = other DNA
aaccggtggcgcattgccacgaag

SEQ ID NO: 30 - DNA, 24 bp, synthetic construct
  misc_feature 1..24: note = Description of Artificial Sequence: Synthetic oligonucleotide
  source 1..24: mol_type = other DNA
aatagcattgcagagaggcgtatc

SEQ ID NO: 31 - DNA, 24 bp, synthetic construct
  misc_feature 1..24: note = Description of Artificial Sequence: Synthetic oligonucleotide
  source 1..24: mol_type = other DNA
aatatgctgtctgaagccatcgct

SEQ ID NO: 32 - DNA, 24 bp, synthetic construct
  misc_feature 1..24: note = Description of Artificial Sequence: Synthetic oligonucleotide
  source 1..24: mol_type = other DNA
aataagtggcagagtgctaaggga

SEQ ID NO: 33 - DNA, 24 bp, synthetic construct
  misc_feature 1..24: note = Description of Artificial Sequence: Synthetic oligonucleotide
  source 1..24: mol_type = other DNA
aatatggagcctgctccaggtggg

SEQ ID NO: 34 - DNA, 24 bp, synthetic construct
  misc_feature 1..24: note = Description of Artificial Sequence: Synthetic oligonucleotide
  source 1..24: mol_type = other DNA
aatcagtacgcagagagtcgccgt

SEQ ID NO: 35 - DNA, 24 bp, synthetic construct
  misc_feature 1..24: note = Description of Artificial Sequence: Synthetic oligonucleotide
  source 1..24: mol_type = other DNA
aatcctaactgagaccttacaccg

SEQ ID NO: 36 - DNA, 24 bp, synthetic construct
  misc_feature 1..24: note = Description of Artificial Sequence: Synthetic oligonucleotide
  source 1..24: mol_type = other DNA
aatgcgccaccggttgatgtgatg

SEQ ID NO: 37 - DNA, 24 bp, synthetic construct
  misc_feature 1..24: note = Description of Artificial Sequence: Synthetic oligonucleotide
  source 1..24: mol_type = other DNA
accccggctctggctaaagaggga

SEQ ID NO: 38 - DNA, 24 bp, synthetic construct
  misc_feature 1..24: note = Description of Artificial Sequence: Synthetic oligonucleotide
  source 1..24: mol_type = other DNA
accccctatttctgacctcccaaa

SEQ ID NO: 39 - DNA, 24 bp, synthetic construct
  misc_feature 1..24: note = Description of Artificial Sequence: Synthetic oligonucleotide
  source 1..24: mol_type = other DNA
acccagaggctcaagtgagcagct

SEQ ID NO: 40 - DNA, 24 bp, synthetic construct
  misc_feature 1..24: note = Description of Artificial Sequence: Synthetic oligonucleotide
  source 1..24: mol_type = other DNA
accctagtcattggaggtgacatc

SEQ ID NO: 41 - DNA, 24 bp, synthetic construct
  misc_feature 1..24: note = Description of Artificial Sequence: Synthetic oligonucleotide
  source 1..24: mol_type = other DNA
acccacgagggcagagtgctgctt

SEQ ID NO: 42 - DNA, 24 bp, synthetic construct
  misc_feature 1..24: note = Description of Artificial Sequence: Synthetic oligonucleotide
  source 1..24: mol_type = other DNA
acccaataagtggcagagtgctaa

SEQ ID NO: 43 - DNA, 24 bp, synthetic construct
  misc_feature 1..24: note = Description of Artificial Sequence: Synthetic oligonucleotide
  source 1..24: mol_type = other DNA
agccgccctcttgcctccactggt

SEQ ID NO: 44 - DNA, 24 bp, synthetic construct
  misc_feature 1..24: note = Description of Artificial Sequence: Synthetic oligonucleotide
  source 1..24: mol_type = other DNA
agccatcgcttcctcctgaaaatg

SEQ ID NO: 45 - DNA, 24 bp, synthetic construct
  misc_feature 1..24: note = Description of Artificial Sequence: Synthetic oligonucleotide
  source 1..24: mol_type = other DNA
agcctcacccctctagccctacat

SEQ ID NO: 46 - DNA, 24 bp, synthetic construct
  misc_feature 1..24: note = Description of Artificial Sequence: Synthetic oligonucleotide
  source 1..24: mol_type = other DNA
agcctgctccaggtggggaataag

SEQ ID NO: 47 - DNA, 24 bp, synthetic construct
  misc_feature 1..24: note = Description of Artificial Sequence: Synthetic oligonucleotide
  source 1..24: mol_type = other DNA
agtaacagacatggaccatcagga

SEQ ID NO: 48 - DNA, 24 bp, synthetic construct
  misc_feature 1..24: note = Description of Artificial Sequence: Synthetic oligonucleotide
  source 1..24: mol_type = other DNA
agtaccagattctgagcagggaga

SEQ ID NO: 49 - DNA, 24 bp, synthetic construct
  misc_feature 1..24: note = Description of Artificial Sequence: Synthetic oligonucleotide
  source 1..24: mol_type = other DNA
agtctccgtgaacgttcccttagc

SEQ ID NO: 50 - DNA, 24 bp, synthetic construct
  misc_feature 1..24: note = Description of Artificial Sequence: Synthetic oligonucleotide
  source 1..24: mol_type = other DNA
agtctgtcctgaacctgatgacac

SEQ ID NO: 51 - DNA, 24 bp, synthetic construct
  misc_feature 1..24: note = Description of Artificial Sequence: Synthetic oligonucleotide
  source 1..24: mol_type = other DNA
atcaggaaacattaacgtactgat

SEQ ID NO: 52 - DNA, 24 bp, synthetic construct
  misc_feature 1..24: note = Description of Artificial Sequence: Synthetic oligonucleotide
  source 1..24: mol_type = other DNA
atcagaatcctcttcgatgccatt

SEQ ID NO: 53 - DNA, 24 bp, synthetic construct
  misc_feature 1..24: note = Description of Artificial Sequence: Synthetic oligonucleotide
  source 1..24: mol_type = other DNA
atcctcacagcagccccttgagaa

SEQ ID NO: 54 - DNA, 24 bp, synthetic construct
  misc_feature 1..24: note = Description of Artificial Sequence: Synthetic oligonucleotide
  source 1..24: mol_type = other DNA
atccaatcaactctatacgaaaat

SEQ ID NO: 55 - DNA, 24 bp, synthetic construct
  misc_feature 1..24: note = Description of Artificial Sequence: Synthetic oligonucleotide
  source 1..24: mol_type = other DNA
atccccaacatgcactgatgttgt

SEQ ID NO: 56 - DNA, 24 bp, synthetic construct
  misc_feature 1..24: note = Description of Artificial Sequence: Synthetic oligonucleotide
  source 1..24: mol_type = other DNA
atccatcggcgctttggtcggcat

SEQ ID NO: 57 - DNA, 24 bp, synthetic construct
  misc_feature 1..24: note = Description of Artificial Sequence: Synthetic oligonucleotide
  source 1..24: mol_type = other DNA
attaacgtactgatgttaacagct

SEQ ID NO: 58 - DNA, 24 bp, synthetic construct
  misc_feature 1..24: note = Description of Artificial Sequence: Synthetic oligonucleotide
  source 1..24: mol_type = other DNA
attaacattaacaagaagcatttg

SEQ ID NO: 59 - DNA, 24 bp, synthetic construct
  misc_feature 1..24: note = Description of Artificial Sequence: Synthetic oligonucleotide
  source 1..24: mol_type = other DNA
attattcaagtggcgcagatctag

SEQ ID NO: 60 - DNA, 24 bp, synthetic construct
  misc_feature 1..24: note = Description of Artificial Sequence: Synthetic oligonucleotide
  source 1..24: mol_type = other DNA
attagaaggagatgctcctgtctc

SEQ ID NO: 61 - DNA, 24 bp, synthetic construct
  misc_feature 1..24: note = Description of Artificial Sequence: Synthetic oligonucleotide
  source 1..24: mol_type = other DNA
attcaccgagcaggagtgagggaa

SEQ ID NO: 62 - DNA, 24 bp, synthetic construct
  misc_feature 1..24: note = Description of Artificial Sequence: Synthetic oligonucleotide
  source 1..24: mol_type = other DNA
attccccacctggagcaggctcca

SEQ ID NO: 63 - DNA, 24 bp, synthetic construct
  misc_feature 1..24: note = Description of Artificial Sequence: Synthetic oligonucleotide
  source 1..24: mol_type = other DNA
attctgatgagcctttagagagaa

SEQ ID NO: 64 - DNA, 24 bp, synthetic construct
  misc_feature 1..24: note = Description of Artificial Sequence: Synthetic oligonucleotide
  source 1..24: mol_type = other DNA
attccctctttagccagagccggg

SEQ ID NO: 65 - DNA, 24 bp, synthetic construct
  misc_feature 1..24: note = Description of Artificial Sequence: Synthetic oligonucleotide
  source 1..24: mol_type = other DNA
attcgcacggctctggagcggcgg

SEQ ID NO: 66 - DNA, 24 bp, synthetic construct
  misc_feature 1..24: note = Description of Artificial Sequence: Synthetic oligonucleotide
  source 1..24: mol_type = other DNA
attgggtcagctgttaacatcagt

SEQ ID NO: 67 - DNA, 24 bp, synthetic construct
  misc_feature 1..24: note = Description of Artificial Sequence: Synthetic oligonucleotide
  source 1..24: mol_type = other DNA
attgttatgaacctgggtgaagtc

SEQ ID NO: 68 - DNA, 24 bp, synthetic construct
  misc_feature 1..24: note = Description of Artificial Sequence: Synthetic oligonucleotide
  source 1..24: mol_type = other DNA
attggaatcctggagtgacccctg

SEQ ID NO: 69 - DNA, 24 bp, synthetic construct
  misc_feature 1..24: note = Description of Artificial Sequence: Synthetic oligonucleotide
  source 1..24: mol_type = other DNA
attggattgagaatagaattcttc

SEQ ID NO: 70 - DNA, 24 bp, synthetic construct
  misc_feature 1..24: note = Description of Artificial Sequence: Synthetic oligonucleotide
  source 1..24: mol_type = other DNA
attggaacatccgcgaaatgatac

SEQ ID NO: 71 - DNA, 24 bp, synthetic construct
  misc_feature 1..24: note = Description of Artificial Sequence: Synthetic oligonucleotide
  source 1..24: mol_type = other DNA
atttggctcagcaggcacctgcct

SEQ ID NO: 72 - DNA, 24 bp, synthetic construct
  misc_feature 1..24: note = Description of Artificial Sequence: Synthetic oligonucleotide
  source 1..24: mol_type = other DNA
atttgctttccacccacctttccc

SEQ ID NO: 73 - DNA, 24 bp, synthetic construct
  misc_feature 1..24: note = Description of Artificial Sequence: Synthetic oligonucleotide
  source 1..24: mol_type = other DNA
atttctgacctcccaaacagctac

SEQ ID NO: 74 - DNA, 24 bp, synthetic construct
  misc_feature 1..24: note = Description of Artificial Sequence: Synthetic oligonucleotide
  source 1..24: mol_type = other DNA
atttcttctttctgcactaaattg

SEQ ID NO: 75 - DNA, 24 bp, synthetic construct
  misc_feature 1..24: note = Description of Artificial Sequence: Synthetic oligonucleotide
  source 1..24: mol_type = other DNA
atttcgcggatgttccaatcagta

SEQ ID NO: 76 - DNA, 24 bp, synthetic construct
  misc_feature 1..24: note = Description of Artificial Sequence: Synthetic oligonucleotide
  source 1..24: mol_type = other DNA
caccgtgcgccgggccttgcagtg

SEQ ID NO: 77 - DNA, 24 bp, synthetic construct
  misc_feature 1..24: note = Description of Artificial Sequence: Synthetic oligonucleotide
  source 1..24: mol_type = other DNA
caccgaggcatctctgcaccgagg

SEQ ID NO: 78 - DNA, 24 bp, synthetic construct
  misc_feature 1..24: note = Description of Artificial Sequence: Synthetic oligonucleotide
  source 1..24: mol_type = other DNA
ccccgcccaaagccgccctcttgc

SEQ ID NO: 79 - DNA, 24 bp, synthetic construct
  misc_feature 1..24: note = Description of Artificial Sequence: Synthetic oligonucleotide
  source 1..24: mol_type = other DNA
ccccgccttcagaagagggtgcat

SEQ ID NO: 80 - DNA, 24 bp, synthetic construct
  misc_feature 1..24: note = Description of Artificial Sequence: Synthetic oligonucleotide
  source 1..24: mol_type = other DNA
ccccagagggttctagacccagag

SEQ ID NO: 81 - DNA, 24 bp, synthetic construct
  misc_feature 1..24: note = Description of Artificial Sequence: Synthetic oligonucleotide
  source 1..24: mol_type = other DNA
ccccagggccagcccagcagccaa

SEQ ID NO: 82 - DNA, 24 bp, synthetic construct
  misc_feature 1..24: note = Description of Artificial Sequence: Synthetic oligonucleotide
  source 1..24: mol_type = other DNA
cgcacggctctggagcggcggctg

SEQ ID NO: 83 - DNA, 24 bp, synthetic construct
  misc_feature 1..24: note = Description of Artificial Sequence: Synthetic oligonucleotide
  source 1..24: mol_type = other DNA
cgcattgccacgaagcaggccaat

SEQ ID NO: 84 - DNA, 24 bp, synthetic construct
  misc_feature 1..24: note = Description of Artificial Sequence: Synthetic oligonucleotide
  source 1..24: mol_type = other DNA
cgccgctccagagccgtgcgaatg

SEQ ID NO: 85 - DNA, 24 bp, synthetic construct
  misc_feature 1..24: note = Description of Artificial Sequence: Synthetic oligonucleotide
  source 1..24: mol_type = other DNA
cgccaccggttgatgtgatgggag

SEQ ID NO: 86 - DNA, 24 bp, synthetic construct
  misc_feature 1..24: note = Description of Artificial Sequence: Synthetic oligonucleotide
  source 1..24: mol_type = other DNA
cgccacatccatcggcgctttggt

SEQ ID NO: 87 - DNA, 24 bp, synthetic construct
  misc_feature 1..24: note = Description of Artificial Sequence: Synthetic oligonucleotide
  source 1..24: mol_type = other DNA
cgccgatggatgtggcgcaggtag

SEQ ID NO: 88 - DNA, 24 bp, synthetic construct
  misc_feature 1..24: note = Description of Artificial Sequence: Synthetic oligonucleotide
  source 1..24: mol_type = other DNA
cgtcagcacctgggaccccgccac

SEQ ID NO: 89 - DNA, 24 bp, synthetic construct
  misc_feature 1..24: note = Description of Artificial Sequence: Synthetic oligonucleotide
  source 1..24: mol_type = other DNA
cgtctccaaggtgaaagcggaagt

SEQ ID NO: 90 - DNA, 24 bp, synthetic construct
  misc_feature 1..24: note = Description of Artificial Sequence: Synthetic oligonucleotide
  source 1..24: mol_type = other DNA
ctcaaacggtccccagagggttct

SEQ ID NO: 91 - DNA, 24 bp, synthetic construct
  misc_feature 1..24: note = Description of Artificial Sequence: Synthetic oligonucleotide
  source 1..24: mol_type = other DNA
ctcaaaactcatgggatgtgattc

SEQ ID NO: 92 - DNA, 24 bp, synthetic construct
  misc_feature 1..24: note = Description of Artificial Sequence: Synthetic oligonucleotide
  source 1..24: mol_type = other DNA
ctccgtgaacgttcccttagcact

SEQ ID NO: 93 - DNA, 24 bp, synthetic construct
  misc_feature 1..24: note = Description of Artificial Sequence: Synthetic oligonucleotide
  source 1..24: mol_type = other DNA
ctccttctaatgagaaacggtgta

SEQ ID NO: 94 - DNA, 24 bp, synthetic construct
  misc_feature 1..24: note = Description of Artificial Sequence: Synthetic oligonucleotide
  source 1..24: mol_type = other DNA
ctccactggttgtgcagccgccgc

SEQ ID NO: 95 - DNA, 24 bp, synthetic construct
  misc_feature 1..24: note = Description of Artificial Sequence: Synthetic oligonucleotide
  source 1..24: mol_type = other DNA
ctccagagccgtgcgaatggggcc

SEQ ID NO: 96 - DNA, 24 bp, synthetic construct
  misc_feature 1..24: note = Description of Artificial Sequence: Synthetic oligonucleotide
  source 1..24: mol_type = other DNA
ctctggggaacacgcccggtgtca

SEQ ID NO: 97 - DNA, 24 bp, synthetic construct
  misc_feature 1..24: note = Description of Artificial Sequence: Synthetic oligonucleotide
  source 1..24: mol_type = other DNA
cttattgggtcagctgttaacatc

SEQ ID NO: 98 - DNA, 24 bp, synthetic construct
  misc_feature 1..24: note = Description of Artificial Sequence: Synthetic oligonucleotide
  source 1..24: mol_type = other DNA
cttattccccacctggagcaggct

SEQ ID NO: 99 - DNA, 24 bp, synthetic construct
  misc_feature 1..24: note = Description of Artificial Sequence: Synthetic oligonucleotide
  source 1..24: mol_type = other DNA
cttactaatcagatggaagctctt

SEQ ID NO: 100 - DNA, 24 bp, synthetic construct
  misc_feature 1..24: note = Description of Artificial Sequence: Synthetic oligonucleotide
  source 1..24: mol_type = other DNA
cttacaccgtttctcattagaagg

SEQ ID NO: 101 - DNA, 24 bp, synthetic construct
  misc_feature 1..24: note = Description of Artificial Sequence: Synthetic oligonucleotide
  source 1..24: mol_type = other DNA
cttccgctttcaccttggagacgg

SEQ ID NO: 102 - DNA, 24 bp, synthetic construct
  misc_feature 1..24: note = Description of Artificial Sequence: Synthetic oligonucleotide
  source 1..24: mol_type = other DNA
cttcacccaggttcataacaatgt

SEQ ID NO: 103 - DNA, 24 bp, synthetic construct
  misc_feature 1..24: note = Description of Artificial Sequence: Synthetic oligonucleotide
  source 1..24: mol_type = other DNA
cttctccccgctccaacgccctca

SEQ ID NO: 104 - DNA, 24 bp, synthetic construct
  misc_feature 1..24: note = Description of Artificial Sequence: Synthetic oligonucleotide
  source 1..24: mol_type = other DNA
cttctaatgagaaacggtgtaagg

SEQ ID NO: 105 - DNA, 24 bp, synthetic construct
  misc_feature 1..24: note = Description of Artificial Sequence: Synthetic oligonucleotide
  source 1..24: mol_type = other DNA
cttcgcgcacctcatggaatccct

SEQ ID NO: 106 - DNA, 24 bp, synthetic construct
  misc_feature 1..24: note = Description of Artificial Sequence: Synthetic oligonucleotide
  source 1..24: mol_type = other DNA
cttgacaggcgagtaacagacatg

SEQ ID NO: 107 - DNA, 24 bp, synthetic construct
  misc_feature 1..24: note = Description of Artificial Sequence: Synthetic oligonucleotide
  source 1..24: mol_type = other DNA
cttgttaatgttaataacttgctt

SEQ ID NO: 108 - DNA, 24 bp, synthetic construct
  misc_feature 1..24: note = Description of Artificial Sequence: Synthetic oligonucleotide
  source 1..24: mol_type = other DNA
cttggttaactgagtgtgtcatca

SEQ ID NO: 109 - DNA, 24 bp, synthetic construct
  misc_feature 1..24: note = Description of Artificial Sequence: Synthetic oligonucleotide
  source 1..24: mol_type = other DNA
cttggggagtcccagaggtatcca

SEQ ID NO: 110 - DNA, 24 bp, synthetic construct
  misc_feature 1..24: note = Description of Artificial Sequence: Synthetic oligonucleotide
  source 1..24: mol_type = other DNA
ctttggtcaggttggctgctgggc

SEQ ID NO: 111 - DNA, 24 bp, synthetic construct
  misc_feature 1..24: note = Description of Artificial Sequence: Synthetic oligonucleotide
  source 1..24: mol_type = other DNA
ctttccctggcctacctcactggc

SEQ ID NO: 112 - DNA, 24 bp, synthetic construct
  misc_feature 1..24: note = Description of Artificial Sequence: Synthetic oligonucleotide
  source 1..24: mol_type = other DNA
ctttagccagagccggggtgtgca

SEQ ID NO: 113 - DNA, 24 bp, synthetic construct
  misc_feature 1..24: note = Description of Artificial Sequence: Synthetic oligonucleotide
  source 1..24: mol_type = other DNA
ctttagagagaaggctgtccttag

SEQ ID NO: 114 - DNA, 24 bp, synthetic construct
  misc_feature 1..24: note = Description of Artificial Sequence: Synthetic oligonucleotide
  source 1..24: mol_type = other DNA
ctttggtcggcatggccccattcg

SEQ ID NO: 115 - DNA, 24 bp, synthetic construct
  misc_feature 1..24: note = Description of Artificial Sequence: Synthetic oligonucleotide
  source 1..24: mol_type = other DNA
gcccggtgtcacgccacttgacag

SEQ ID NO: 116 - DNA, 24 bp, synthetic construct
  misc_feature 1..24: note = Description of Artificial Sequence: Synthetic oligonucleotide
  source 1..24: mol_type = other DNA
gccccacgcttcaggcacgaagga

SEQ ID NO: 117 - DNA, 24 bp, synthetic construct
  misc_feature 1..24: note = Description of Artificial Sequence: Synthetic oligonucleotide
  source 1..24: mol_type = other DNA
gtcacgccacttgacaggcgagta

SEQ ID NO: 118 - DNA, 24 bp, synthetic construct
  misc_feature 1..24: note = Description of Artificial Sequence: Synthetic oligonucleotide
  source 1..24: mol_type = other DNA
gtcatcaggttcaggacagactgc

SEQ ID NO: 119 - DNA, 24 bp, synthetic construct
  misc_feature 1..24: note = Description of Artificial Sequence: Synthetic oligonucleotide
  source 1..24: mol_type = other DNA
gtccccagagggttctagacccag

SEQ ID NO: 120 - DNA, 24 bp, synthetic construct
  misc_feature 1..24: note = Description of Artificial Sequence: Synthetic oligonucleotide
  source 1..24: mol_type = other DNA
gtccaggagacaggagcatctcct

SEQ ID NO: 121 - DNA, 24 bp, synthetic construct
  misc_feature 1..24: note = Description of Artificial Sequence: Synthetic oligonucleotide
  source 1..24: mol_type = other DNA
gtcccaggtgctgacgtaggtagt

SEQ ID NO: 122 - DNA, 24 bp, synthetic construct
  misc_feature 1..24: note = Description of Artificial Sequence: Synthetic oligonucleotide
  source 1..24: mol_type = other DNA
gtcctccccattggcctgcttcgt

SEQ ID NO: 123 - DNA, 24 bp, synthetic construct
  misc_feature 1..24: note = Description of Artificial Sequence: Synthetic oligonucleotide
  source 1..24: mol_type = other DNA
gttactcgcctgtcaagtggcgtg

SEQ ID NO: 124 - DNA, 24 bp, synthetic construct
  misc_feature 1..24: note = Description of Artificial Sequence: Synthetic oligonucleotide
  source 1..24: mol_type = other DNA
gttatgaacctgggtgaagtccca

SEQ ID NO: 125 - DNA, 24 bp, synthetic construct
  misc_feature 1..24: note = Description of Artificial Sequence: Synthetic oligonucleotide
  source 1..24: mol_type = other DNA
gttaatgttaataacttgcttcaa

SEQ ID NO: 126 - DNA, 24 bp, synthetic construct
  misc_feature 1..24: note = Description of Artificial Sequence: Synthetic oligonucleotide
  source 1..24: mol_type = other DNA
gttaaccaaggtcagaacattcac

SEQ ID NO: 127 - DNA, 24 bp, synthetic construct
  misc_feature 1..24: note = Description of Artificial Sequence: Synthetic oligonucleotide
  source 1..24: mol_type = other DNA
gttcccttagcactctgccactta

SEQ ID NO: 128 - DNA, 24 bp, synthetic construct
  misc_feature 1..24: note = Description of Artificial Sequence: Synthetic oligonucleotide
  source 1..24: mol_type = other DNA
gttcatttgtccagaggaaaccac

SEQ ID NO: 129 - DNA, 24 bp, synthetic construct
  misc_feature 1..24: note = Description of Artificial Sequence: Synthetic oligonucleotide
  source 1..24: mol_type = other DNA
gttccctgtcttgtttgtgagagg

SEQ ID NO: 130 - DNA, 24 bp, synthetic construct
  misc_feature 1..24: note = Description of Artificial Sequence: Synthetic oligonucleotide
  source 1..24: mol_type = other DNA
gttcaggacagactgcctccttcg

SEQ ID NO: 131 - DNA, 24 bp, synthetic construct
  misc_feature 1..24: note = Description of Artificial Sequence: Synthetic oligonucleotide
  source 1..24: mol_type = other DNA
gttggggattcctggtgccagaaa

SEQ ID NO: 132 - DNA, 24 bp, synthetic construct
  misc_feature 1..24: note = Description of Artificial Sequence: Synthetic oligonucleotide
  source 1..24: mol_type = other DNA
gttgggacttcacccaggttcata

SEQ ID NO: 133 - DNA, 24 bp, synthetic construct
  misc_feature 1..24: note = Description of Artificial Sequence: Synthetic oligonucleotide
  source 1..24: mol_type = other DNA
gttgagggcgttggagcggggaga

SEQ ID NO: 134 - DNA, 24 bp, synthetic construct
  misc_feature 1..24: note = Description of Artificial Sequence: Synthetic oligonucleotide
  source 1..24: mol_type = other DNA
gttgattggattgagaatagaatt

SEQ ID NO: 135 - DNA, 24 bp, synthetic construct
  misc_feature 1..24: note = Description of Artificial Sequence: Synthetic oligonucleotide
  source 1..24: mol_type = other DNA
gttgtgcagccgccgctccagagc

SEQ ID NO: 136 - DNA, 24 bp, synthetic construct
  misc_feature 1..24: note = Description of Artificial Sequence: Synthetic oligonucleotide
  source 1..24: mol_type = other DNA
gtttcctgatggtccatgtctgtt

SEQ ID NO: 137 - DNA, 24 bp, synthetic construct
  misc_feature 1..24: note = Description of Artificial Sequence: Synthetic oligonucleotide
  source 1..24: mol_type = other DNA
gtttgacttgggatagtggaatag

SEQ ID NO: 138 - DNA, 24 bp, synthetic construct
  misc_feature 1..24: note = Description of Artificial Sequence: Synthetic oligonucleotide
  source 1..24: mol_type = other DNA
gtttgggaggtcagaaataggggg

SEQ ID NO: 139 - DNA, 24 bp, synthetic construct
  misc_feature 1..24: note = Description of Artificial Sequence: Synthetic oligonucleotide
  source 1..24: mol_type = other DNA
gtttctcattagaaggagatgctc

SEQ ID NO: 140 - DNA, 24 bp, synthetic construct
  misc_feature 1..24: note = Description of Artificial Sequence: Synthetic oligonucleotide
  source 1..24: mol_type = other DNA
gtttcacctcggtgcagagatgcc

SEQ ID NO: 141 - DNA, 24 bp, synthetic construct
  misc_feature 1..24: note = Description of Artificial Sequence: Synthetic oligonucleotide
  source 1..24: mol_type = other DNA
tacatctctctttcttctcccctc

SEQ ID NO: 142 - DNA, 24 bp, synthetic construct
  misc_feature 1..24: note = Description of Artificial Sequence: Synthetic oligonucleotide
  source 1..24: mol_type = other DNA
tacaggcaaagctgagcaaaagta

SEQ ID NO: 143 - DNA, 24 bp, synthetic construct
  misc_feature 1..24: note = Description of Artificial Sequence: Synthetic oligonucleotide
  source 1..24: mol_type = other DNA
tacaaacggcagaagctggaggag

SEQ ID NO: 144 - DNA, 24 bp, synthetic construct
  misc_feature 1..24: note = Description of Artificial Sequence: Synthetic oligonucleotide
  source 1..24: mol_type = other DNA
tacaagaccagcatgtactcacct

SEQ ID NO: 145 - DNA, 24 bp, synthetic construct
  misc_feature 1..24: note = Description of Artificial Sequence: Synthetic oligonucleotide
  source 1..24: mol_type = other DNA
tacccacgttcgtggccccatctt

SEQ ID NO: 146 - DNA, 24 bp, synthetic construct
  misc_feature 1..24: note = Description of Artificial Sequence: Synthetic oligonucleotide
  source 1..24: mol_type = other DNA
taccagattctgagcagggagagg

SEQ ID NO: 147 - DNA, 24 bp, synthetic construct
  misc_feature 1..24: note = Description of Artificial Sequence: Synthetic oligonucleotide
  source 1..24: mol_type = other DNA
tacctcactggccccaccccagag

SEQ ID NO: 148 - DNA, 24 bp, synthetic construct
  misc_feature 1..24: note = Description of Artificial Sequence: Synthetic oligonucleotide
  source 1..24: mol_type = other DNA
tacctgcgccacatccatcggcgc

SEQ ID NO: 149 - DNA, 24 bp, synthetic construct
  misc_feature 1..24: note = Description of Artificial Sequence: Synthetic oligonucleotide
  source 1..24: mol_type = other DNA
tatagagttgattggattgagaat

SEQ ID NO: 150 - DNA, 24 bp, synthetic construct
  misc_feature 1..24: note = Description of Artificial Sequence: Synthetic oligonucleotide
  source 1..24: mol_type = other DNA
tatattcaagaaggttatctcaag

SEQ ID NO: 151 - DNA, 24 bp, synthetic construct
  misc_feature 1..24: note = Description of Artificial Sequence: Synthetic oligonucleotide
  source 1..24: mol_type = other DNA
tatatattcaagaaggttatctca

SEQ ID NO: 152 - DNA, 24 bp, synthetic construct
  misc_feature 1..24: note = Description of Artificial Sequence: Synthetic oligonucleotide
  source 1..24: mol_type = other DNA
tatagacatgtcccatttgtggga

SEQ ID NO: 153 - DNA, 24 bp, synthetic construct
  misc_feature 1..24: note = Description of Artificial Sequence: Synthetic oligonucleotide
  source 1..24: mol_type = other DNA
tatcgcctctccctgctcagaatc

SEQ ID NO: 154 - DNA, 24 bp, synthetic construct
  misc_feature 1..24: note = Description of Artificial Sequence: Synthetic oligonucleotide
  source 1..24: mol_type = other DNA
tatctcaagaaactggcttggaaa

SEQ ID NO: 155 - DNA, 24 bp, synthetic construct
  misc_feature 1..24: note = Description of Artificial Sequence: Synthetic oligonucleotide
  source 1..24: mol_type = other DNA
tatccagttcagtcaagtttgcct

SEQ ID NO: 156 - DNA, 24 bp, synthetic construct
  misc_feature 1..24: note = Description of Artificial Sequence: Synthetic oligonucleotide
  source 1..24: mol_type = other DNA
tatcccaagtcaaacttctcttca

SEQ ID NO: 157 - DNA, 24 bp, synthetic construct
  misc_feature 1..24: note = Description of Artificial Sequence: Synthetic oligonucleotide
  source 1..24: mol_type = other DNA
tatgttcgggtgctgtgaacttcc

SEQ ID NO: 158 - DNA, 24 bp, synthetic construct
  misc_feature 1..24: note = Description of Artificial Sequence: Synthetic oligonucleotide
  source 1..24: mol_type = other DNA
tatgaacctgggtgaagtcccaac

SEQ ID NO: 159 - DNA, 24 bp, synthetic construct
  misc_feature 1..24: note = Description of Artificial Sequence: Synthetic oligonucleotide
  source 1..24: mol_type = other DNA
tatgtagctgtttgggaggtcaga

SEQ ID NO: 160 - DNA, 24 bp, synthetic construct
  misc_feature 1..24: note = Description of Artificial Sequence: Synthetic oligonucleotide
  source 1..24: mol_type = other DNA
tatgggacattttcagaactccaa

SEQ ID NO: 161 - DNA, 24 bp, synthetic construct
  misc_feature 1..24: note = Description of Artificial Sequence: Synthetic oligonucleotide
  source 1..24: mol_type = other DNA
tattgggtcagctgttaacatcag

SEQ ID NO: 162 - DNA, 24 bp, synthetic construct
  misc_feature 1..24: note = Description of Artificial Sequence: Synthetic oligonucleotide
  source 1..24: mol_type = other DNA
tatttctgacctcccaaacagcta

SEQ ID NO: 163 - DNA, 24 bp, synthetic construct
  misc_feature 1..24: note = Description of Artificial Sequence: Synthetic oligonucleotide
  source 1..24: mol_type = other DNA
tattctcaatccaatcaactctat

SEQ ID NO: 164 - DNA, 24 bp, synthetic construct
  misc_feature 1..24: note = Description of Artificial Sequence: Synthetic oligonucleotide
  source 1..24: mol_type = other DNA
tattggtcgaaatgcatgtcaatc

SEQ ID NO: 165 - DNA, 24 bp, synthetic construct
  misc_feature 1..24: note = Description of Artificial Sequence: Synthetic oligonucleotide
  source 1..24: mol_type = other DNA
tccatgtctgttactcgcctgtca

SEQ ID NO: 166 - DNA, 24 bp, synthetic construct
  misc_feature 1..24: note = Description of Artificial Sequence: Synthetic oligonucleotide
  source 1..24: mol_type = other DNA
tccaggagacaggagcatctcctt

SEQ ID NO: 167 - DNA, 24 bp, synthetic construct
  misc_feature 1..24: note = Description of Artificial Sequence: Synthetic oligonucleotide
  source 1..24: mol_type = other DNA
tccagtcccaaatatgtagctgtt

SEQ ID NO: 168 - DNA, 24 bp, synthetic construct
  misc_feature 1..24: note = Description of Artificial Sequence: Synthetic oligonucleotide
  source 1..24: mol_type = other DNA
tccccagagggttctagacccaga

SEQ ID NO: 169 - DNA, 24 bp, synthetic construct
  misc_feature 1..24: note = Description of Artificial Sequence: Synthetic oligonucleotide
  source 1..24: mol_type = other DNA
tccccaaactctccagtctgttta

SEQ ID NO: 170 - DNA, 24 bp, synthetic construct
  misc_feature 1..24: note = Description of Artificial Sequence: Synthetic oligonucleotide
  source 1..24: mol_type = other DNA
tcccgtcacccctgtttctggcac

SEQ ID NO: 171 - DNA, 24 bp, synthetic construct
  misc_feature 1..24: note = Description of Artificial Sequence: Synthetic oligonucleotide
  source 1..24: mol_type = other DNA
tcccaggtgctgacgtaggtagtg

SEQ ID NO: 172 - DNA, 24 bp, synthetic construct
  misc_feature 1..24: note = Description of Artificial Sequence: Synthetic oligonucleotide
  source 1..24: mol_type = other DNA
tccctctttagccagagccggggt

SEQ ID NO: 173 - DNA, 24 bp, synthetic construct
  misc_feature 1..24: note = Description of Artificial Sequence: Synthetic oligonucleotide
  source 1..24: mol_type = other DNA
tccgtgaacgttcccttagcactc

SEQ ID NO: 174 - DNA, 24 bp, synthetic construct
  misc_feature 1..24: note = Description of Artificial Sequence: Synthetic oligonucleotide
  source 1..24: mol_type = other DNA
tccgagcttctggcggtctcaagc

SEQ ID NO: 175 - DNA, 24 bp, synthetic construct
  misc_feature 1..24: note = Description of Artificial Sequence: Synthetic oligonucleotide
  source 1..24: mol_type = other DNA
tccgcacgtaacctcactttcctg

SEQ ID NO: 176 - DNA, 24 bp, synthetic construct
  misc_feature 1..24: note = Description of Artificial Sequence: Synthetic oligonucleotide
  source 1..24: mol_type = other DNA
tcctgatggtccatgtctgttact

SEQ ID NO: 177 - DNA, 24 bp, synthetic construct
  misc_feature 1..24: note = Description of Artificial Sequence: Synthetic oligonucleotide
  source 1..24: mol_type = other DNA
tgcacacagcaggcctttggtcag

SEQ ID NO: 178 - DNA, 24 bp, synthetic construct
  misc_feature 1..24: note = Description of Artificial Sequence: Synthetic oligonucleotide
  source 1..24: mol_type = other DNA
tgcagaaagaagaaattcaatcct

SEQ ID NO: 179 - DNA, 24 bp, synthetic construct
  misc_feature 1..24: note = Description of Artificial Sequence: Synthetic oligonucleotide
  source 1..24: mol_type = other DNA
tgccacttattgggtcagctgtta

SEQ ID NO: 180 - DNA, 24 bp, synthetic construct
  misc_feature 1..24: note = Description of Artificial Sequence: Synthetic oligonucleotide
  source 1..24: mol_type = other DNA
tgcctcgcatcagcgtgatcagca

SEQ ID NO: 181 - DNA, 24 bp, synthetic construct
  misc_feature 1..24: note = Description of Artificial Sequence: Synthetic oligonucleotide
  source 1..24: mol_type = other DNA
tgcctccactggttgtgcagccgc

SEQ ID NO: 182 - DNA, 24 bp, synthetic construct
  misc_feature 1..24: note = Description of Artificial Sequence: Synthetic oligonucleotide
  source 1..24: mol_type = other DNA
tgccgaccaaagcgccgatggatg

SEQ ID NO: 183 - DNA, 24 bp, synthetic construct
  misc_feature 1..24: note = Description of Artificial Sequence: Synthetic oligonucleotide
  source 1..24: mol_type = other DNA
tgtaatgaaatggcagcttgtttc

SEQ ID NO: 184 - DNA, 24 bp, synthetic construct
  misc_feature 1..24: note = Description of Artificial Sequence: Synthetic oligonucleotide
  source 1..24: mol_type = other DNA
tgtactttgtcctccggttctgga

SEQ ID NO: 185 - DNA, 24 bp, synthetic construct
  misc_feature 1..24: note = Description of Artificial Sequence: Synthetic oligonucleotide
  source 1..24: mol_type = other DNA
tgtacctcaccactgacattaatt

SEQ ID NO: 186 - DNA, 24 bp, synthetic construct
  misc_feature 1..24: note = Description of Artificial Sequence: Synthetic oligonucleotide
  source 1..24: mol_type = other DNA
tgtaaccacagtcaagtagttaat

SEQ ID NO: 187 - DNA, 24 bp, synthetic construct
  misc_feature 1..24: note = Description of Artificial Sequence: Synthetic oligonucleotide
  source 1..24: mol_type = other DNA
tgtaaggtctcagttaggattgaa

SEQ ID NO: 188 - DNA, 24 bp, synthetic construct
  misc_feature 1..24: note = Description of Artificial Sequence: Synthetic oligonucleotide
  source 1..24: mol_type = other DNA
tgtcaatctcccagcgtctttatc

SEQ ID NO: 189 - DNA, 24 bp, synthetic construct
  misc_feature 1..24: note = Description of Artificial Sequence: Synthetic oligonucleotide
  source 1..24: mol_type = other DNA
tgtcttgtttgtgagaggaattca

SEQ ID NO: 190 - DNA, 24 bp, synthetic construct
  misc_feature 1..24: note = Description of Artificial Sequence: Synthetic oligonucleotide
  source 1..24: mol_type = other DNA
tgtccagaggaaaccactgttggg

SEQ ID NO: 191 - DNA, 24 bp, synthetic construct
  misc_feature 1..24: note = Description of Artificial Sequence: Synthetic oligonucleotide
  source 1..24: mol_type = other DNA
tgtctattccactatcccaagtca

SEQ ID NO: 192 - DNA, 24 bp, synthetic construct
  misc_feature 1..24: note = Description of Artificial Sequence: Synthetic oligonucleotide
  source 1..24: mol_type = other DNA
tgtccctcacccatctccctgtga

SEQ ID NO: 193 - DNA, 24 bp, synthetic construct
  misc_feature 1..24: note = Description of Artificial Sequence: Synthetic oligonucleotide
  source 1..24: mol_type = other DNA
tgtgcagccgccgctccagagccg

SEQ ID NO: 194 - DNA, 24 bp, synthetic construct
  misc_feature 1..24: note = Description of Artificial Sequence: Synthetic oligonucleotide
  source 1..24: mol_type = other DNA
tgtgagaggaattcaaactgaggc

SEQ ID NO: 195 - DNA, 24 bp, synthetic construct
  misc_feature 1..24: note = Description of Artificial Sequence: Synthetic oligonucleotide
  source 1..24: mol_type = other DNA
tgtggcgcaggtagcgcgcccact

SEQ ID NO: 196 - DNA, 24 bp, synthetic construct
  misc_feature 1..24: note = Description of Artificial Sequence: Synthetic oligonucleotide
  source 1..24: mol_type = other DNA
tgtggttccagaaccggaggacaa

SEQ ID NO: 197 - DNA, 24 bp, synthetic construct
  misc_feature 1..24: note = Description of Artificial Sequence: Synthetic oligonucleotide
  source 1..24: mol_type = other DNA
tgtgatgggagcccttcttcttct

SEQ ID NO: 198 - DNA, 24 bp, synthetic construct
  misc_feature 1..24: note = Description of Artificial Sequence: Synthetic oligonucleotide
  source 1..24: mol_type = other DNA
ttacaggcaaagctgagcaaaagt

SEQ ID NO: 199 - DNA, 24 bp, synthetic construct
  misc_feature 1..24: note = Description of Artificial Sequence: Synthetic oligonucleotide
  source 1..24: mol_type = other DNA
ttactcatctctgccagaccacct

SEQ ID NO: 200 - DNA, 24 bp, synthetic construct
  misc_feature 1..24: note = Description of Artificial Sequence: Synthetic oligonucleotide
  source 1..24: mol_type = other DNA
ttactgattctggggtcaacatct

SEQ ID NO: 201 - DNA, 24 bp, synthetic construct
  misc_feature 1..24: note = Description of Artificial Sequence: Synthetic oligonucleotide
  source 1..24: mol_type = other DNA
ttacaaatgaatggcatcgaagag

SEQ ID NO: 202 - DNA, 24 bp, synthetic construct
  misc_feature 1..24: note = Description of Artificial Sequence: Synthetic oligonucleotide
  source 1..24: mol_type = other DNA
ttacaccgtttctcattagaagga

SEQ ID NO: 203 - DNA, 24 bp, synthetic construct
  misc_feature 1..24: note = Description of Artificial Sequence: Synthetic oligonucleotide
  source 1..24: mol_type = other DNA
ttactagggcaataagcaacacct

SEQ ID NO: 204 - DNA, 24 bp, synthetic construct
  misc_feature 1..24: note = Description of Artificial Sequence: Synthetic oligonucleotide
  source 1..24: mol_type = other DNA
ttcagtctccgtgaacgttccctt

SEQ ID NO: 205 - DNA, 24 bp, synthetic construct
  misc_feature 1..24: note = Description of Artificial Sequence: Synthetic oligonucleotide
  source 1..24: mol_type = other DNA
ttcacccaggttcataacaatgtt

SEQ ID NO: 206 - DNA, 24 bp, synthetic construct
  misc_feature 1..24: note = Description of Artificial Sequence: Synthetic oligonucleotide
  source 1..24: mol_type = other DNA
ttcacccagcttccctgtggtggc

SEQ ID NO: 207 - DNA, 24 bp, synthetic construct
  misc_feature 1..24: note = Description of Artificial Sequence: Synthetic oligonucleotide
  source 1..24: mol_type = other DNA
ttcaatcctaactgagaccttaca

SEQ ID NO: 208 - DNA, 24 bp, synthetic construct
  misc_feature 1..24: note = Description of Artificial Sequence: Synthetic oligonucleotide
  source 1..24: mol_type = other DNA
ttcaccttggagacggcgactctc

SEQ ID NO: 209 - DNA, 24 bp, synthetic construct
  misc_feature 1..24: note = Description of Artificial Sequence: Synthetic oligonucleotide
  source 1..24: mol_type = other DNA
ttcctgatggtccatgtctgttac

SEQ ID NO: 210 - DNA, 24 bp, synthetic construct
  misc_feature 1..24: note = Description of Artificial Sequence: Synthetic oligonucleotide
  source 1..24: mol_type = other DNA
ttccctggcctacctcactggccc

SEQ ID NO: 211 - DNA, 24 bp, synthetic construct
  misc_feature 1..24: note = Description of Artificial Sequence: Synthetic oligonucleotide
  source 1..24: mol_type = other DNA
ttccaaagcccattccctctttag

SEQ ID NO: 212 - DNA, 24 bp, synthetic construct
  misc_feature 1..24: note = Description of Artificial Sequence: Synthetic oligonucleotide
  source 1..24: mol_type = other DNA
ttccattgtgcaaaagactccctt

SEQ ID NO: 213 - DNA, 24 bp, synthetic construct
  misc_feature 1..24: note = Description of Artificial Sequence: Synthetic oligonucleotide
  source 1..24: mol_type = other DNA
ttccgagcttctggcggtctcaag

SEQ ID NO: 214 - DNA, 24 bp, synthetic construct
  misc_feature 1..24: note = Description of Artificial Sequence: Synthetic oligonucleotide
  source 1..24: mol_type = other DNA
ttcgtggccccatctttctcaagg

SEQ ID NO: 215 - DNA, 24 bp, synthetic construct
  misc_feature 1..24: note = Description of Artificial Sequence: Synthetic oligonucleotide
  source 1..24: mol_type = other DNA
ttcgagagtgaggacgtgtgtgtc

SEQ ID NO: 216 - DNA, 24 bp, synthetic construct
  misc_feature 1..24: note = Description of Artificial Sequence: Synthetic oligonucleotide
  source 1..24: mol_type = other DNA
ttcggagcgaaaaccaagacaggt

SEQ ID NO: 217 - DNA, 24 bp, synthetic construct
  misc_feature 1..24: note = Description of Artificial Sequence: Synthetic oligonucleotide
  source 1..24: mol_type = other DNA
ttcgaccaatttagtgcagaaaga

SEQ ID NO: 218 - DNA, 24 bp, synthetic construct
  misc_feature 1..24: note = Description of Artificial Sequence: Synthetic oligonucleotide
  source 1..24: mol_type = other DNA
ttcgcacggctctggagcggcggc

SEQ ID NO: 219 - DNA, 24 bp, synthetic construct
  misc_feature 1..24: note = Description of Artificial Sequence: Synthetic oligonucleotide
  source 1..24: mol_type = other DNA
ttctgccctcccgtcacccctgtt

SEQ ID NO: 220 - DNA, 24 bp, synthetic construct
  misc_feature 1..24: note = Description of Artificial Sequence: Synthetic oligonucleotide
  source 1..24: mol_type = other DNA
ttctgccctttactcatctctgcc

SEQ ID NO: 221 - DNA, 24 bp, synthetic construct
  misc_feature 1..24: note = Description of Artificial Sequence: Synthetic oligonucleotide
  source 1..24: mol_type = other DNA
ttctgacctcccaaacagctacat

SEQ ID NO: 222 - DNA, 24 bp, synthetic construct
  misc_feature 1..24: note = Description of Artificial Sequence: Synthetic oligonucleotide
  source 1..24: mol_type = other DNA
ttctttcgaccaatttagtgcaga

SEQ ID NO: 223 - DNA, 24 bp, synthetic construct
  misc_feature 1..24: note = Description of Artificial Sequence: Synthetic oligonucleotide
  source 1..24: mol_type = other DNA
ttctggcggtctcaagcactacct

SEQ ID NO: 224 - DNA, 24 bp, synthetic construct
  misc_feature 1..24: note = Description of Artificial Sequence: Synthetic oligonucleotide
  source 1..24: mol_type = other DNA
tttatttcccttcagctaaaataa

SEQ ID NO: 225 - DNA, 24 bp, synthetic construct
  misc_feature 1..24: note = Description of Artificial Sequence: Synthetic oligonucleotide
  source 1..24: mol_type = other DNA
tttattttagctgaagggaaataa

SEQ ID NO: 226 - DNA, 24 bp, synthetic construct
  misc_feature 1..24: note = Description of Artificial Sequence: Synthetic oligonucleotide
  source 1..24: mol_type = other DNA
tttatccgtgttccttgactctgg

SEQ ID NO: 227 - DNA, 24 bp, synthetic construct
  misc_feature 1..24: note = Description of Artificial Sequence: Synthetic oligonucleotide
  source 1..24: mol_type = other DNA
tttaccttcggagcgaaaaccaag

SEQ ID NO: 228 - DNA, 24 bp, synthetic construct
  misc_feature 1..24: note = Description of Artificial Sequence: Synthetic oligonucleotide
  source 1..24: mol_type = other DNA
tttaggatgccactaaaagggaaa

SEQ ID NO: 229 - DNA, 24 bp, synthetic construct
  misc_feature 1..24: note = Description of Artificial Sequence: Synthetic oligonucleotide
  source 1..24: mol_type = other DNA
tttagattgaaggaaaagttacaa

SEQ ID NO: 230 - DNA, 24 bp, synthetic construct
  misc_feature 1..24: note = Description of Artificial Sequence: Synthetic oligonucleotide
  source 1..24: mol_type = other DNA
tttccctcactcctgctcggtgaa

SEQ ID NO: 231 - DNA, 24 bp, synthetic construct
  misc_feature 1..24: note = Description of Artificial Sequence: Synthetic oligonucleotide
  source 1..24: mol_type = other DNA
tttcctgatggtccatgtctgtta

SEQ ID NO: 232 - DNA, 24 bp, synthetic construct
  misc_feature 1..24: note = Description of Artificial Sequence: Synthetic oligonucleotide
  source 1..24: mol_type = other DNA
tttctcatctgtgcccctccctcc

SEQ ID NO: 233 - DNA, 24 bp, synthetic construct
  misc_feature 1..24: note = Description of Artificial Sequence: Synthetic oligonucleotide
  source 1..24: mol_type = other DNA
tttcaccttggagacggcgactct

SEQ ID NO: 234 - DNA, 24 bp, synthetic construct
  misc_feature 1..24: note = Description of Artificial Sequence: Synthetic oligonucleotide
  source 1..24: mol_type = other DNA
tttcgctccgaaggtaaaagaaat

SEQ ID NO: 235 - DNA, 24 bp, synthetic construct
  misc_feature 1..24: note = Description of Artificial Sequence: Synthetic oligonucleotide
  source 1..24: mol_type = other DNA
tttcagcctcacccctctagccct

SEQ ID NO: 236 - DNA, 24 bp, synthetic construct
  misc_feature 1..24: note = Description of Artificial Sequence: Synthetic oligonucleotide
  source 1..24: mol_type = other DNA
tttcttctcccctctgctggatac

SEQ ID NO: 237 - DNA, 24 bp, synthetic construct
  misc_feature 1..24: note = Description of Artificial Sequence: Synthetic oligonucleotide
  source 1..24: mol_type = other DNA
tttccgagcttctggcggtctcaa

SEQ ID NO: 238 - DNA, 24 bp, synthetic construct
  misc_feature 1..24: note = Description of Artificial Sequence: Synthetic oligonucleotide
  source 1..24: mol_type = other DNA
tttgaggagtgttcagtctccgtg

SEQ ID NO: 239 - DNA, 24 bp, synthetic construct
  misc_feature 1..24: note = Description of Artificial Sequence: Synthetic oligonucleotide
  source 1..24: mol_type = other DNA
tttggctcagcaggcacctgcctc

SEQ ID NO: 240 - DNA, 24 bp, synthetic construct
  misc_feature 1..24: note = Description of Artificial Sequence: Synthetic oligonucleotide
  source 1..24: mol_type = other DNA
tttgtcctccggttctggaaccac

SEQ ID NO: 241 - DNA, 24 bp, synthetic construct
  misc_feature 1..24: note = Description of Artificial Sequence: Synthetic oligonucleotide
  source 1..24: mol_type = other DNA
tttgtggttgcccaccctagtcat

SEQ ID NO: 242 - DNA, 24 bp, synthetic construct
  misc_feature 1..24: note = Description of Artificial Sequence: Synthetic oligonucleotide
  source 1..24: mol_type = other DNA
tttgtactttgtcctccggttctg

SEQ ID NO: 243 - DNA, 24 bp, synthetic construct
  misc_feature 1..24: note = Description of Artificial Sequence: Synthetic oligonucleotide
  source 1..24: mol_type = other DNA
tttgggcggggtccagttccggga

SEQ ID NO: 244 - DNA, 24 bp, synthetic construct
  misc_feature 1..24: note = Description of Artificial Sequence: Synthetic oligonucleotide
  source 1..24: mol_type = other DNA
tttggtcggcatggccccattcgc

SEQ ID NO: 245 - DNA, 24 bp, synthetic construct
  misc_feature 1..24: note = Description of Artificial Sequence: Synthetic oligonucleotide
  source 1..24: mol_type = other DNA
ttttatttcccttcagctaaaata

SEQ ID NO: 246 - DNA, 24 bp, synthetic construct
  misc_feature 1..24: note = Description of Artificial Sequence: Synthetic oligonucleotide
  source 1..24: mol_type = other DNA
ttttcaggaggaagcgatggcttc

SEQ ID NO: 247 - DNA, 24 bp, synthetic construct
  misc_feature 1..24: note = Description of Artificial Sequence: Synthetic oligonucleotide
  source 1..24: mol_type = other DNA
ttttccgagcttctggcggtctca

SEQ ID NO: 248 - DNA, 24 bp, synthetic construct
  misc_feature 1..24: note = Description of Artificial Sequence: Synthetic oligonucleotide
  source 1..24: mol_type = other DNA
ttttcgtatagagttgattggatt

SEQ ID NO: 249 - DNA, 24 bp, synthetic construct
  misc_feature 1..24: note = Description of Artificial Sequence: Synthetic oligonucleotide
  source 1..24: mol_type = other DNA
ttttgagctaaagtctggctgtag

SEQ ID NO: 250 - DNA, 24 bp, synthetic construct
  misc_feature 1..24: note = Description of Artificial Sequence: Synthetic oligonucleotide
  source 1..24: mol_type = other DNA
tttgagagtctggatgagaaatgc

SEQ ID NO: 251 - DNA, 24 bp, synthetic construct
  misc_feature 1..24: note = Description of Artificial Sequence: Synthetic oligonucleotide
  source 1..24: mol_type = other DNA
tttctaccctcttctctgcctttc

SEQ ID NO: 252 - DNA, 24 bp, synthetic construct
  misc_feature 1..24: note = Description of Artificial Sequence: Synthetic oligonucleotide
  source 1..24: mol_type = other DNA
tttgctctaggaaccctcagcccc

SEQ ID NO: 253 - DNA, 24 bp, synthetic construct
  misc_feature 1..24: note = Description of Artificial Sequence: Synthetic oligonucleotide
  source 1..24: mol_type = other DNA
tttctccaaagccactaggcaggc

SEQ ID NO: 254 - DNA, 24 bp, synthetic construct
  misc_feature 1..24: note = Description of Artificial Sequence: Synthetic oligonucleotide
  source 1..24: mol_type = other DNA
tttaggaaagcaggagctattcag

SEQ ID NO: 255 - DNA, 24 bp, synthetic construct
  misc_feature 1..24: note = Description of Artificial Sequence: Synthetic oligonucleotide
  source 1..24: mol_type = other DNA
tttggaaccaaatttggtgagtgc

SEQ ID NO: 256 - DNA, 24 bp, synthetic construct
  misc_feature 1..24: note = Description of Artificial Sequence: Synthetic oligonucleotide
  source 1..24: mol_type = other DNA
attcaggaagcaggggtcctccag

SEQ ID NO: 257 - DNA, 24 bp, synthetic construct
  misc_feature 1..24: note = Description of Artificial Sequence: Synthetic oligonucleotide
  source 1..24: mol_type = other DNA
attgggctttggaaccaaatttgg

SEQ ID NO: 258 - DNA, 24 bp, synthetic construct
  misc_feature 1..24: note = Description of Artificial Sequence: Synthetic oligonucleotide
  source 1..24: mol_type = other DNA
attccgtcatagggatagatcggg

SEQ ID NO: 259 - DNA, 24 bp, synthetic construct
  misc_feature 1..24: note = Description of Artificial Sequence: Synthetic oligonucleotide
  source 1..24: mol_type = other DNA
cttgtttctccaaagccactaggc

SEQ ID NO: 260 - DNA, 24 bp, synthetic construct
  misc_feature 1..24: note = Description of Artificial Sequence: Synthetic oligonucleotide
  source 1..24: mol_type = other DNA
cttcctgaatagctcctgctttcc

SEQ ID NO: 261 - DNA, 24 bp, synthetic construct
  misc_feature 1..24: note = Description of Artificial Sequence: Synthetic oligonucleotide
  source 1..24: mol_type = other DNA
cttatcagtcctgaaaagaacccc

SEQ ID NO: 262 - DNA, 24 bp, synthetic construct
  misc_feature 1..24: note = Description of Artificial Sequence: Synthetic oligonucleotide
  source 1..24: mol_type = other DNA
gttgcatttgctctccacctccca

SEQ ID NO: 263 - DNA, 24 bp, synthetic construct
  misc_feature 1..24: note = Description of Artificial Sequence: Synthetic oligonucleotide
  source 1..24: mol_type = other DNA
gttagcgcgcggtgaggggagggg

SEQ ID NO: 264 - DNA, 24 bp, synthetic construct
  misc_feature 1..24: note = Description of Artificial Sequence: Synthetic oligonucleotide
  source 1..24: mol_type = other DNA
gttccaaagcccaatctaaaaaac

SEQ ID NO: 265 - DNA, 24 bp, synthetic construct
  misc_feature 1..24: note = Description of Artificial Sequence: Synthetic oligonucleotide
  source 1..24: mol_type = other DNA
ttcaggaagcaggggtcctccagg

SEQ ID NO: 266 - DNA, 24 bp, synthetic construct
  misc_feature 1..24: note = Description of Artificial Sequence: Synthetic oligonucleotide
  source 1..24: mol_type = other DNA
ttcctggaggccagcactcaccaa

SEQ ID NO: 267 - DNA, 24 bp, synthetic construct
  misc_feature 1..24: note = Description of Artificial Sequence: Synthetic oligonucleotide
  source 1..24: mol_type = other DNA
ttcaggactgataagagcgcgcag

SEQ ID NO: 268 - DNA, 24 bp, synthetic construct
  misc_feature 1..24: note = Description of Artificial Sequence: Synthetic oligonucleotide
  source 1..24: mol_type = other DNA
ctccaaagccactaggcaggcgtt

SEQ ID NO: 269 - DNA, 24 bp, synthetic construct
  misc_feature 1..24: note = Description of Artificial Sequence: Synthetic oligonucleotide
  source 1..24: mol_type = other DNA
ctccaggaaatctggagccctggc

SEQ ID NO: 270 - DNA, 24 bp, synthetic construct
  misc_feature 1..24: note = Description of Artificial Sequence: Synthetic oligonucleotide
  source 1..24: mol_type = other DNA
ctccctccctcgcctccaccctgt

SEQ ID NO: 271 - DNA, 24 bp, synthetic construct
  misc_feature 1..24: note = Description of Artificial Sequence: Synthetic oligonucleotide
  source 1..24: mol_type = other DNA
tcccgcccccaccgggccggcctc

SEQ ID NO: 272 - DNA, 24 bp, synthetic construct
  misc_feature 1..24: note = Description of Artificial Sequence: Synthetic oligonucleotide
  source 1..24: mol_type = other DNA
tcccctcaccgcgcgctaacgcct

SEQ ID NO: 273 - DNA, 24 bp, synthetic construct
  misc_feature 1..24: note = Description of Artificial Sequence: Synthetic oligonucleotide
  source 1..24: mol_type = other DNA
tccctcgcctccaccctgttggtt

SEQ ID NO: 274 - DNA, 24 bp, synthetic construct
  misc_feature 1..24: note = Description of Artificial Sequence: Synthetic oligonucleotide
  source 1..24: mol_type = other DNA
tttgtactgatggtatggggccaa

SEQ ID NO: 275 - DNA, 24 bp, synthetic construct
  misc_feature 1..24: note = Description of Artificial Sequence: Synthetic oligonucleotide
  source 1..24: mol_type = other DNA
tttgaagtccaactcctaagccag

SEQ ID NO: 276 - DNA, 24 bp, synthetic construct
  misc_feature 1..24: note = Description of Artificial Sequence: Synthetic oligonucleotide
  source 1..24: mol_type = other DNA
tttgcaagtgtatttacgtaatat

SEQ ID NO: 277 - DNA, 24 bp, synthetic construct
  misc_feature 1..24: note = Description of Artificial Sequence: Synthetic oligonucleotide
  source 1..24: mol_type = other DNA
attggccaaccctagggtgtggct

SEQ ID NO: 278 - DNA, 24 bp, synthetic construct
  misc_feature 1..24: note = Description of Artificial Sequence: Synthetic oligonucleotide
  source 1..24: mol_type = other DNA
attgctactaaaaacatcctcctt

SEQ ID NO: 279 - DNA, 24 bp, synthetic construct
  misc_feature 1..24: note = Description of Artificial Sequence: Synthetic oligonucleotide
  source 1..24: mol_type = other DNA
attgggaaaacgatcttcaatatg

SEQ ID NO: 280 - DNA, 24 bp, synthetic construct
  misc_feature 1..24: note = Description of Artificial Sequence: Synthetic oligonucleotide
  source 1..24: mol_type = other DNA
cttagacctcaccctgtggagcca

SEQ ID NO: 281 - DNA, 24 bp, synthetic construct
  misc_feature 1..24: note = Description of Artificial Sequence: Synthetic oligonucleotide
  source 1..24: mol_type = other DNA
cttaggagttggacttcaaaccct

SEQ ID NO: 282 - DNA, 24 bp, synthetic construct
  misc_feature 1..24: note = Description of Artificial Sequence: Synthetic oligonucleotide
  source 1..24: mol_type = other DNA
cttaccaagctgtgattccaaata

SEQ ID NO: 283 - DNA, 24 bp, synthetic construct
  misc_feature 1..24: note = Description of Artificial Sequence: Synthetic oligonucleotide
  source 1..24: mol_type = other DNA
tatgcccagccctggctcctgccc

SEQ ID NO: 284 - DNA, 24 bp, synthetic construct
  misc_feature 1..24: note = Description of Artificial Sequence: Synthetic oligonucleotide
  source 1..24: mol_type = other DNA
tatctcttggccccataccatcag

SEQ ID NO: 285 - DNA, 24 bp, synthetic construct
  misc_feature 1..24: note = Description of Artificial Sequence: Synthetic oligonucleotide
  source 1..24: mol_type = other DNA
tatcccaaagctgaattatggtag

SEQ ID NO: 286 - DNA, 24 bp, synthetic construct
  misc_feature 1..24: note = Description of Artificial Sequence: Synthetic oligonucleotide
  source 1..24: mol_type = other DNA
tgtcatcacttagacctcaccctg

SEQ ID NO: 287 - DNA, 24 bp, synthetic construct
  misc_feature 1..24: note = Description of Artificial Sequence: Synthetic oligonucleotide
  source 1..24: mol_type = other DNA
tgtactgatggtatggggccaaga

SEQ ID NO: 288 - DNA, 24 bp, synthetic construct
  misc_feature 1..24: note = Description of Artificial Sequence: Synthetic oligonucleotide
  source 1..24: mol_type = other DNA
tgtagatggatctcttcctgcgtc

SEQ ID NO: 289 - DNA, 24 bp, synthetic construct
  misc_feature 1..24: note = Description of Artificial Sequence: Synthetic oligonucleotide
  source 1..24: mol_type = other DNA
ttcaaaccctcagccctccctcta

SEQ ID NO: 290 - DNA, 24 bp, synthetic construct
  misc_feature 1..24: note = Description of Artificial Sequence: Synthetic oligonucleotide
  source 1..24: mol_type = other DNA
ttccaaatattacgtaaatacact

SEQ ID NO: 291 - DNA, 24 bp, synthetic construct
  misc_feature 1..24: note = Description of Artificial Sequence: Synthetic oligonucleotide
  source 1..24: mol_type = other DNA
ttcagctttgggatatgtagatgg

SEQ ID NO: 292 - DNA, 24 bp, synthetic construct
  misc_feature 1..24: note = Description of Artificial Sequence: Synthetic oligonucleotide
  source 1..24: mol_type = other DNA
ctccctgctcctgggagtagattg

SEQ ID NO: 293 - DNA, 24 bp, synthetic construct
  misc_feature 1..24: note = Description of Artificial Sequence: Synthetic oligonucleotide
  source 1..24: mol_type = other DNA
ctccctctaagatatatctcttgg

SEQ ID NO: 294 - DNA, 24 bp, synthetic construct
  misc_feature 1..24: note = Description of Artificial Sequence: Synthetic oligonucleotide
  source 1..24: mol_type = other DNA
ctccagaatatgcaaaatacttac

SEQ ID NO: 295 - DNA, 24 bp, synthetic construct
  misc_feature 1..24: note = Description of Artificial Sequence: Synthetic oligonucleotide
  source 1..24: mol_type = other DNA
tacctgtccttggctcttctggca

SEQ ID NO: 296 - DNA, 24 bp, synthetic construct
  misc_feature 1..24: note = Description of Artificial Sequence: Synthetic oligonucleotide
  source 1..24: mol_type = other DNA
taccatcagtacaaattgctacta

SEQ ID NO: 297 - DNA, 24 bp, synthetic construct
  misc_feature 1..24: note = Description of Artificial Sequence: Synthetic oligonucleotide
  source 1..24: mol_type = other DNA
taccataattcagctttgggatat

SEQ ID NO: 298 - DNA, 24 bp, synthetic construct
  misc_feature 1..24: note = Description of Artificial Sequence: Synthetic oligonucleotide
  source 1..24: mol_type = other DNA
tttcaagcctcgggaaactgccct

SEQ ID NO: 299 - DNA, 24 bp, synthetic construct
  misc_feature 1..24: note = Description of Artificial Sequence: Synthetic oligonucleotide
  source 1..24: mol_type = other DNA
tttctttgtttgcaggtcagtgcc

SEQ ID NO: 300 - DNA, 24 bp, synthetic construct
  misc_feature 1..24: note = Description of Artificial Sequence: Synthetic oligonucleotide
  source 1..24: mol_type = other DNA
tttgggctggcgctcgagctctcc

SEQ ID NO: 301 - DNA, 24 bp, synthetic construct
  misc_feature 1..24: note = Description of Artificial Sequence: Synthetic oligonucleotide
  source 1..24: mol_type = other DNA
attcctggtttgggctggcgctcg

SEQ ID NO: 302 - DNA, 24 bp, synthetic construct
  misc_feature 1..24: note = Description of Artificial Sequence: Synthetic oligonucleotide
  source 1..24: mol_type = other DNA
attagtgccattattgtggcgaat

SEQ ID NO: 303 - DNA, 24 bp, synthetic construct
  misc_feature 1..24: note = Description of Artificial Sequence: Synthetic oligonucleotide
  source 1..24: mol_type = other DNA
attctcggcactggcgtgagagtt

SEQ ID NO: 304 - DNA, 24 bp, synthetic construct
  misc_feature 1..24: note = Description of Artificial Sequence: Synthetic oligonucleotide
  source 1..24: mol_type = other DNA
cttccccggagtcgaggactgtgg

SEQ ID NO: 305 - DNA, 24 bp, synthetic construct
  misc_feature 1..24: note = Description of Artificial Sequence: Synthetic oligonucleotide
  source 1..24: mol_type = other DNA
cttcggccacaagatggcactgac

SEQ ID NO: 306 - DNA, 24 bp, synthetic construct
  misc_feature 1..24: note = Description of Artificial Sequence: Synthetic oligonucleotide
  source 1..24: mol_type = other DNA
cttataaagtgaggaaaacaaatt

SEQ ID NO: 307 - DNA, 24 bp, synthetic construct
  misc_feature 1..24: note = Description of Artificial Sequence: Synthetic oligonucleotide
  source 1..24: mol_type = other DNA
ttccccggagtcgaggactgtggg

SEQ ID NO: 308 - DNA, 24 bp, synthetic construct
  misc_feature 1..24: note = Description of Artificial Sequence: Synthetic oligonucleotide
  source 1..24: mol_type = other DNA
ttcggccacaagatggcactgacc

SEQ ID NO: 309 - DNA, 24 bp, synthetic construct
  misc_feature 1..24: note = Description of Artificial Sequence: Synthetic oligonucleotide
  source 1..24: mol_type = other DNA
ttcccagcgagccctttgattcct

SEQ ID NO: 310 - DNA, 24 bp, synthetic construct
  misc_feature 1..24: note = Description of Artificial Sequence: Synthetic oligonucleotide
  source 1..24: mol_type = other DNA
ctccggggaaggcagggcagtttc

SEQ ID NO: 311 - DNA, 24 bp, synthetic construct
  misc_feature 1..24: note = Description of Artificial Sequence: Synthetic oligonucleotide
  source 1..24: mol_type = other DNA
ctccagccgggtatgacttcggcc

SEQ ID NO: 312 - DNA, 24 bp, synthetic construct
  misc_feature 1..24: note = Description of Artificial Sequence: Synthetic oligonucleotide
  source 1..24: mol_type = other DNA
ctcctttctttggcccactgagaa

SEQ ID NO: 313 - DNA, 24 bp, synthetic construct
  misc_feature 1..24: note = Description of Artificial Sequence: Synthetic oligonucleotide
  source 1..24: mol_type = other DNA
tttcaggctgtgaaccttggtggg

SEQ ID NO: 314 - DNA, 24 bp, synthetic construct
  misc_feature 1..24: note = Description of Artificial Sequence: Synthetic oligonucleotide
  source 1..24: mol_type = other DNA
tttcctgctccctcctcgccaatg

SEQ ID NO: 315 - DNA, 24 bp, synthetic construct
  misc_feature 1..24: note = Description of Artificial Sequence: Synthetic oligonucleotide
  source 1..24: mol_type = other DNA
tttgctaggaatattgaagggggc

SEQ ID NO: 316 - DNA, 24 bp, synthetic construct
  misc_feature 1..24: note = Description of Artificial Sequence: Synthetic oligonucleotide
  source 1..24: mol_type = other DNA
attgcggcgggctgcgggccaggc

SEQ ID NO: 317 - DNA, 24 bp, synthetic construct
  misc_feature 1..24: note = Description of Artificial Sequence: Synthetic oligonucleotide
  source 1..24: mol_type = other DNA
attacccatccgcccccggaaact

SEQ ID NO: 318 - DNA, 24 bp, synthetic construct
  misc_feature 1..24: note = Description of Artificial Sequence: Synthetic oligonucleotide
  source 1..24: mol_type = other DNA
attcctagcaaagagggaacggct

SEQ ID NO: 319 - DNA, 24 bp, synthetic construct
  misc_feature 1..24: note = Description of Artificial Sequence: Synthetic oligonucleotide
  source 1..24: mol_type = other DNA
cttccccttcattgcggcgggctg

SEQ ID NO: 320 - DNA, 24 bp, synthetic construct
  misc_feature 1..24: note = Description of Artificial Sequence: Synthetic oligonucleotide
  source 1..24: mol_type = other DNA
cttccccttcattgcggcgggctg

SEQ ID NO: 321 - DNA, 24 bp, synthetic construct
  misc_feature 1..24: note = Description of Artificial Sequence: Synthetic oligonucleotide
  source 1..24: mol_type = other DNA
cttcccctgcccccttcaatattc

SEQ ID NO: 322 - DNA, 24 bp, synthetic construct
  misc_feature 1..24: note = Description of Artificial Sequence: Synthetic oligonucleotide
  source 1..24: mol_type = other DNA
gttcacagcctgaaaattacccat

SEQ ID NO: 323 - DNA, 24 bp, synthetic construct
  misc_feature 1..24: note = Description of Artificial Sequence: Synthetic oligonucleotide
  source 1..24: mol_type = other DNA
gttacgtgcggacagggcctgaga

SEQ ID NO: 324 - DNA, 24 bp, synthetic construct
  misc_feature 1..24: note = Description of Artificial Sequence: Synthetic oligonucleotide
  source 1..24: mol_type = other DNA
gttggagcggggagaaggccaggg

SEQ ID NO: 325 - DNA, 24 bp, synthetic construct
  misc_feature 1..24: note = Description of Artificial Sequence: Synthetic oligonucleotide
  source 1..24: mol_type = other DNA
ttccacacgcggctcgggcccggg

SEQ ID NO: 326 - DNA, 24 bp, synthetic construct
  misc_feature 1..24: note = Description of Artificial Sequence: Synthetic oligonucleotide
  source 1..24: mol_type = other DNA
ttcaggctgtgaaccttggtgggg

SEQ ID NO: 327 - DNA, 24 bp, synthetic construct
  misc_feature 1..24: note = Description of Artificial Sequence: Synthetic oligonucleotide
  source 1..24: mol_type = other DNA
ttcctgctccctcctcgccaatgc

SEQ ID NO: 328 - DNA, 24 bp, synthetic construct
  misc_feature 1..24: note = Description of Artificial Sequence: Synthetic oligonucleotide
  source 1..24: mol_type = other DNA
ttccccttcattgcggcgggctgc

SEQ ID NO: 329 - DNA, 24 bp, synthetic construct
  misc_feature 1..24: note = Description of Artificial Sequence: Synthetic oligonucleotide
  source 1..24: mol_type = other DNA
ttcccctgcccccttcaatattcc

SEQ ID NO: 330 - DNA, 24 bp, synthetic construct
  misc_feature 1..24: note = Description of Artificial Sequence: Synthetic oligonucleotide
  source 1..24: mol_type = other DNA
tccccttcattgcggcgggctgcg

SEQ ID NO: 331 - DNA, 24 bp, synthetic construct
  misc_feature 1..24: note = Description of Artificial Sequence: Synthetic oligonucleotide
  source 1..24: mol_type = other DNA
tccctcctcgccaatgccccgcgg

SEQ ID NO: 332 - DNA, 24 bp, synthetic construct
  misc_feature 1..24: note = Description of Artificial Sequence: Synthetic oligonucleotide
  source 1..24: mol_type = other DNA
tcccctgcccccttcaatattcct

SEQ ID NO: 333 - DNA, 24 bp, synthetic construct
  misc_feature 1..24: note = Description of Artificial Sequence: Synthetic oligonucleotide
  source 1..24: mol_type = other DNA
ctcctcgccaatgccccgcgggcg

SEQ ID NO: 334 - DNA, 24 bp, synthetic construct
  misc_feature 1..24: note = Description of Artificial Sequence: Synthetic oligonucleotide
  source 1..24: mol_type = other DNA
ctccctcctcgccaatgccccgcg

SEQ ID NO: 335 - DNA, 24 bp, synthetic construct
  misc_feature 1..24: note = Description of Artificial Sequence: Synthetic oligonucleotide
  source 1..24: mol_type = other DNA
ctccaggattccaatagatctgtg

SEQ ID NO: 336 - DNA, 23 bp, synthetic construct
  misc_feature 1..23: note = Description of Artificial Sequence: Synthetic oligonucleotide
  source 1..23: mol_type = other DNA
agggtgtgcagacggcagtcact

SEQ ID NO: 337 - DNA, 23 bp, synthetic construct
  misc_feature 1..23: note = Description of Artificial Sequence: Synthetic oligonucleotide
  source 1..23: mol_type = other DNA
agggagcagcgtcttcgagagtg

SEQ ID NO: 338 - DNA, 23 bp, synthetic construct
  misc_feature 1..23: note = Description of Artificial Sequence: Synthetic oligonucleotide
  source 1..23: mol_type = other DNA
tggggtgagtgagtgtgtgcgtg

SEQ ID NO: 339 - DNA, 23 bp, synthetic construct
  misc_feature 1..23: note = Description of Artificial Sequence: Synthetic oligonucleotide
  source 1..23: mol_type = other DNA
aggggggcggatgggtaattttc

SEQ ID NO: 340 - DNA, 23 bp, synthetic construct
  misc_feature 1..23: note = Description of Artificial Sequence: Synthetic oligonucleotide
  source 1..23: mol_type = other DNA
aggggcattggcgaggagggagc

SEQ ID NO: 341 - DNA, 23 bp, synthetic construct
  misc_feature 1..23: note = Description of Artificial Sequence: Synthetic oligonucleotide
  source 1..23: mol_type = other DNA
agggcaaagagggaacggctctc

SEQ ID NO: 342 - DNA, 24 bp, synthetic construct
  misc_feature 1..24: note = Description of Artificial Sequence: Synthetic oligonucleotide
  source 1..24: mol_type = other DNA
tttatccgtgttccttgactctgg

SEQ ID NO: 343 - DNA, 24 bp, synthetic construct
  misc_feature 1..24: note = Description of Artificial Sequence: Synthetic oligonucleotide
  source 1..24: mol_type = other DNA
tttccctcactcctgctcggtgaa

SEQ ID NO: 344 - DNA, 24 bp, synthetic construct
  misc_feature 1..24: note = Description of Artificial Sequence: Synthetic oligonucleotide
  source 1..24: mol_type = other DNA
tttctcatctgtgcccctccctcc

SEQ ID NO: 345 - DNA, 24 bp, synthetic construct
  misc_feature 1..24: note = Description of Artificial Sequence: Synthetic oligonucleotide
  source 1..24: mol_type = other DNA
tttcagcctcacccctctagccct

SEQ ID NO: 346 - DNA, 24 bp, synthetic construct
  misc_feature 1..24: note = Description of Artificial Sequence: Synthetic oligonucleotide
  source 1..24: mol_type = other DNA
tttcttctcccctctgctggatac

SEQ ID NO: 347 - DNA, 24 bp, synthetic construct
  misc_feature 1..24: note = Description of Artificial Sequence: Synthetic oligonucleotide
  source 1..24: mol_type = other DNA
tttccgagcttctggcggtctcaa

SEQ ID NO: 348 - DNA, 24 bp, synthetic construct
  misc_feature 1..24: note = Description of Artificial Sequence: Synthetic oligonucleotide
  source 1..24: mol_type = other DNA
tttgtggttgcccaccctagtcat

SEQ ID NO: 349 - DNA, 24 bp, synthetic construct
  misc_feature 1..24: note = Description of Artificial Sequence: Synthetic oligonucleotide
  source 1..24: mol_type = other DNA
tttggtcggcatggccccattcgc

SEQ ID NO: 350 - DNA, 23 bp, synthetic construct
  misc_feature 1..23: note = Description of Artificial Sequence: Synthetic primer
  source 1..23: mol_type = other DNA
ccagaatgcacaaagtactgcac

SEQ ID NO: 351 - DNA, 21 bp, synthetic construct
  misc_feature 1..21: note = Description of Artificial Sequence: Synthetic primer
  source 1..21: mol_type = other DNA
gccaaagcccgagagagtgcc

SEQ ID NO: 352 - DNA, 27 bp, synthetic construct
  misc_feature 1..27: note = Description of Artificial Sequence: Synthetic primer
  source 1..27: mol_type = other DNA
gctgtgtctgtaaactgatggctaaca

SEQ ID NO: 353 - DNA, 29 bp, synthetic construct
  misc_feature 1..29: note = Description of Artificial Sequence: Synthetic primer
  source 1..29: mol_type = other DNA
ttgcattctactcaattgcattctgtggg

SEQ ID NO: 354 - DNA, 20 bp, synthetic construct
  misc_feature 1..20: note = Description of Artificial Sequence: Synthetic primer
  source 1..20: mol_type = other DNA
ggagcagctggtcagagggg

SEQ ID NO: 355 - DNA, 22 bp, synthetic construct
  misc_feature 1..22: note = Description of Artificial Sequence: Synthetic primer
  source 1..22: mol_type = other DNA
ccatagggaagggggacactgg

SEQ ID NO: 356 - DNA, 28 bp, synthetic construct
  misc_feature 1..28: note = Description of Artificial Sequence: Synthetic primer
  source 1..28: mol_type = other DNA
ctgcctcctattcatacacacttacggg

SEQ ID NO: 357 - DNA, 25 bp, synthetic construct
  misc_feature 1..25: note = Description of Artificial Sequence: Synthetic primer
  source 1..25: mol_type = other DNA
ctctgttggtggaaactccctgacc

SEQ ID NO: 358 - DNA, 20 bp, synthetic construct
  misc_feature 1..20: note = Description of Artificial Sequence: Synthetic primer
  source 1..20: mol_type = other DNA
gggccgggaaagagttgctg

SEQ ID NO: 359 - DNA, 22 bp, synthetic construct
  misc_feature 1..22: note = Description of Artificial Sequence: Synthetic primer
  source 1..22: mol_type = other DNA
gccctacatctgctctccctcc

SEQ ID NO: 360 - DNA, 25 bp, synthetic construct
  misc_feature 1..25: note = Description of Artificial Sequence: Synthetic primer
  source 1..25: mol_type = other DNA
ccagcacaacttactcgcacttgac

SEQ ID NO: 361 - DNA, 22 bp, synthetic construct
  misc_feature 1..22: note = Description of Artificial Sequence: Synthetic primer
  source 1..22: mol_type = other DNA
catcaccaacccacagccaagg

SEQ ID NO: 362 - DNA, 27 bp, synthetic construct
  misc_feature 1..27: note = Description of Artificial Sequence: Synthetic primer
  source 1..27: mol_type = other DNA
cagctccacaaacttggtgccaaattc

SEQ ID NO: 363 - DNA, 23 bp, synthetic construct
  misc_feature 1..23: note = Description of Artificial Sequence: Synthetic primer
  source 1..23: mol_type = other DNA
ccgcaatgaaggggaagctcgac

SEQ ID NO: 364 - DNA, 28 bp, synthetic construct
  misc_feature 1..28: note = Description of Artificial Sequence: Synthetic primer
  source 1..28: mol_type = other DNA
cgctgttcaggtctctgctagaagtagg

SEQ ID NO: 365 - DNA, 23 bp, synthetic construct
  misc_feature 1..23: note = Description of Artificial Sequence: Synthetic primer
  source 1..23: mol_type = other DNA
ccagaccagagaccactgggaag

SEQ ID NO: 366 - DNA, 33 bp, synthetic construct
  misc_feature 1..33: note = Description of Artificial Sequence: Synthetic primer
  source 1..33: mol_type = other DNA
gacaaatgtatcatgctattataagatgttgac

SEQ ID NO: 367 - DNA, 29 bp, synthetic construct
  misc_feature 1..29: note = Description of Artificial Sequence: Synthetic primer
  source 1..29: mol_type = other DNA
ccatttactgagagtaattataattgtgc

SEQ ID NO: 368 - DNA, 30 bp, synthetic construct
  misc_feature 1..30: note = Description of Artificial Sequence: Synthetic primer
  source 1..30: mol_type = other DNA
ccaaggacaggaatatcttataccctctgt

SEQ ID NO: 369 - DNA, 28 bp, synthetic construct
  misc_feature 1..28: note = Description of Artificial Sequence: Synthetic primer
  source 1..28: mol_type = other DNA
tgtcattgtccttgtcctttagctaccg

SEQ ID NO: 370 - DNA, 22 bp, synthetic construct
  misc_feature 1..22: note = Description of Artificial Sequence: Synthetic primer
  source 1..22: mol_type = other DNA
caaaacagccaagcttgcatgc

SEQ ID NO: 371 - DNA, 33 bp, synthetic construct
  misc_feature 1..33: note = Description of Artificial Sequence: Synthetic primer
  source 1..33: mol_type = other DNA
agctgccatcggtatttcacaccgcatacgtac

SEQ ID NO: 372 - DNA, 33 bp, synthetic construct
  misc_feature 1..33: note = Description of Artificial Sequence: Synthetic primer
  source 1..33: mol_type = other DNA
agctggcaacggtatttcacaccgcatacgtac

SEQ ID NO: 373 - DNA, 33 bp, synthetic construct
  misc_feature 1..33: note = Description of Artificial Sequence: Synthetic primer
  source 1..33: mol_type = other DNA
agctgatgccggtatttcacaccgcatacgtac

SEQ ID NO: 374 - DNA, 33 bp, synthetic construct
  misc_feature 1..33: note = Description of Artificial Sequence: Synthetic primer
  source 1..33: mol_type = other DNA
agctggatgcggtatttcacaccgcatacgtac

SEQ ID NO: 375 - DNA, 33 bp, synthetic construct
  misc_feature 1..33: note = Description of Artificial Sequence: Synthetic primer
  source 1..33: mol_type = other DNA
agctgcgatcggtatttcacaccgcatacgtac

SEQ ID NO: 376 - DNA, 69 bp, synthetic construct
  misc_feature 1..69: note = Description of Artificial Sequence: Synthetic oligonucleotide
  modified_base 13..15: mod_base = OTHER; note = a, c, t, g, unknown or other
  modified_base 18..27: mod_base = OTHER; note = a, c, t, g, unknown or other
  source 1..69: mol_type = other DNA
agaccggaattcnnngtnnnnnnnnnnggaatcccttctgcagcacctgggcgcaggtcacgaggcatg

SEQ ID NO: 377 - DNA, 69 bp, synthetic construct
  misc_feature 1..69: note = Description of Artificial Sequence: Synthetic oligonucleotide
  modified_base 13..15: mod_base = OTHER; note = a, c, t, g, unknown or other
  modified_base 18..27: mod_base = OTHER; note = a, c, t, g, unknown or other
  source 1..69: mol_type = other DNA
agaccggaattcnnngtnnnnnnnnnnctgatggtccatgtctgttactcgcgcaggtcacgaggcatg

SEQ ID NO: 378 - DNA, 15 bp, synthetic construct
  misc_feature 1..15: note = Description of Artificial Sequence: Synthetic primer
  source 1..15: mol_type = other DNA
cctcgtgacctgcgc

SEQ ID NO: 379 - DNA, 37 bp, synthetic construct
  misc_feature 1..37: note = Description of Artificial Sequence: Synthetic oligonucleotide
  source 1..37: mol_type = other DNA
aattctttaggaatcccttctgcagcacctgggcatg

SEQ ID NO: 380 - DNA, 29 bp, synthetic construct
  misc_feature 1..29: note = Description of Artificial Sequence: Synthetic oligonucleotide
  source 1..29: mol_type = other DNA
cccaggtgctgcagaagggattcctaaag

SEQ ID NO: 381 - DNA, 37 bp, synthetic construct
  misc_feature 1..37: note = Description of Artificial Sequence: Synthetic oligonucleotide
  source 1..37: mol_type = other DNA
aattccttaggaatcccttctgcagcacctgggcatg

SEQ ID NO: 382 - DNA, 29 bp, synthetic construct
  misc_feature 1..29: note = Description of Artificial Sequence: Synthetic oligonucleotide
  source 1..29: mol_type = other DNA
cccaggtgctgcagaagggattcctaagg

SEQ ID NO: 383 - DNA, 37 bp, synthetic construct
  misc_feature 1..37: note = Description of Artificial Sequence: Synthetic oligonucleotide
  source 1..37: mol_type = other DNA
aattcacctggaatcccttctgcagcacctgggcatg

SEQ ID NO: 384 - DNA, 29 bp, synthetic construct
  misc_feature 1..29: note = Description of Artificial Sequence: Synthetic oligonucleotide
  source 1..29: mol_type = other DNA
cccaggtgctgcagaagggattccaggtg

SEQ ID NO: 385 - DNA, 37 bp, synthetic construct
  misc_feature 1..37: note = Description of Artificial Sequence: Synthetic oligonucleotide
  source 1..37: mol_type = other DNA
aattctttactgatggtccatgtctgttactcgcatg

SEQ ID NO: 386 - DNA, 29 bp, synthetic construct
  misc_feature 1..29: note = Description of Artificial Sequence: Synthetic oligonucleotide
  source 1..29: mol_type = other DNA
cgagtaacagacatggaccatcagtaaag

SEQ ID NO: 387 - DNA, 37 bp, synthetic construct
  misc_feature 1..37: note = Description of Artificial Sequence: Synthetic oligonucleotide
  source 1..37: mol_type = other DNA
aattccttactgatggtccatgtctgttactcgcatg

SEQ ID NO: 388 - DNA, 29 bp, synthetic construct
  misc_feature 1..29: note = Description of Artificial Sequence: Synthetic oligonucleotide
  source 1..29: mol_type = other DNA
cgagtaacagacatggaccatcagtaagg

SEQ ID NO: 389 - DNA, 37 bp, synthetic construct
  misc_feature 1..37: note = Description of Artificial Sequence: Synthetic oligonucleotide
  source 1..37: mol_type = other DNA
aattcacctctgatggtccatgtctgttactcgcatg

SEQ ID NO: 390 - DNA, 29 bp, synthetic construct
  misc_feature 1..29: note = Description of Artificial Sequence: Synthetic oligonucleotide
  source 1..29: mol_type = other DNA
cgagtaacagacatggaccatcagaggtg

SEQ ID NO: 391 - DNA, 22 bp, synthetic construct
  misc_feature 1..22: note = Description of Artificial Sequence: Synthetic primer
  source 1..22: mol_type = other DNA
atggtgagcagagtgccctatc

SEQ ID NO: 392 - DNA, 22 bp, synthetic construct
  misc_feature 1..22: note = Description of Artificial Sequence: Synthetic primer
  source 1..22: mol_type = other DNA
atggtccctggcagtctccaaa

SEQ ID NO: 393 - DNA, 23 bp, synthetic construct
  misc_feature 1..23: note = Description of Artificial Sequence: Synthetic primer
  source 1..23: mol_type = other DNA
ccatcggactctcataggttgtc

SEQ ID NO: 394 - DNA, 24 bp, synthetic construct
  misc_feature 1..24: note = Description of Artificial Sequence: Synthetic primer
  source 1..24: mol_type = other DNA
gacctgtacttattgtctctcatc

SEQ ID NO: 395 - DNA, 20 bp, synthetic construct
  misc_feature 1..20: note = Description of Artificial Sequence: Synthetic primer
  source 1..20: mol_type = other DNA
gcacgtggatcctgagaact

SEQ ID NO: 396 - DNA, 21 bp, synthetic construct
  misc_feature 1..21: note = Description of Artificial Sequence: Synthetic primer
  source 1..21: mol_type = other DNA
attggacagcaagaaagcgag

SEQ ID NO: 397 - DNA, 24 bp, synthetic construct
  misc_feature 1..24: note = Description of Artificial Sequence: Synthetic primer
  source 1..24: mol_type = other DNA
cattatgctgaggatttggaaagg

SEQ ID NO: 398 - DNA, 22 bp, synthetic construct
  misc_feature 1..22: note = Description of Artificial Sequence: Synthetic primer
  source 1..22: mol_type = other DNA
cttgagcacacagagggctaca

SEQ ID NO: 399 - DNA, 21 bp, synthetic construct
  misc_feature 1..21: note = Description of Artificial Sequence: Synthetic primer
  source 1..21: mol_type = other DNA
gctccagagccgtgcgaatgg

SEQ ID NO: 400 - DNA, 22 bp, synthetic construct
  misc_feature 1..22: note = Description of Artificial Sequence: Synthetic primer
  source 1..22: mol_type = other DNA
gccctacatctgctctccctcc

SEQ ID NO: 401 - DNA, 26 bp, synthetic construct
  misc_feature 1..26: note = Description of Artificial Sequence: Synthetic primer
  source 1..26: mol_type = other DNA
cagctgacccaataagtggcagagtg

SEQ ID NO: 402 - DNA, 21 bp, synthetic construct
  misc_feature 1..21: note = Description of Artificial Sequence: Synthetic primer
  source 1..21: mol_type = other DNA
tcaggttggctgctgggctgg

SEQ ID NO: 403 - DNA, 19 bp, synthetic construct
  misc_feature 1..19: note = Description of Artificial Sequence: Synthetic primer
  source 1..19: mol_type = other DNA
ccccagtggctgctctggg

SEQ ID NO: 404 - DNA, 22 bp, synthetic construct
  misc_feature 1..22: note = Description of Artificial Sequence: Synthetic primer
  source 1..22: mol_type = other DNA
catcgatgtcctccccattggc

SEQ ID NO: 405 - DNA, 22 bp, synthetic construct
  misc_feature 1..22: note = Description of Artificial Sequence: Synthetic primer
  source 1..22: mol_type = other DNA
gctgtctgaagccatcgcttcc

SEQ ID NO: 406 - DNA, 23 bp, synthetic construct
  misc_feature 1..23: note = Description of Artificial Sequence: Synthetic primer
  source 1..23: mol_type = other DNA
cagaggtatccagcagaggggag

SEQ ID NO: 407 - DNA, 24 bp, synthetic construct
  misc_feature 1..24: note = Description of Artificial Sequence: Synthetic primer
  source 1..24: mol_type = other DNA
ccttcggagcgaaaaccaagacag

SEQ ID NO: 408 - DNA, 25 bp, synthetic construct
  misc_feature 1..25: note = Description of Artificial Sequence: Synthetic primer
  source 1..25: mol_type = other DNA
caggcaggacgaatcacactgaatg

SEQ ID NO: 409 - DNA, 21 bp, synthetic construct
  misc_feature 1..21: note = Description of Artificial Sequence: Synthetic primer
  source 1..21: mol_type = other DNA
gctccagagccgtgcgaatgg

SEQ ID NO: 410 - DNA, 23 bp, synthetic construct
  misc_feature 1..23: note = Description of Artificial Sequence: Synthetic primer
  source 1..23: mol_type = other DNA
gcacctcatggaatcccttctgc

SEQ ID NO: 411 - DNA, 20 bp, synthetic construct
  misc_feature 1..20: note = Description of Artificial Sequence: Synthetic primer
  source 1..20: mol_type = other DNA
gaagctggaggaggaagggc

SEQ ID NO: 412 - DNA, 21 bp, synthetic construct
  misc_feature 1..21: note = Description of Artificial Sequence: Synthetic primer
  source 1..21: mol_type = other DNA
cagcagcaagcagcactctgc

SEQ ID NO: 413 - DNA, 22 bp, synthetic construct
  misc_feature 1..22: note = Description of Artificial Sequence: Synthetic primer
  source 1..22: mol_type = other DNA
gccctcttgcctccactggttg

SEQ ID NO: 414 - DNA, 23 bp, synthetic construct
  misc_feature 1..23: note = Description of Artificial Sequence: Synthetic primer
  source 1..23: mol_type = other DNA
ccaatagcattgcagagaggcgt

SEQ ID NO: 415 - DNA, 367 bp, synthetic construct
  misc_feature 1..367: note = Description of Artificial Sequence: Synthetic polynucleotide
  source 1..367: mol_type = other DNA
tgtacaaaaaagcaggctttaaaggaaccaattcagtcgactggatccggtaccaaggtcgggcaggaagagggcctatttcccatgattccttcatatttgcatatacgatacaaggctgttagagagataattagaattaatttgactgtaaacacaaagatattagtacaaaatacgtgacgtagaaagtaataatttcttgggtagtttgcagttttaaaattatgttttaaaatggactatcatatgcttaccgtaacttgaaagtatttcgatttcttggctttatatatcttgtggaaaggacgaaacaccgtaatttctactcttgtagatggagacgattaatgcgtctccttttttt

SEQ ID NO: 416 - DNA, 367 bp, synthetic construct
  misc_feature 1..367: note = Description of Artificial Sequence: Synthetic polynucleotide
  source 1..367: mol_type = other DNA
tgtacaaaaaagcaggctttaaaggaaccaattcagtcgactggatccggtaccaaggtcgggcaggaagagggcctatttcccatgattccttcatatttgcatatacgatacaaggctgttagagagataattagaattaatttgactgtaaacacaaagatattagtacaaaatacgtgacgtagaaagtaataatttcttgggtagtttgcagttttaaaattatgttttaaaatggactatcatatgcttaccgtaacttgaaagtatttcgatttcttggctttatatatcttgtggaaaggacgaaacaccgaatttctactaagtgtagatggagacgattaatgcgtctccttttttt

SEQ ID NO: 417 - DNA, 366 bp, synthetic construct
  misc_feature 1..366: note = Description of Artificial Sequence: Synthetic polynucleotide
  source 1..366: mol_type = other DNA
tgtacaaaaaagcaggctttaaaggaaccaattcagtcgactggatccggtaccaaggtcgggcaggaagagggcctatttcccatgattccttcatatttgcatatacgatacaaggctgttagagagataattagaattaatttgactgtaaacacaaagatattagtacaaaatacgtgacgtagaaagtaataatttcttgggtagtttgcagttttaaaattatgttttaaaatggactatcatatgcttaccgtaacttgaaagtatttcgatttcttggctttatatatcttgtggaaaggacgaaacaccgaatttctactgttgtagatggagacgattaatgcgtctccttttttt

SEQ ID NO: 418 - DNA, 367 bp, synthetic construct
  misc_feature 1..367: note = Description of Artificial Sequence: Synthetic polynucleotide
  source 1..367: mol_type = other DNA
tgtacaaaaaagcaggctttaaaggaaccaattcagtcgactggatccggtaccaaggtcgggcaggaagagggcctatttcccatgattccttcatatttgcatatacgatacaaggctgttagagagataattagaattaatttgactgtaaacacaaagatattagtacaaaatacgtgacgtagaaagtaataatttcttgggtagtttgcagttttaaaattatgttttaaaatggactatcatatgcttaccgtaacttgaaagtatttcgatttcttggctttatatatcttgtggaaaggacgaaacaccgaatttctactgtttgtagatggagacgattaatgcgtctccttttttt

SEQ ID NO: 419 - DNA, 120 bp, synthetic construct
  misc_feature 1..120: note = Description of Artificial Sequence: Synthetic polynucleotide
  source 1..120: mol_type = other DNA
taatacgactcactatagtaatttctactcttgtagatggagacccatgccatagcgttgttcggaatatgaatttttgaacagattcaccaacacctagtggtctcctttaaaaagctt

SEQ ID NO: 420 - DNA, 120 bp, synthetic construct
  misc_feature 1..120: note = Description of Artificial Sequence: Synthetic polynucleotide
  source 1..120: mol_type = other DNA
taatacgactcactatagaatttctactaagtgtagatggagacccatgccatagcgttgttcggaatatgaatttttgaacagattcaccaacacctagtggtctcctttaaaaagctt

SEQ ID NO: 421 - DNA, 4059 bp, synthetic construct; identical to SEQ ID NO: 6
  misc_feature 1..4059: note = Description of Artificial Sequence: Synthetic polynucleotide
  source 1..4059: mol_type = other DNA

SEQ ID NO: 422 - DNA, 4059 bp, synthetic construct
  misc_feature 1..4059: note = Description of Artificial Sequence: Synthetic polynucleotide
  source 1..4059: mol_type = other DNA
atgacacagttcgagggctttaccaacctgtatcaggtgagcaagacactgcggtttgagctgatcccacagggcaagaccctgaagcacatccaggagcagggcttcatcgaggaggacaaggcccgcaatgatcactacaaggagctgaagcccatcatcgatcggatctacaagacctatgccgaccagtgcctgcagctggtgcagctggattgggagaacctgagcgccgccatcgactcctatagaaaggagaaaaccgaggagacaaggaacgccctgatcgaggagcaggccacatatcgcaatgccatccacgactacttcatcggccggacagacaacctgaccgatgccatcaataagagacacgccgagatctacaagggcctgttcaaggccgagctgtttaatggcaaggtgctgaagcagctgggcaccgtgaccacaaccgagcacgagaacgccctgctgcggagcttcgacaagtttacaacctacttctccggcttttatagaaacaggaagaacgtgttcagcgccgaggatatcagcacagccatcccacaccgcatcgtgcaggacaacttccccaagtttaaggagaattgtcacatcttcacacgcctgatcaccgccgtgcccagcctgcgggagcactttgagaacgtgaagaaggccatcggcatcttcgtgagcacctccatcgaggaggtgttttccttccctttttataaccagctgctgacacagacccagatcgacctgtataaccagctgctgggaggaatctctcgggaggcaggcaccgagaagatcaagggcctgaacgaggtgctgaatctggccatccagaagaatgatgagacagcccacatcatcgcctccctgccacacagattcatccccctgtttaagcagatcctgtccgataggaacaccctgtctttcatcctggaggagtttaagagcgacgaggaagtgatccagtccttctgcaagtacaagacactgctgagaaacgagaacgtgctggagacagccgaggccctgtttaacgagctgaacagcatcgacctgacacacatcttcatcagccacaagaagctggagacaatcagcagcgccctgtgcgaccactgggatacactgaggaatgccctgtatgagcggagaatctccgagctgacaggcaagatcaccaagtctgccaaggagaaggtgcagcgcagcctgaagcacgaggatatcaacctgcaggagatcatctctgccgcaggcaaggagctgagcgaggccttcaagcagaaaaccagcgagatcctgtcccacgcacacgccgccctggatcagccactgcctacaaccctgaagaagcaggaggagaaggagatcctgaagtctcagctggacagcctgctgggcctgtaccacctgctggactggtttgccgtggatgagtccaacgaggtggaccccgagttctctgcccggctgaccggcatcaagctggagatggagccttctctgagcttctacaacaaggccagaaattatgccaccaagaagccctactccgtggagaagttcaagctgaactttcagatgcctacactggccagaggctgggacgtgaataaggagaagaacaatggcgccatcctgtttgtgaagaacggcctgtactatctgggcatcatgccaaagcagaagggcaggtataaggccctgagcttcgagcccacagagaaaaccagcgagggctttgataagatgtactatgactacttccctgatgccgccaagatgatcccaaagtgcagcacccagctgaaggccgtgacagcccactttcagacccacacaacccccatcctgctgtccaacaatttcatcgagcctctggagatcacaaaggagatctacgacctgaacaatcctgagaaggagccaaagaagtttcagacagcctacgccaagaaaaccggcgaccagaagggctacagagaggccctgtgcaagtggatcgacttcacaagggattttctgtccaagtataccaagacaacctctatcgatctgtctagcctgcggccatcctctcagtataaggacctgggcgagtactatgccgagctgaatcccctgctgtaccacatcagcttccagagaatcgccgagaaggagatcatggatgccgtggagacaggcaagctgtacctgttccagatctataacaaggactttgccaagggccaccacggcaagcctaatctgcacacactgtattggaccggcctgttttctccagagaacctggccaagacaagcatcaagctgaatggccaggccgagctgttctaccgccctaagtccaggatgaagaggatggcacaccggctgggagagaagatgctgaacaagaagctgaaggatcagaaaaccccaatccccgacaccctgtaccaggagctgtacgactatgtgaatcacagactgtcccacgacctgtctgatgaggccagggccctgctgcccaacgtgatcaccaaggaggtgtctcacgagatcatcaaggataggcgctttaccagcgacaagttctttttccacgtgcctatcacactgaactatcaggccgccaattccccatctaagttcaaccagagggtgaatgcctacctgaaggagcaccccgagacacctatcatcggcatcgatcggggcgagagaaacctgatctatatcacagtgatcgactccaccggcaagatcctggagcagcggagcctgaacaccatccagcagtttgattaccagaagaagctggacaacagggagaaggagagggtggcagcaaggcaggcctggtctgtggtgggcacaatcaaggatctgaagcagggctatctgagccaggtcatccacgagatcgtggacctgatgatccactaccaggccgtggtggtgctggagaacctgaatttcggctttaagagcaagaggaccggcatcgccgagaaggccgtgtaccagcagttcgagaagatgctgatcgataagctgaattgcctggtgctgaaggactatccagcagagaaagtgggaggcgtgctgaacccataccagctgacagaccagttcacctcctttgccaagatgggcacccagtctggcttcctgttttacgtgcctgccccatatacatctaagatcgatcccctgaccggcttcgtggaccccttcgtgtggaaaaccatcaagaatcacgagagccgcaagcacttcctggagggcttcgactttctgcactacgacgtgaaaaccggcgacttcatcctgcactttaagatgaacagaaatctgtccttccagaggggcctgcccggctttatgcctgcatgggatatcgtgttcgagaagaacgagacacagtttgacgccaagggcacccctttcatcgccggcaagagaatcgtgccagtgatcgagaatcacagattcaccggcagataccgggacctgtatcctgccaacgagctgatcgccctgctggaggagaagggcatcgtgttcagggatggctccaacatcctgccaaagctgctggagaatgacgattctcacgccatcgacaccatggtggccctgatccgcagcgtgctgcagatgcggaactccaatgccgccacaggcgaggactatatcaacagccccgtgcgcgatctgaatggcgtgtgcttcgactcccggtttcagaacccagagtggcccatggacgccgatgccaatggcgcctaccacatcgccctgaagggccagctgctgctgaatcacctgaaggagagcaaggatctgaagctgcagaacggcatctccaatcaggactggctggcctacatccaggagctgcgcaacaaaaggccggcggccacgaaaaaggccggccaggcaaaaaagaaaaagggatcctacccatacgatgttccagattacgcttatccctacgacgtgcctgattatgcatacccatatgatgtccccgactatgcctaa

SEQ ID NO: 423 - DNA, 4059 bp, synthetic construct
  misc_feature 1..4059: note = Description of Artificial Sequence: Synthetic polynucleotide
  source 1..4059: mol_type = other DNA
atgacacagttcgagggctttaccaacctgtatcaggtgagcaagacactgcggtttgagctgatcccacagggcaagaccctgaagcacatccaggagcagggcttcatcgaggaggacaaggcccgcaatgatcactacaaggagctgaagcccatcatcgatcggatctacaagacctatgccgaccagtgcctgcagctggtgcagctggattgggagaacctgagcgccgccatcgactcctatagaaaggagaaaaccgaggagacaaggaacgccctgatcgaggagcaggccacatatcgcaatgccatccacgactacttcatcggccggacagacaacctgaccgatgccatcaataagagacacgccgagatctacaagggcctgttcaaggccgagctgtttaatggcaaggtgctgaagcagctgggcaccgtgaccacaaccgagcacgagaacgccctgctgcggagcttcgacaagtttacaacctacttctccggcttttatagaaacaggaagaacgtgttcagcgccgaggatatcagcacagccatcccacaccgcatcgtgcaggacaacttccccaagtttaaggagaattgtcacatcttcacacgcctgatcaccgccgtgcccagcctgcgggagcactttgagaacgtgaagaaggccatcggcatcttcgtgagcacctccatcgaggaggtgttttccttccctttttataaccagctgctgacacagacccagatcgacctgtataaccagctgctgggaggaatctctcgggaggcaggcaccgagaagatcaagggcctgaacgaggtgctgaatctggccatccagaagaatgatgagacagcccacatcatcgcctccctgccacacagattcatccccctgtttaagcagatcctgtccgataggaacaccctgtctttcatcctggaggagtttaagagcgacgaggaagtgatccagtccttctgcaagtacaagacactgctgagaaacgagaacgtgctggagacagccgaggccctgtttaacgagctgaacagcatcgacctgacacacatcttcatcagccacaagaagctggagacaatcagcagcgccctgtgcgaccactgggatacactgaggaatgccctgtatgagcggagaatctccgagctgacaggcaagatcaccaagtctgccaaggagaaggtgcagcgcagcctgaagcacgaggatatcaacctgcaggagatcatctctgccgcaggcaaggagctgagcgaggccttcaagcagaaaaccagcgagatcctgtcccacgcacacgccgccctggatcagccactgcctacaaccctgaagaagcaggaggagaaggagatcctgaagtctcagctggacagcctgctgggcctgtaccacctgctggactggtttgccgtggatgagtccaacgaggtggaccccgagttctctgcccggctgaccggcatcaagctggagatggagccttctctgagcttctacaacaaggccagaaattatgccaccaagaagccctactccgtggagaagttcaagctgaactttcagatgcctacactggccagaggctgggacgtgaatagagagaagaacaatggcgccatcctgtttgtgaagaacggcctgtactatctgggcatcatgccaaagcagaagggcaggtataaggccctgagcttcgagcccacagagaaaaccagcgagggctttgataagatgtactatgactacttccctgatgccgccaagatgatcccaaagtgcagcacccagctgaaggccgtgacagcccactttcagacccacacaacccccatcctgctgtccaacaatttcatcgagcctctggagatcacaaaggagatctacgacctgaacaatcctgagaaggagccaaagaagtttcagacagcctacgccaagaaaaccggcgaccagaagggctacagagaggccctgtgcaagtggatcgacttcacaagggattttctgtccaagtataccaagacaacctctatcgatctgtctagcctgcggccatcctctcagtataaggacctgggcgagtactatgccgagctgaatcccctgctgtaccacatcagcttccagagaatcgccgagaaggagatcatggatgccgtggagacaggcaagctgtacctgttccagatctataacaaggactttgccaagggccaccacggcaagcctaatctgcacacactgtattggaccggcctgttttctccagagaacctggccaagacaagcatcaagctgaatggccaggccgagctgttctaccgccctaagtccaggatgaagaggatggcacaccggctgggagagaagatgctgaacaagaagctgaaggatcagaaaaccccaatccccgacaccctgtaccaggagctgtacgactatgtgaatcacagactgtcccacgacctgtctgatgaggccagggccctgctgcccaacgtgatcaccaaggaggtgtctcacgagatcatcaaggataggcgctttaccagcgacaagttctttttccacgtgcctatcacactgaactatcaggccgccaattccccatctaagttcaaccagagggtgaatgcctacctgaaggagcaccccgagacacctatcatcggcatcgatcggggcgagagaaacctgatctatatcacagtgatcgactccaccggcaagatcctggagcagcggagcctgaacaccatccagcagtttgattaccagaagaagctggacaacagggagaaggagagggtggcagcaaggcaggcctggtctgtggtgggcacaatcaaggatctgaagcagggctatctgagccaggtcatccacgagatcgtggacctgatgatccactaccaggccgtggtggtgctggagaacctgaatttcggctttaagagcaagaggaccggcatcgccgagaaggccgtgtaccagcagttcgagaagatgctgatcgataagctgaattgcctggtgctgaaggactatccagcagagaaagtgggaggcgtgctgaacccataccagctgacagaccagttcacctcctttgccaagatgggcacccagtctggcttcctgttttacgtgcctgccccatatacatctaagatcgatcccctgaccggcttcgtggaccccttcgtgtggaaaaccatcaagaatcacgagagccgcaagcacttcctggagggcttcgactttctgcactacgacgtgaaaaccggcgacttcatcctgcactttaagatgaacagaaatctgtccttccagaggggcctgcccggctttatgcctgcatgggatatcgtgttcgagaagaacgagacacagtttgacgccaagggcacccctttcatcgccggcaagagaatcgtgccagtgatcgagaatcacagattcaccggcagataccgggacctgtatcctgccaacgagctgatcgccctgctggaggagaagggcatcgtgttcagggatggctccaacatcctgccaaagctgctggagaatgacgattctcacgccatcgacaccatggtggccctgatccgcagcgtgctgcagatgcggaactccaatgccgccacaggcgaggactatatcaacagccccgtgcgcgatctgaatggcgtgtgcttcgactcccggtttcagaacccagagtggcccatggacgccgatgccaatggcgcctaccacatcgccctgaagggccagctgctgctgaatcacctgaaggagagcaaggatctgaagctgcagaacggcatctccaatcaggactggctggcctacatccaggagctgcgcaacaaaaggccggcggccacgaaaaaggccggccaggcaaaaaagaaaaagggatcctacccatacgatgttccagattacgcttatccctacgacgtgcctgattatgcatacccatatgatgtccccgactatgcctaa

SEQ ID NO: 424 - DNA, 4059 bp, synthetic construct
  misc_feature 1..4059: note = Description of Artificial Sequence: Synthetic polynucleotide
  source 1..4059: mol_type = other DNA
atgacacagttcgagggctttaccaacctgtatcaggtgagcaagacactgcggtttgagctgatcccacagggcaagaccctgaagcacatccaggagcagggcttcatcgaggaggacaaggcccgcaatgatcactacaaggagctgaagcccatcatcgatcggatctacaagacctatgccgaccagtgcctgcagctggtgcagctggattgggagaacctgagcgccgccatcgactcctatagaaaggagaaaaccgaggagacaaggaacgccctgatcgaggagcaggccacatatcgcaatgccatccacgactacttcatcggccggacagacaacctgaccgatgccatcaataagagacacgccgagatctacaagggcctgttcaaggccgagctgtttaatggcaaggtgctgaagcagctgggcaccgtgaccacaaccgagcacgagaacgccctgctgcggagcttcgacaagtttacaacctacttctccggcttttatagaaacaggaagaacgtgttcagcgccgaggatatcagcacagccatcccacaccgcatcgtgcaggacaacttccccaagtttaaggagaattgtcacatcttcacacgcctgatcaccgccgtgcccagcctgcgggagcactttgagaacgtgaagaaggccatcggcatcttcgtgagcacctccatcgaggaggtgttttccttccctttttataaccagctgctgacacagacccagatcgacctgtataaccagctgctgggaggaatctctcgggaggcaggcaccgagaagatcaagggcctgaacgaggtgctggccctggccatccagaagaatgatgagacagcccacatcatcgcctccctgccacacagattcatccccctgtttaagcagatcctgtccgataggaacaccctgtctttcatcctggaggagtttaagagcgacgaggaagtgatccagtccttctgcaagtacaagacactgctgagaaacgagaacgtgctggagacagccgaggccctgtttaacgagctgaacagcatcgacctgacacacatcttcatcagccacaagaagctggagacaatcagcagcgccctgtgcgaccactgggatacactgaggaatgccctgtatgagcggagaatctccgagctgacaggcaagatcaccaagtctgccaaggagaaggtgcagcgcagcctgaagcacgaggatatcaacctgcaggagatcatctctgccgcaggcaaggagctgagcgaggccttcaagcagaaaaccagcgagatcctgtcccacgcacacgccgccctggatcagccactgcctacaaccctgaagaagcaggaggagaaggagatcctgaagtctcagctggacagcctgctgggcctgtaccacctgctggactggtttgccgtggatgagtccaacgaggtggaccccgagttctctgcccggctgaccggcatcaagctggagatggagccttctctgagcttctacaacaaggccagaaattatgccaccaagaagccctactccgtggagaagttcaagctgaactttcagatgcctacactggccagaggctgggacgtgaatagagagaagaacaatggcgccatcctgtttgtgaagaacggcctgtactatctgggcatcatgccaaagcagaagggcaggtataaggccctgagcttcgagcccacagagaaaaccagcgagggctttgataagatgtactatgactacttccctgatgccgccaagatgatcccaaagtgcagcacccagctgaaggccgtgacagcccactttcagacccacacaacccccatcctgctgtccaacaatttcatcgagcctctggagatcacaaaggagatctacgacctgaacaatcctgagaaggagccaaagaagtttcagacagcctacgccaagaaaaccggcgaccagaagggctacagagaggccctgtgcaagtggatcgacttcacaagggattttctgtccaagtataccaagacaacctctatcgatctgtctagcctgcggccatcctctcagtataaggacctgggcgagtactatgccgagctgaatcccctgctgtaccacatcagcttccagagaatcgccgagaaggagatcatggatgccgtggagacaggcaagctgtacctgttccagatctataacaaggactttgccaagggccaccacggcaagcctaatctgcacacactgtattggaccggcctgttttctccagagaacctggccaagacaagcatcaagctgaatggccaggccgagctgttctaccgccctaagtccaggatgaagaggatggcacaccggctgggagagaagatgctgaacaagaagctgaaggatcagaaaaccccaatccccgacaccctgtaccaggagctgtacgactatgtgaatcacagactgtcccacgacctgtctgatgaggccagggccctgctgcccaacgtgatcaccaaggaggtgtctcacgagatcatcaaggataggcgctttaccagcgacaagttctttttccacgtgcctatcacactgaactatcaggccgccaattccccatctaagttcaaccagagggtgaatgcctacctgaaggagcaccccgagacacctatcatcggcatcgatcggggcgagagaaacctgatctatatcacagtgatcgactccaccggcaagatcctggagcagcggagcctgaacaccatccagcagtttgattaccagaagaagctggacaacagggagaaggagagggtggcagcaaggcaggcctggtctgtggtgggcacaatcaaggatctgaagcagggctatctgagccaggtcatccacgagatcgtggacctgatgatccactaccaggccgtggtggtgctggagaacctgaatttcggctttaagagcaagaggaccggcatcgccgagaaggccgtgtaccagcagttcgagaagatgctgatcgataagctgaattgcctggtgctgaaggactatccagcagagaaagtgggaggcgtgctgaacccataccagctgacagaccagttcacctcctttgccaagatgggcacccagtctggcttcctgttttacgtgcctgccccatatacatctaagatcgatcccctgaccggcttcgtggaccccttcgtgtggaaaaccatcaagaatcacgagagccgcaagcacttcctggagggcttcgactttctgcactacgacgtgaaaaccggcgacttcatcctgcactttaagatgaacagaaatctgtccttccagaggggcctgcccggctttatgcctgcatgggatatcgtgttcgagaagaacgagacacagtttgacgccaagggcacccctttcatcgccggcaagagaatcgtgccagtgatcgagaatcacagattcaccggcagataccgggacctgtatcctgccaacgagctgatcgccctgctggaggagaagggcatcgtgttcagggatggctccaacatcctgccaaagctgctggagaatgacgattctcacgccatcgacaccatggtggccctgatccgcagcgtgctgcagatgcggaactccaatgccgccacaggcgaggactatatcaacagccccgtgcgcgatctgaatggcgtgtgcttcgactcccggtttcagaacccagagtggcccatggacgccgatgccaatggcgcctaccacatcgccctgaagggccagctgctgctgaatcacctgaaggagagcaaggatctgaagctgcagaacggcatctccaatcaggactggctggcctacatccaggagctgcgcaacaaaaggccggcggccacgaaaaaggccggccaggcaaaaaagaaaaagggatcctacccatacgatgttccagattacgcttatccctacgacgtgcctgattatgcatacccatatgatgtccccgactatgcctaa

SEQ ID NO: 425 - DNA, 4011 bp, synthetic construct
  misc_feature 1..4011: note = Description of Artificial Sequence: Synthetic polynucleotide
  source 1..4011: mol_type = other DNA
atggggacacagttcgagggctttaccaacctgtatcaggtgagcaagacactgcggtttgagctgatcccacagggcaagaccctgaagcacatccaggagcagggcttcatcgaggaggacaaggcccgcaatgatcactacaaggagctgaagcccatcatcgatcggatctacaagacctatgccgaccagtgcctgcagctggtgcagctggattgggagaacctgagcgccgccatcgactcctatagaaaggagaaaaccgaggagacaaggaacgccctgatcgaggagcaggccacatatcgcaatgccatccacgactacttcatcggccggacagacaacctgaccgatgccatcaataagagacacgccgagatctacaagggcctgttcaaggccgagctgtttaatggcaaggtgctgaagcagctgggcaccgtgaccacaaccgagcacgagaacgccctgctgcggagcttcgacaagtttacaacctacttctccggcttttatgagaacaggaagaacgtgttcagcgccgaggatatcagcacagccatcccacaccgcatcgtgcaggacaacttccccaagtttaaggagaattgtcacatcttcacacgcctgatcaccgccgtgcccagcctgcgggagcactttgagaacgtgaagaaggccatcggcatcttcgtgagcacctccatcgaggaggtgttttccttccctttttataaccagctgctgacacagacccagatcgacctgtataaccagctgctgggaggaatctctcgggaggcaggcaccgagaagatcaagggcctgaacgaggtgctgaatctggccatccagaagaatgatgagacagcccacatcatcgcctccctgccacacagattcatccccctgtttaagcagatcctgtccgataggaacaccctgtctttcatcctggaggagtttaagagcgacgaggaagtgatccagtccttctgcaagtacaagacactgctgagaaacgagaacgtgctggagacagccgaggccctgtttaacgagctgaacagcatcgacctgacacacatcttcatcagccacaagaagctggagacaatcagcagcgccctgtgcgaccactgggatacactgaggaatgccctgtatgagcggagaatctccgagctgacaggcaagatcaccaagtctgccaaggagaaggtgcagcgcagcctgaagcacgaggatatcaacctgcaggagatcatctctgccgcaggcaaggagctgagcgaggccttcaagcagaaaaccagcgagatcctgtcccacgcacacgccgccctggatcagccactgcctacaaccctgaagaagcaggaggagaaggagatcctgaagtctcagctggacagcctgctgggcctgtaccacctgctggactggtttgccgtggatgagtccaacgaggtggaccccgagttctctgcccggctgaccggcatcaagctggagatggagccttctctgagcttctacaacaaggccagaaattatgccaccaagaagccctactccgtggagaagttcaagctgaactttcagatgcctacactggcctctggctgggacgtgaataaggagaagaacaatggcgccatcctgtttgtgaagaacggcctgtactatctgggcatcatgccaaagcagaagggcaggtataaggccctgagcttcgagcccacagagaaaaccagcgagggctttgataagatgtactatgactacttccctgatgccgccaagatgatcccaaagtgcagcacccagctgaaggccgtgacagcccactttcagacccacacaacccccatcctgctgtccaacaatttcatcgagcctctggagatcacaaaggagatctacgacctgaacaatcctgagaaggagccaaagaagtttcagacagcctacgccaagaaaaccggcgaccagaagggctacagagaggccctgtgcaagtggatcgacttcacaagggattttctgtccaagtataccaagacaacctctatcgatctgtctagcctgcggccatcctctcagtataaggacctgggcgagtactatgccgagctgaatcccctgctgtaccacatcagcttccagagaatcgccgagaaggagatcatggatgccgtggagacaggcaagctgtacctgttccagatctataacaaggactttgccaagggccaccacggcaagcctaatctgcacacactgtattggaccggcctgttttctccagagaacctggccaagacaagcatcaagctgaatggccaggccgagctgttctaccgccctaagtccaggatgaagaggatggcacaccggctgggagagaagatgctgaacaagaagctgaaggatcagaaaaccccaatccccgacaccctgtaccaggagctgtacgactatgtgaatcacagactgtcccacgacctgtctgatgaggccagggccctgctgcccaacgtgatcaccaaggaggtgtctcacgagatcatcaaggataggcgctttaccagcgacaagttctttttccacgtgcctatcacactgaactatcaggccgccaattccccatctaagttcaaccagagggtgaatgcctacctgaaggagcaccccgagacacctatcatcggcatcgatcggggcgagagaaacctgatctatatcacagtgatcgactccaccggcaagatcctggagcagcggagcctgaacaccatccagcagtttgattaccagaagaagctggacaacagggagaaggagagggtggcagcaaggcaggcctggtctgtggtgggcacaatcaaggatctgaagcagggctatctgagccaggtcatccacgagatcgtggacctgatgatccactaccaggccgtggtggtgctggagaacctgaatttcggctttaagagcaagaggaccggcatcgccgagaaggccgtgtaccagcagttcgagaagatgctgatcgataagctgaattgcctggtgctgaaggactatccagcagagaaagtgggaggcgtgctgaacccataccagctgacagaccagttcacctcctttgccaagatgggcacccagtctggcttcctgttttacgtgcctgccccatatacatctaagatcgatcccctgaccggcttcgtggaccccttcgtgtggaaaaccatcaagaatcacgagagccgcaagcacttcctggagggcttcgactttctgcactacgacgtgaaaaccggcgacttcatcctgcactttaagatgaacagaaatctgtccttccagaggggcctgcccggctttatgcctgcatgggatatcgtgttcgagaagaacgagacacagtttgacgccaagggcacccctttcatcgccggcaagagaatcgtgccagtgatcgagaatcacagattcaccggcagataccgggacctgtatcctgccaacgagctgatcgccctgctggaggagaagggcatcgtgttcagggatggctccaacatcctgccaaagctgctggagaatgacgattctcacgccatcgacacgatggtggccctgatccgcagcgtgctgcagatgcggaactccaatgccgccacaggcgaggactatatcaacagccccgtgcgcgatctgaatggcgtgtgcttcgactcccggtttcagaacccagagtggccaatggacgccgatgccaatggcgcctaccacatcgccctgaagggccagctgctgctgaatcacctgaaggagagcaaggatctgaagctgcagaacggcatctccaatcaggactggctggcctacatccaggagctgcgcaacaaaaggccggcggccacgaaaaaggccggccaggcaaaaaagaaaaagggagcggccgcactcgagcaccaccaccaccaccactga

SEQ ID NO: 426 - DNA, 3780 bp, synthetic construct
  misc_feature 1..3780: note = Description of Artificial Sequence: Synthetic polynucleotide
  source 1..3780: mol_type = other DNA
atggggagcaaactggaaaaatttacgaattgttatagcctgtccaagaccctgcgtttcaaagccatccccgttggcaaaacccaggagaatattgataataaacgtctgctggttgaggatgaaaaaagagcagaagactataagggagtcaaaaaactgctggatcggtactacctgagctttataaatgacgtgctgcatagcattaaactgaaaaatctgaataactatattagtctgttccgcaagaaaacccgaacagagaaagaaaataaagagctggaaaacctggagatcaatctgcgtaaagagatcgcaaaagcttttaaaggaaatgaaggttataaaagcctgttcaaaaaagacattattgaaaccatcctgccggaatttctggatgataaagacgagatagcgctcgtgaacagcttcaacgggttcacgaccgccttcacgggctttttcgataacagggaaaatatgttttcagaggaagccaaaagcacctcgatagcgttccgttgcattaatgaaaatttgacaagatatatcagcaacatggatattttcgagaaagttgatgcgatctttgacaaacatgaagtgcaggagattaaggaaaaaattctgaacagcgattatgatgttgaggattttttcgagggggaattttttaactttgtactgacacaggaaggtatagatgtgtataatgctattatcggcgggttcgttaccgaatccggcgagaaaattaagggtctgaatgagtacatcaatctgtataaccaaaagaccaaacagaaactgccaaaattcaaaccgctgtacaagcaagtcctgagcgatcgggaaagcttgagcttttacggtgaaggttataccagcgacgaggaggtactggaggtctttcgcaataccctgaacaagaacagcgaaattttcagctccattaaaaagctggagaaactgtttaagaattttgacgagtacagcagcgcaggtatttttgtgaagaacggacctgccataagcaccattagcaaggatatttttggagagtggaatgttatccgtgataaatggaacgcggaatatgatgacatacacctgaaaaagaaggctgtggtaactgagaaatatgaagacgatcgccgcaaaagctttaaaaaaatcggcagctttagcctggagcagctgcaggaatatgcggacgccgacctgagcgtggtcgagaaactgaaggaaattattatccaaaaagtggatgagatttacaaggtatatggtagcagcgaaaaactgtttgatgcggacttcgttctggaaaaaagcctgaaaaaaaatgatgctgttgttgcgatcatgaaagacctgctcgatagcgttaagagctttgaaaattacattaaagcattctttggcgagggcaaagaaacaaacagagacgaaagcttttatggcgacttcgtcctggcttatgacatcctgttgaaggtagatcatatatatgatgcaattcgtaattacgtaacccaaaagccgtacagcaaagataagttcaaactgtatttccagaacccgcagtttatgggtggctgggacaaagacaaggagacagactatcgcgccactattctgcgttacggcagcaagtactatctcgccatcatggacaaaaaatatgcaaagtgtctgcagaaaatcgataaagacgacgtgaacggaaattacgaaaagattaattataagctgctgccagggcccaacaagatgttaccgaaagtatttttttccaaaaaatggatggcatactataacccgagcgaggatatacagaagatttacaaaaatgggaccttcaaaaagggggatatgttcaatctgaatgactgccacaaactgatcgatttttttaaagatagcatcagccgttatcctaaatggtcaaacgcgtatgattttaatttctccgaaacggagaaatataaagacattgctggtttctatcgcgaagtcgaagaacagggttataaagttagctttgaatcggccagcaagaaagaggttgataaactggtggaggagggtaagctgtatatgtttcagatttataacaaagactttagcgacaaaagccacggtactcctaatctgcatacgatgtactttaaactgctgtttgatgagaataaccacggccaaatccgtctctccggtggagcagaactttttatgcggcgtgcgagcctaaaaaaggaagaactggtggtgcatcccgccaacagcccgattgctaacaaaaatccagataatcctaagaagaccaccacactgtcgtacgatgtctataaggataaacgtttctcggaagaccagtatgaattgcatataccgatagcaattaataaatgcccaaaaaacattttcaaaatcaacactgaagttcgtgtgctgctgaaacatgatgataatccgtatgtgatcggaattgaccgtggggagagaaatctgctgtatattgtagtcgttgatggcaagggcaacatcgttgagcagtatagcctgaatgaaataattaataattttaacggtatacgtattaaaaccgactatcatagcctgctggataaaaaggagaaagagcgttttgaggcacgccaaaattggacgagcatcgaaaacatcaaggaactgaaggcaggatatatcagccaagtagtccataaaatctgtgaactggtggagaagtacgacgctgtcattgccctggaagacctcaatagcggctttaaaaacagccgggtgaaggtggagaaacaggtataccaaaagtttgaaaagatgctcattgataagctgaactatatggttgataaaaagagcaacccgtgcgccactggcggtgcactgaaagggtaccaaattaccaataaatttgaaagctttaaaagcatgagcacgcagaatgggtttattttttatataccagcatggctgacgagcaagattgaccccagcactggttttgtcaatctgctgaaaaccaaatacacaagcattgcggatagcaaaaaatttatttcgagcttcgaccgtattatgtatgttccggaggaagatctgtttgaatttgccctggattataaaaacttcagccgcaccgatgcagattatatcaaaaaatggaagctgtacagttatggtaatcgtatacgtatcttccgtaatccgaagaaaaacaatgtgttcgattgggaagaggtctgtctgaccagcgcgtataaagaactgttcaacaagtacggaataaattatcagcaaggtgacattcgcgcactgctgtgtgaacagtcagataaagcattttatagcagctttatggcgctgatgagcctgatgctccagatgcgcaacagcataaccggtcgcacagatgttgactttctgatcagccctgtgaagaatagcgacggcatcttctacgattccaggaactatgaagcacaggaaaacgctattctgcctaaaaatgccgatgccaacggcgcctataatattgcacggaaggttctgtgggcgattggacagttcaagaaagcggaagatgagaagctggataaggtaaaaattgctattagcaataaggaatggctggagtacgcacagacatcggttaaacacggtagtaaaaggccggcggccacgaaaaaggccggccaggcaaaaaagaaaaagggagcggccgcactcgagcaccaccaccaccaccactga

SEQ ID NO: 427 - DNA, 4011 bp, synthetic construct
  misc_feature 1..4011: note = Description of Artificial Sequence: Synthetic polynucleotide
  source 1..4011: mol_type = other DNA
atggggacacagttcgagggctttaccaacctgtatcaggtgagcaagacactgcggtttgagctgatcccacagggcaagaccctgaagcacatccaggagcagggcttcatcgaggaggacaaggcccgcaatgatcactacaaggagctgaagcccatcatcgatcggatctacaagacctatgccgaccagtgcctgcagctggtgcagctggattgggagaacctgagcgccgccatcgactcctatagaaaggagaaaaccgaggagacaaggaacgccctgatcgaggagcaggccacatatcgcaatgccatccacgactacttcatcggccggacagacaacctgaccgatgccatcaataagagacacgccgagatctacaagggcctgttcaaggccgagctgtttaatggcaaggtgctgaagcagctgggcaccgtgaccacaaccgagcacgagaacgccctgctgcggagcttcgacaagtttacaacctacttctccggcttttatagaaacaggaagaacgtgttcagcgccgaggatatcagcacagccatcccacaccgcatcgtgcaggacaacttccccaagtttaaggagaattgtcacatcttcacacgcctgatcaccgccgtgcccagcctgcgggagcactttgagaacgtgaagaaggccatcggcatcttcgtgagcacctccatcgaggaggtgttttccttccctttttataaccagctgctgacacagacccagatcgacctgtataaccagctgctgggaggaatctctcgggaggcaggcaccgagaagatcaagggcctgaacgaggtgctgaatctggccatccagaagaatgatgagacagcccacatcatcgcctccctgccacacagattcatccccctgtttaagcagatcctgtccgataggaacaccctgtctttcatcctggaggagtttaagagcgacgaggaagtgatccagtccttctgcaagtacaagacactgctgagaaacgagaacgtgctggagacagccgaggccctgtttaacgagctgaacagcatcgacctgacacacatcttcatcagccacaagaagctggagacaatcagcagcgccctgtgcgaccactgggatacactgaggaatgccctgtatgagcggagaatctccgagctgacaggcaagatcaccaagtctgccaaggagaaggtgcagcgcagcctgaagcacgaggatatcaacctgcaggagatcatctctgccgcaggcaaggagctgagcgaggccttcaagcagaaaaccagcgagatcctgtcccacgcacacgccgccctggatcagccactgcctacaaccctgaagaagcaggaggagaaggagatcctgaagtctcagctggacagcctgctgggcctgtaccacctgctggactggtttgccgtggatgagtccaacgaggtggaccccgagttctctgcccggctgaccggcatcaagctggagatggagccttctctgagcttctacaacaaggccagaaattatgccaccaagaagccctactccgtggagaagttcaagctgaactttcagatgcctacactggccagaggctgggacgtgaatagagagaagaacaatggcgccatcctgtttgtgaagaacggcctgtactatctgggcatcatgccaaagcagaagggcaggtataaggccctgagcttcgagcccacagagaaaaccagcgagggctttgataagatgtactatgactacttccctgatgccgccaagatgatcccaaagtgcagcacccagctgaaggccgtgacagcccactttcagacccacacaacccccatcctgctgtccaacaatttcatcgagcctctggagatcacaaaggagatctacgacctgaacaatcctgagaaggagccaaagaagtttcagacagcctacgccaagaaaaccggcgaccagaagggctacagagaggccctgtgcaagtggatcgacttcacaagggattttctgtccaagtataccaagacaacctctatcgatctgtctagcctgcggccatcctctcagtataaggacctgggcgagtactatgccgagctgaatcccctgctgtaccacatcagcttccagagaatcgccgagaaggagatcatggatgccgtggagacaggcaagctgtacctgttccagatctataacaaggactttgccaagggccaccacggcaagcctaatctgcacacactgtattggaccggcctgttttctccagagaacctggccaagacaagcatcaagctgaatggccaggccgagctgttctaccgccctaagtccaggatgaagaggatggcacaccggctgggagagaagatgctgaacaagaagctgaaggatcagaaaaccccaatccccgacaccctgtaccaggagctgtacgactatgtgaatcacagactgtcccacgacctgtctgatgaggccagggccctgctgcccaacgtgatcaccaaggaggtgtctcacgagatcatcaaggataggcgctttaccagcgacaagttctttttccacgtgcctatcacactgaactatcaggccgccaattccccatctaagttcaaccagagggtgaatgcctacctgaaggagcaccccgagacacctatcatcggcatcgatcggggcgagagaaacctgatctatatcacagtgatcgactccaccggcaagatcctggagcagcggagcctgaacaccatccagcagtttgattaccagaagaagctggacaacagggagaaggagagggtggcagcaaggcaggcctggtctgtggtgggcacaatcaaggatctgaagcagggctatctgagccaggtcatccacgagatcgtggacctgatgatccactaccaggccgtggtggtgctggagaacctgaatttcggctttaagagcaagaggaccggcatcgccgagaaggccgtgtaccagcagttcgagaagatgctgatcgataagctgaattgcctggtgctgaaggactatccagcagagaaagtgggaggcgtgctgaacccataccagctgacagaccagttcacctcctttgccaagatgggcacccagtctggcttcctgttttacgtgcctgccccatatacatctaagatcgatcccctgaccggcttcgtggaccccttcgtgtggaaaaccatcaagaatcacgagagccgcaagcacttcctggagggcttcgactttctgcactacgacgtgaaaaccggcgacttcatcctgcactttaagatgaacagaaatctgtccttccagaggggcctgcccggctttatgcctgcatgggatatcgtgttcgagaagaacgagacacagtttgacgccaagggcacccctttcatcgccggcaagagaatcgtgccagtgatcgagaatcacagattcaccggcagataccgggacctgtatcctgccaacgagctgatcgccctgctggaggagaagggcatcgtgttcagggatggctccaacatcctgccaaagctgctggagaatgacgattctcacgccatcgacacgatggtggccctgatccgcagcgtgctgcagatgcggaactccaatgccgccacaggcgaggactatatcaacagccccgtgcgcgatctgaatggcgtgtgcttcgactcccggtttcagaacccagagtggccaatggacgccgatgccaatggcgcctaccacatcgccctgaagggccagctgctgctgaatcacctgaaggagagcaaggatctgaagctgcagaacggcatctccaatcaggactggctggcctacatccaggagctgcgcaacaaaaggccggcggccacgaaaaaggccggccaggcaaaaaagaaaaagggagcggccgcactcgagcaccaccaccaccaccactga

SEQ ID NO: 428 - DNA, 4011 bp, synthetic construct
  misc_feature 1..4011: note = Description of Artificial Sequence: Synthetic polynucleotide
  source 1..4011: mol_type = other DNA
atggggacacagttcgagggctttaccaacctgtatcaggtgagcaagacactgcggtttgagctgatcccacagggcaagaccctgaagcacatccaggagcagggcttcatcgaggaggacaaggcccgcaatgatcactacaaggagctgaagcccatcatcgatcggatctacaagacctatgccgaccagtgcctgcagctggtgcagctggattgggagaacctgagcgccgccatcgactcctatagaaaggagaaaaccgaggagacaaggaacgccctgatcgaggagcaggccacatatcgcaatgccatccacgactacttcatcggccggacagacaacctgaccgatgccatcaataagagacacgccgagatctacaagggcctgttcaaggccgagctgtttaatggcaaggtgctgaagcagctgggcaccgtgaccacaaccgagcacgagaacgccctgctgcggagcttcgacaagtttacaacctacttctccggcttttatagaaacaggaagaacgtgttcagcgccgaggatatcagcacagccatcccacaccgcatcgtgcaggacaacttccccaagtttaaggagaattgtcacatcttcacacgcctgatcaccgccgtgcccagcctgcgggagcactttgagaacgtgaagaaggccatcggcatcttcgtgagcacctccatcgaggaggtgttttccttccctttttataaccagctgctgacacagacccagatcgacctgtataaccagctgctgggaggaatctctcgggaggcaggcaccgagaagatcaagggcctgaacgaggtgctgaatctggccatccagaagaatgatgagacagcccacatcatcgcctccctgccacacagattcatccccctgtttaagcagatcctgtccgataggaacaccctgtctttcatcctggaggagtttaagagcgacgaggaagtgatccagtccttctgcaagtacaagacactgctgagaaacgagaacgtgctggagacagccgaggccctgtttaacgagctgaacagcatcgacctgacacacatcttcatcagccacaagaagctggagacaatcagcagcgccctgtgcgaccactgggatacactgaggaatgccctgtatgagcggagaatctccgagctgacaggcaagatcaccaagtctgccaaggagaaggtgcagcgcagcctgaagcacgaggatatcaacctgcaggagatcatctctgccgcaggcaaggagctgagcgaggccttcaagcagaaaaccagcgagatcctgtcccacgcacacgccgccctggatcagccactgcctacaaccctgaagaagcaggaggagaaggagatcctgaagtctcagctggacagcctgctgggcctgtaccacctgctggactggtttgccgtggatgagtccaacgaggtggaccccgagttctctgcccggctgaccggcatcaagctggagatggagccttctctgagcttctacaacaaggccagaaattatgccaccaagaagccctactccgtggagaagttcaagctgaactttcagatgcctacactggccagaggctgggacgtgaataaggagaagaacaatggcgccatcctgtttgtgaagaacggcctgtactatctgggcatcatgccaaagcagaagggcaggtataaggccctgagcttcgagcccacagagaaaaccagcgagggctttgataagatgtactatgactacttccctgatgccgccaagatgatcccaaagtgcagcacccagctgaaggccgtgacagcccactttcagacccacacaacccccatcctgctgtccaacaatttcatcgagcctctggagatcacaaaggagatctacgacctgaacaatcctgagaaggagccaaagaagtttcagacagcctacgccaagaaaaccggcgaccagaagggctacagagaggccctgtgcaagtggatcgacttcacaagggattttctgtccaagtataccaagacaacctctatcgatctgtctagcctgcggccatcctctcagtataaggacctgggcgagtactatgccgagctgaatcccctgctgtaccacatcagcttccagagaatcgccgagaaggagatcatggatgccgtggagacaggcaagctgtacctgttccagatctataacaaggactttgccaagggccaccacggcaagcctaatctgcacacactgtattggaccggcctgttttctccagagaacctggccaagacaagcatcaagctgaatggccaggccgagctgttctaccgccctaagtccaggatgaagaggatggcacaccggctgggagagaagatgctgaacaagaagctgaaggatcagaaaaccccaatccccgacaccctgtaccaggagctgtacgactatgtgaatcacagactgtcccacgacctgtctgatgaggccagggccctgctgcccaacgtgatcaccaaggaggtgtctcacgagatcatcaaggataggcgctttaccagcgacaagttctttttccacgtgcctatcacactgaactatcaggccgccaattccccatctaagttcaaccagagggtgaatgcctacctgaaggagcaccccgagacacctatcatcggcatcgatcggggcgagagaaacctgatctatatcacagtgatcgactccaccggcaagatcctggagcagcggagcctgaacaccatccagcagtttgattaccagaagaagctggacaacagggagaaggagagggtggcagcaaggcaggcctggtctgtggtgggcacaatcaaggatctgaagcagggctatctgagccaggtcatccacgagatcgtggacctgatgatccactaccaggccgtggtggtgctggagaacctgaatttcggctttaagagcaagaggaccggcatcgccgagaaggccgtgtaccagcagttcgagaagatgctgatcgataagctgaattgcctggtgctgaaggactatccagcagagaaagtgggaggcgtgctgaacccataccagctgacagaccagttcacctcctttgccaagatgggcacccagtctggcttcctgttttacgtgcctgccccatatacatctaagatcgatcccctgaccggcttcgtggaccccttcgtgtggaaaaccatcaagaatcacgagagccgcaagcacttcctggagggcttcgactttctgcactacgacgtgaaaaccggcgacttcatcctgcactttaagatgaacagaaatctgtccttccagaggggcctgcccggctttatgcctgcatgggatatcgtgttcgagaagaacgagacacagtttgacgccaagggcacccctttcatcgccggcaagagaatcgtgccagtgatcgagaatcacagattcaccggcagataccgggacctgtatcctgccaacgagctgatcgccctgctggaggagaagggcatcgtgttcagggatggctccaacatcctgccaaagctgctggagaatgacgattctcacgccatcgacacgatggtggccctgatccgcagcgtgctgcagatgcggaactccaatgccgccacaggcgaggactatatcaacagccccgtgcgcgatctgaatggcgtgtgcttcgactcccggtttcagaacccagagtggccaatggacgccgatgccaatggcgcctaccacatcgccctgaagggccagctgctgctgaatcacctgaaggagagcaaggatctgaagctgcagaacggcatctccaatcaggactggctggcctacatccaggagctgcgcaacaaaaggccggcggccacgaaaaaggccggccaggcaaaaaagaaaaagggagcggccgcactcgagcaccaccaccaccaccactga

SEQ ID NO: 429 - DNA, 4011 bp, synthetic construct
  misc_feature 1..4011: note = Description of Artificial Sequence: Synthetic polynucleotide
  source 1..4011: mol_type = other DNA
atggggacacagttcgagggctttaccaacctgtatcaggtgagcaagacactgcggtttgagctgatcccacagggcaagaccctgaagcacatccaggagcagggcttcatcgaggaggacaaggcccgcaatgatcactacaaggagctgaagcccatcatcgatcggatctacaagacctatgccgaccagtgcctgcagctggtgcagctggattgggagaacctgagcgccgccatcgactcctatagaaaggagaaaaccgaggagacaaggaacgccctgatcgaggagcaggccacatatcgcaatgccatccacgactacttcatcggccggacagacaacctgaccgatgccatcaataagagacacgccgagatctacaagggcctgttcaaggccgagctgtttaatggcaaggtgctgaagcagctgggcaccgtgaccacaaccgagcacgagaacgccctgctgcggagcttcgacaagtttacaacctacttctccggcttttatagaaacaggaagaacgtgttcagcgccgaggatatcagcacagccatcccacaccgcatcgtgcaggacaacttccccaagtttaaggagaattgtcacatcttcacacgcctgatcaccgccgtgcccagcctgcgggagcactttgagaacgtgaagaaggccatcggcatcttcgtgagcacctccatcgaggaggtgttttccttccctttttataaccagctgctgacacagacccagatcgacctgtataaccagctgctgggaggaatctctcgggaggcaggcaccgagaagatcaagggcctgaacgaggtgctggccctggccatccagaagaatgatgagacagcccacatcatcgcctccctgccacacagattcatccccctgtttaagcagatcctgtccgataggaacaccctgtctttcatcctggaggagtttaagagcgacgaggaagtgatccagtccttctgcaagtacaagacactgctgagaaacgagaacgtgctggagacagccgaggccctgtttaacgagctgaacagcatcgacctgacacacatcttcatcagccacaagaagctggagacaatcagcagcgccctgtgcgaccactgggatacactgaggaatgccctgtatgagcggagaatctccgagctgacaggcaagatcaccaagtctgccaaggagaaggtgcagcgcagcctgaagcacgaggatatcaacctgcaggagatcatctctgccgcaggcaaggagctgagcgaggccttcaagcagaaaaccagcgagatcctgtcccacgcacacgccgccctggatcagccactgcctacaaccctgaagaagcaggaggagaaggagatcctgaagtctcagctggacagcctgctgggcctgtaccacctgctggactggtttgccgtggatgagtccaacgaggtggaccccgagttctctgcccggctgaccggcatcaagctggagatggagccttctctgagcttctacaacaaggccagaaattatgccaccaagaagccctactccgtggagaagttcaagctgaactttcagatgcctacactggccagaggctgggacgtgaatagagagaagaacaatggcgccatcctgtttgtgaagaacggcctgtactatctgggcatcatgccaaagcagaagggcaggtataaggccctgagcttcgagcccacagagaaaaccagcgagggctttgataagatgtactatgactacttccctgatgccgccaagatgatcccaaagtgcagcacccagctgaaggccgtgacagcccactttcagacccacacaacccccatcctgctgtccaacaatttcatcgagcctctggagatcacaaaggagatctacgacctgaacaatcctgagaaggagccaaagaagtttcagacagcctacgccaagaaaaccggcgaccagaagggctacagagaggccctgtgcaagtggatcgacttcacaagggattttctgtccaagtataccaagacaacctctatcgatctgtctagcctgcggccatcctctcagtataaggacctgggcgagtactatgccgagctgaatcccctgctgtaccacatcagcttccagagaatcgccgagaaggagatcatggatgccgtggagacaggcaagctgtacctgttccagatctataacaaggactttgccaagggccaccacggcaagcctaatctgcacacactgtattggaccggcctgttttctccagagaacctggccaagacaagcatcaagctgaatggccaggccgagctgttctaccgccctaagtccaggatgaagaggatggcacaccggctgggagagaagatgctgaacaagaagctgaaggatcagaaaaccccaatccccgacaccctgtaccaggagctgtacgactatgtgaatcacagactgtcccacgacctgtctgatgaggccagggccctgctgcccaacgtgatcaccaaggaggtgtctcacgagatcatcaaggataggcgctttaccagcgacaagttctttttccacgtgcctatcacactgaactatcaggccgccaattccccatctaagttcaaccagagggtgaatgcctacctgaaggagcaccccgagacacctatcatcggcatcgatcggggcgagagaaacctgatctatatcacagtgatcgactccaccggcaagatcctggagcagcggagcctgaacaccatccagcagtttgattaccagaagaagctggacaacagggagaaggagagggtggcagcaaggcaggcctggtctgtggtgggcacaatcaaggatctgaagcagggctatctgagccaggtcatccacgagatcgtggacctgatgatccactaccaggccgtggtggtgctggagaacctgaatttcggctttaagagcaagaggaccggcatcgccgagaaggccgtgtaccagcagttcgagaagatgctgatcgataagctgaattgcctggtgctgaaggactatccagcagagaaagtgggaggcgtgctgaacccataccagctgacagaccagttcacctcctttgccaagatgggcacccagtctggcttcctgttttacgtgcctgccccatatacatctaagatcgatcccctgaccggcttcgtggaccccttcgtgtggaaaaccatcaagaatcacgagagccgcaagcacttcctggagggcttcgactttctgcactacgacgtgaaaaccggcgacttcatcctgcactttaagatgaacagaaatctgtccttccagaggggcctgcccggctttatgcctgcatgggatatcgtgttcgagaagaacgagacacagtttgacgccaagggcacccctttcatcgccggcaagagaatcgtgccagtgatcgagaatcacagattcaccggcagataccgggacctgtatcctgccaacgagctgatcgccctgctggaggagaagggcatcgtgttcagggatggctccaacatcctgccaaagctgctggagaatgacgattctcacgccatcgacacgatggtggccctgatccgcagcgtgctgcagatgcggaactccaatgccgccacaggcgaggactatatcaacagccccgtgcgcgatctgaatggcgtgtgcttcgactcccggtttcagaacccagagtggccaatggacgccgatgccaatggcgcctaccacatcgccctgaagggccagctgctgctgaatcacctgaaggagagcaaggatctgaagctgcagaacggcatctccaatcaggactggctggcctacatccaggagctgcgcaacaaaaggccggcggccacgaaaaaggccggccaggcaaaaaagaaaaagggagcggccgcactcgagcaccaccaccaccaccactga

SEQ ID NO: 430 - DNA, 4257 bp, synthetic construct
  misc_feature 1..4257: note = Description of Artificial Sequence: Synthetic polynucleotide
  source 1..4257: mol_type = other DNA
atgctgttccaggactttacccacctgtatccactgtccaagacagtgagatttgagctgaagcccatcgataggaccctggagcacatccacgccaagaacttcctgtctcaggacgagacaatggccgatatgcaccagaaggtgaaagtgatcctggacgattaccaccgcgacttcatcgccgatatgatgggcgaggtgaagctgaccaagctggccgagttctatgacgtgtacctgaagtttcggaagaacccaaaggacgatgagctgcagaagcagctgaaggatctgcaggccgtgctgagaaaggagatcgtgaagcccatcggcaatggcggcaagtataaggccggctacgacaggctgttcggcgccaagctgtttaaggacggcaaggagctgggcgatctggccaagttcgtgatcgcacaggagggagagagctccccaaagctggcccacctggcccacttcgagaagttttccacctatttcacaggctttcacgataaccggaagaatatgtattctgacgaggataagcacaccgccatcgcctaccgcctgatccacgagaacctgccccggtttatcgacaatctgcagatcctgaccacaatcaagcagaagcactctgccctgtacgatcagatcatcaacgagctgaccgccagcggcctggacgtgtctctggccagccacctggatggctatcacaagctgctgacacaggagggcatcaccgcctacaatacactgctgggaggaatctccggagaggcaggctctcctaagatccagggcatcaacgagctgatcaattctcaccacaaccagcactgccacaagagcgagagaatcgccaagctgaggccactgcacaagcagatcctgtccgacggcatgagcgtgtccttcctgccctctaagtttgccgacgatagcgagatgtgccaggccgtgaacgagttctatcgccactacgccgacgtgttcgccaaggtgcagagcctgttcgacggctttgacgatcaccagaaggatggcatctacgtggagcacaagaacctgaatgagctgtccaagcaggccttcggcgactttgcactgctgggacgcgtgctggacggatactatgtggatgtggtgaatccagagttcaacgagcggtttgccaaggccaagaccgacaatgccaaggccaagctgacaaaggagaaggataagttcatcaagggcgtgcactccctggcctctctggagcaggccatcgagcactataccgcaaggcacgacgatgagagcgtgcaggcaggcaagctgggacagtacttcaagcacggcctggccggagtggacaaccccatccagaagatccacaacaatcacagcaccatcaagggctttctggagagggagcgccctgcaggagagagagccctgccaaagatcaagtccggcaagaatcctgagatgacacagctgaggcagctgaaggagctgctggataacgccctgaatgtggcccacttcgccaagctgctgaccacaaagaccacactggacaatcaggatggcaacttctatggcgagtttggcgtgctgtacgacgagctggccaagatccccaccctgtataacaaggtgagagattacctgagccagaagcctttctccaccgagaagtacaagctgaactttggcaatccaacactgctgaatggctgggacctgaacaaggagaaggataatttcggcgtgatcctgcagaaggacggctgctactatctggccctgctggacaaggcccacaagaaggtgtttgataacgcccctaatacaggcaagagcatctatcagaagatgatctataagtacctggaggtgaggaagcagttccccaaggtgttcttttccaaggaggccatcgccatcaactaccacccttctaaggagctggtggagatcaaggacaagggccggcagagatccgacgatgagcgcctgaagctgtatcggtttatcctggagtgtctgaagatccaccctaagtacgataagaagttcgagggcgccatcggcgacatccagctgtttaagaaggataagaagggcagagaggtgccaatcagcgagaaggacctgttcgataagatcaacggcatcttttctagcaagcctaagctggagatggaggacttctttatcggcgagttcaagaggtataacccaagccaggacctggtggatcagtataatatctacaagaagatcgactccaacgataatcgcaagaaggagaatttctacaacaatcaccccaagtttaagaaggatctggtgcggtactattacgagtctatgtgcaagcacgaggagtgggaggagagcttcgagttttccaagaagctgcaggacatcggctgttacgtggatgtgaacgagctgtttaccgagatcgagacacggagactgaattataagatctccttctgcaacatcaatgccgactacatcgatgagctggtggagcagggccagctgtatctgttccagatctacaacaaggacttttccccaaaggcccacggcaagcccaatctgcacaccctgtacttcaaggccctgttttctgaggacaacctggccgatcctatctataagctgaatggcgaggcccagatcttctacagaaaggcctccctggacatgaacgagacaacaatccacagggccggcgaggtgctggagaacaagaatcccgataatcctaagaagagacagttcgtgtacgacatcatcaaggataagaggtacacacaggacaagttcatgctgcacgtgccaatcaccatgaactttggcgtgcagggcatgacaatcaaggagttcaataagaaggtgaaccagtctatccagcagtatgacgaggtgaacgtgatcggcatcgatcggggcgagagacacctgctgtacctgaccgtgatcaatagcaagggcgagatcctggagcagtgttccctgaacgacatcaccacagcctctgccaatggcacacagatgaccacaccttaccacaagatcctggataagagggagatcgagcgcctgaacgcccgggtgggatggggcgagatcgagacaatcaaggagctgaagtctggctatctgagccacgtggtgcaccagatcagccagctgatgctgaagtacaacgccatcgtggtgctggaggacctgaatttcggctttaagaggggccgctttaaggtggagaagcagatctatcagaacttcgagaatgccctgatcaagaagctgaaccacctggtgctgaaggacaaggccgacgatgagatcggctcttacaagaatgccctgcagctgaccaacaatttcacagatctgaagagcatcggcaagcagaccggcttcctgttttatgtgcccgcctggaacacctctaagatcgaccctgagacaggctttgtggatctgctgaagccaagatacgagaacatcgcccagagccaggccttctttggcaagttcgacaagatctgctataatgccgacaaggattacttcgagtttcacatcgactacgccaagtttaccgataaggccaagaatagccgccagatctggacaatctgttcccacggcgacaagcggtacgtgtacgataagacagccaaccagaataagggcgccgccaagggcatcaacgtgaatgatgagctgaagtccctgttcgcccgccaccacatcaacgagaagcagcccaacctggtcatggacatctgccagaacaatgataaggagtttcacaagtctctgatgtacctgctgaaaaccctgctggccctgcggtacagcaacgcctcctctgacgaggatttcatcctgtcccccgtggcaaacgacgagggcgtgttctttaatagcgccctggccgacgatacacagcctcagaatgccgatgccaacggcgcctaccacatcgccctgaagggcctgtggctgctgaatgagctgaagaactccgacgatctgaacaaggtgaagctggccatcgacaatcagacctggctgaatttcgcccagaacaggaaaaggccggcggccacgaaaaaggccggccaggcaaaaaagaaaaagggatcctacccatacgatgttccagattacgcttatccctacgacgtgcctgattatgcatacccatatgatgtccccgactatgcctaa

SEQ ID NO: 431 - DNA, 5658 bp, synthetic construct
  misc_feature 1..5658: note = Description of Artificial Sequence: Synthetic polynucleotide
  source 1..5658: mol_type = other DNA
atgacacagttcgagggctttaccaacctgtatcaggtgagcaagacactgcggtttgagctgatcccacagggcaagaccctgaagcacatccaggagcagggcttcatcgaggaggacaaggcccgcaatgatcactacaaggagctgaagcccatcatcgatcggatctacaagacctatgccgaccagtgcctgcagctggtgcagctggattgggagaacctgagcgccgccatcgactcctatagaaaggagaaaaccgaggagacaaggaacgccctgatcgaggagcaggccacatatcgcaatgccatccacgactacttcatcggccggacagacaacctgaccgatgccatcaataagagacacgccgagatctacaagggcctgttcaaggccgagctgtttaatggcaaggtgctgaagcagctgggcaccgtgaccacaaccgagcacgagaacgccctgctgcggagcttcgacaagtttacaacctacttctccggcttttatgagaacaggaagaacgtgttcagcgccgaggatatcagcacagccatcccacaccgcatcgtgcaggacaacttccccaagtttaaggagaattgtcacatcttcacacgcctgatcaccgccgtgcccagcctgcgggagcactttgagaacgtgaagaaggccatcggcatcttcgtgagcacctccatcgaggaggtgttttccttccctttttataaccagctgctgacacagacccagatcgacctgtataaccagctgctgggaggaatctctcgggaggcaggcaccgagaagatcaagggcctgaacgaggtgctgaatctggccatccagaagaatgatgagacagcccacatcatcgcctccctgccacacagattcatccccctgtttaagcagatcctgtccgataggaacaccctgtctttcatcctggaggagtttaagagcgacgaggaagtgatccagtccttctgcaagtacaagacactgctgagaaacgagaacgtgctggagacagccgaggccctgtttaacgagctgaacagcatcgacctgacacacatcttcatcagccacaagaagctggagacaatcagcagcgccctgtgcgaccactgggatacactgaggaatgccctgtatgagcggagaatctccgagctgacaggcaagatcaccaagtctgccaaggagaaggtgcagcgcagcctgaagcacgaggatatcaacctgcaggagatcatctctgccgcaggcaaggagctgagcgaggccttcaagcagaaaaccagcgagatcctgtcccacgcacacgccgccctggatcagccactgcctacaaccctgaagaagcaggaggagaaggagatcctgaagtctcagctggacagcctgctgggcctgtaccacctgctggactggtttgccgtggatgagtccaacgaggtggaccccgagttctctgcccggctgaccggcatcaagctggagatggagccttctctgagcttctacaacaaggccagaaattatgccaccaagaagccctactccgtggagaagttcaagctgaactttcagatgcctacactggcctctggctgggacgtgaataaggagaagaacaatggcgccatcctgtttgtgaagaacggcctgtactatctgggcatcatgccaaagcagaagggcaggtataaggccctgagcttcgagcccacagagaaaaccagcgagggctttgataagatgtactatgactacttccctgatgccgccaagatgatcccaaagtgcagcacccagctgaaggccgtgacagcccactttcagacccacacaacccccatcctgctgtccaacaatttcatcgagcctctggagatcacaaaggagatctacgacctgaacaatcctgagaaggagccaaagaagtttcagacagcctacgccaagaaaaccggcgaccagaagggctacagagaggccctgtgcaagtggatcgacttcacaagggattttctgtccaagtataccaagacaacctctatcgatctgtctagcctgcggccatcctctcagtataaggacctgggcgagtactatgccgagctgaatcccctgctgtaccacatcagcttccagagaatcgccgagaaggagatcatggatgccgtggagacaggcaagctgtacctgttccagatctataacaaggactttgccaagggccaccacggcaagcctaatctgcacacactgtattggaccggcctgttttctccagagaacctggccaagacaagcatcaagctgaatggccaggccgagctgttctaccgccctaagtccaggatgaagaggatggcacaccggctgggagagaagatgctgaacaagaagctgaaggatcagaaaaccccaatccccgacaccctgtaccaggagctgtacgactatgtgaatcacagactgtcccacgacctgtctgatgaggccagggccctgctgcccaacgtgatcaccaaggaggtgtctcacgagatcatcaaggataggcgctttaccagcgacaagttctttttccacgtgcctatcacactgaactatcaggccgccaattccccatctaagttcaaccagagggtgaatgcctacctgaaggagcaccccgagacacctatcatcggcatcgcccggggcgagagaaacctgatctatatcacagtgatcgactccaccggcaagatcctggagcagcggagcctgaacaccatccagcagtttgattaccagaagaagctggacaacagggagaaggagagggtggcagcaaggcaggcctggtctgtggtgggcacaatcaaggatctgaagcagggctatctgagccaggtcatccacgagatcgtggacctgatgatccactaccaggccgtggtggtgctggagaacctgaatttcggctttaagagcaagaggaccggcatcgccgagaaggccgtgtaccagcagttcgagaagatgctgatcgataagctgaattgcctggtgctgaaggactatccagcagagaaagtgggaggcgtgctgaacccataccagctgacagaccagttcacctcctttgccaagatgggcacccagtctggcttcctgttttacgtgcctgccccatatacatctaagatcgatcccctgaccggcttcgtggaccccttcgtgtggaaaaccatcaagaatcacgagagccgcaagcacttcctggagggcttcgactttctgcactacgacgtgaaaaccggcgacttcatcctgcactttaagatgaacagaaatctgtccttccagaggggcctgcccggctttatgcctgcatgggatatcgtgttcgagaagaacgagacacagtttgacgccaagggcacccctttcatcgccggcaagagaatcgtgccagtgatcgagaatcacagattcaccggcagataccgggacctgtatcctgccaacgagctgatcgccctgctggaggagaagggcatcgtgttcagggatggctccaacatcctgccaaagctgctggagaatgacgattctcacgccatcgacaccatggtggccctgatccgcagcgtgctgcagatgcggaactccaatgccgccacaggcgaggactatatcaacagccccgtgcgcgatctgaatggcgtgtgcttcgactcccggtttcagaacccagagtggcccatggacgccgatgccaatggcgcctaccacatcgccctgaagggccagctgctgctgaatcacctgaaggagagcaaggatctgaagctgcagaacggcatctccaatcaggactggctggcctacatccaggagctgcgcaacaaaaggccggcggccacgaaaaaggccggccaggcaaaaaagaaaaagggatcctacccatacgatgttccagattacgcttatccctacgacgtgcctgattatgcatacccatatgatgtccccgactatgccggaagcgaggccagcggttccggacgggctgacgcattggacgattttgatctggatatgctgggaagtgacgccctcgatgattttgaccttgacatgcttggttcggatgcccttgatgactttgacctcgacatgctcggcagtgacgcccttgatgatttcgacctggacatgctgattaactctagaagttccggatctccgaaaaagaaacgcaaagttggtagccagtacctgcccgacaccgacgaccggcaccggatcgaggaaaagcggaagcggacctacgagacattcaagagcatcatgaagaagtcccccttcagcggccccaccgaccctagacctccacctagaagaatcgccgtgcccagcagatccagcgccagcgtgccaaaacctgccccccagccttaccccttcaccagcagcctgagcaccatcaactacgacgagttccctaccatggtgttccccagcggccagatctctcaggcctctgctctggctccagcccctcctcaggtgctgcctcaggctcctgctcctgcaccagctccagccatggtgtctgcactggctcaggcaccagcacccgtgcctgtgctggctcctggacctccacaggctgtggctccaccagcccctaaacctacacaggccggcgagggcacactgtctgaagctctgctgcagctgcagttcgacgacgaggatctgggagccctgctgggaaacagcaccgatcctgccgtgttcaccgacctggccagcgtggacaacagcgagttccagcagctgctgaaccagggcatccctgtggcccctcacaccaccgagcccatgctgatggaataccccgaggccatcacccggctcgtgacaggcgctcagaggcctcctgatccagctcctgcccctctgggagcaccaggcctgcctaatggactgctgtctggcgacgaggacttcagctctatcgccgatatggatttctcagccttgctgggctctggcagcggcagccgggattccagggaagggatgtttttgccgaagcctgaggccggctccgctattagtgacgtgtttgagggccgcgaggtgtgccagccaaaacgaatccggccatttcatcctccaggaagtccatgggccaaccgcccactccccgccagcctcgcaccaacaccaaccggtccagtacatgagccagtcgggtcactgaccccggcaccagtccctcagccactggatccagcgcccgcagtgactcccgaggccagtcacctgttggaggatcccgatgaagagacgagccaggctgtcaaagcccttcgggagatggccgatactgtgattccccagaaggaagaggctgcaatctgtggccaaatggacctttcccatccgcccccaaggggccatctggatgagctgacaaccacacttgagtccatgaccgaggatctgaacctggactcacccctgaccccggaattgaacgagattctggataccttcctgaacgacgagtgcctcttgcatgccatgcatatcagcacaggactgtccatcttcgacacatctctgttttaa

SEQ ID NO: 432 - protein, 1885 aa, synthetic construct
  REGION 1..1885: note = Description of Artificial Sequence: Synthetic polypeptide
MTQFEGFTNLYQVSKTLRFELIPQGKTLKHIQEQGFIEEDKARNDHYKELKPIIDRIYKTYADQCLQLVQLDWENLSAAIDSYRKEKTEETRNALIEEQATYRNAIHDYFIGRTDNLTDAINKRHAEIYKGLFKAELFNGKVLKQLGTVTTTEHENALLRSFDKFTTYFSGFYENRKNVFSAEDISTAIPHRIVQDNFPKFKENCHIFTRLITAVPSLREHFENVKKAIGIFVSTSIEEVFSFPFYNQLLTQTQIDLYNQLLGGISREAGTEKIKGLNEVLNLAIQKNDETAHIIASLPHRFIPLFKQILSDRNTLSFILEEFKSDEEVIQSFCKYKTLLRNENVLETAEALFNELNSIDLTHIFISHKKLETISSALCDHWDTLRNALYERRISELTGKITKSAKEKVQRSLKHEDINLQEIISAAGKELSEAFKQKTSEILSHAHAALDQPLPTTLKKQEEKEILKSQLDSLLGLYHLLDWFAVDESNEVDPEFSARLTGIKLEMEPSLSFYNKARNYATKKPYSVEKFKLNFQMPTLASGWDVNKEKNNGAILFVKNGLYYLGIMPKQKGRYKALSFEPTEKTSEGFDKMYYDYFPDAAKMIPKCSTQLKAVTAHFQTHTTPILLSNNFIEPLEITKEIYDLNNPEKEPKKFQTAYAKKTGDQKGYREALCKWIDFTRDFLSKYTKTTSIDLSSLRPSSQYKDLGEYYAELNPLLYHISFQRIAEKEIMDAVETGKLYLFQIYNKDFAKGHHGKPNLHTLYWTGLFSPENLAKTSIKLNGQAELFYRPKSRMKRMAHRLGEKMLNKKLKDQKTPIPDTLYQELYDYVNHRLSHDLSDEARALLPNVITKEVSHEIIKDRRFTSDKFFFHVPITLNYQAANSPSKFNQRVNAYLKEHPETPIIGIARGERNLIYITVIDSTGKILEQRSLNTIQQFDYQKKLDNREKERVAARQAWSVVGTIKDLKQGYLSQVIHEIVDLMIHYQAVVVLENLNFGFKSKRTGIAEKAVYQQFEKMLIDKLNCLVLKDYPAEKVGGVLNPYQLTDQFTSFAKMGTQSGFLFYVPAPYTSKIDPLTGFVDPFVWKTIKNHESRKHFLEGFDFLHYDVKTGDFILHFKMNRNLSFQRGLPGFMPAWDIVFEKNETQFDAKGTPFIAGKRIVPVIENHRFTGRYRDLYPANELIALLEEKGIVFRDGSNILPKLLENDDSHAIDTMVALIRSVLQMRNSNAATGEDYINSPVRDLNGVCFDSRFQNPEWPMDADANGAYHIALKGQLLLNHLKESKDLKLQNGISNQDWLAYIQELRNKRPAATKKAGQAKKKKGSYPYDVPDYAYPYDVPDYAYPYDVPDYAGSEASGSGRADALDDFDLDMLGSDALDDFDLDMLGSDALDDFDLDMLGSDALDDFDLDMLINSRSSGSPKKKRKVGSQYLPDTDDRHRIEEKRKRTYETFKSIMKKSPFSGPTDPRPPPRRIAVPSRSSASVPKPAPQPYPFTSSLSTINYDEFPTMVFPSGQISQASALAPAPPQVLPQAPAPAPAPAMVSALAQAPAPVPVLAPGPPQAVAPPAPKPTQAGEGTLSEALLQLQFDDEDLGALLGNSTDPAVFTDLASVDNSEFQQLLNQGIPVAPHTTEPMLMEYPEAITRLVTGAQRPPDPAPAPLGAPGLPNGLLSGDEDFSSIADMDFSALLGSGSGSRDSREGMFLPKPEAGSAISDVFEGREVCQPKRIRPFHPPGSPWANRPLPASLAPTPTGPVHEPVGSLTPAPVPQPLDPAPAVTPEASHLLEDPDEETSQAVKALREMADTVIPQKEEAAICGQMDLSHPPPRGHLDELTTTLESMTEDLNLDSPLTPELNEILDTFLNDECLLHAMHISTGLSIFDTSLF

SEQ ID NO: 433 - DNA, 5655 bp, synthetic construct
  misc_feature 1..5655: note = Description of Artificial Sequence: Synthetic polynucleotide
  source 1..5655: mol_type = other DNA
atgacacagttcgagggctttaccaacctgtatcaggtgagcaagacactgcggtttgagctgatcccacagggcaagaccctgaagcacatccaggagcagggcttcatcgaggaggacaaggcccgcaatgatcactacaaggagctgaagcccatcatcgatcggatctacaagacctatgccgaccagtgcctgcagctggtgcagctggattgggagaacctgagcgccgccatcgactcctatagaaaggagaaaaccgaggagacaaggaacgccctgatcgaggagcaggccacatatcgcaatgccatccacgactacttcatcggccggacagacaacctgaccgatgccatcaataagagacacgccgagatctacaagggcctgttcaaggccgagctgtttaatggcaaggtgctgaagcagctgggcaccgtgaccacaaccgagcacgagaacgccctgctgcggagcttcgacaagtttacaacctacttctccggcttttatagaaacaggaagaacgtgttcagcgccgaggatatcagcacagccatcccacaccgcatcgtgcaggacaacttccccaagtttaaggagaattgtcacatcttcacacgcctgatcaccgccgtgcccagcctgcgggagcactttgagaacgtgaagaaggccatcggcatcttcgtgagcacctccatcgaggaggtgttttccttccctttttataaccagctgctgacacagacccagatcgacctgtataaccagctgctgggaggaatctctcgggaggcaggcaccgagaagatcaagggcctgaacgaggtgctgaatctggccatccagaagaatgatgagacagcccacatcatcgcctccctgccacacagattcatccccctgtttaagcagatcctgtccgataggaacaccctgtctttcatcctggaggagtttaagagcgacgaggaagtgatccagtccttctgcaagtacaagacactgctgagaaacgagaacgtgctggagacagccgaggccctgtttaacgagctgaacagcatcgacctgacacacatcttcatcagccacaagaagctggagacaatcagcagcgccctgtgcgaccactgggatacactgaggaatgccctgtatgagcggagaatctccgagctgacaggcaagatcaccaagtctgccaaggagaaggtgcagcgcagcctgaagcacgaggatatcaacctgcaggagatcatctctgccgcaggcaaggagctgagcgaggccttcaagcagaaaaccagcgagatcctgtcccacgcacacgccgccctggatcagccactgcctacaaccctgaagaagcaggaggagaaggagatcctgaagtctcagctggacagcctgctgggcctgtaccacctgctggactggtttgccgtggatgagtccaacgaggtggaccccgagttctctgcccggctgaccggcatcaagctggagatggagccttctctgagcttctacaacaaggccagaaattatgccaccaagaagccctactccgtggagaagttcaagctgaactttcagatgcctacactggccagaggctgggacgtgaatagagagaagaacaatggcgccatcctgtttgtgaagaacggcctgtactatctgggcatcatgccaaagcagaagggcaggtataaggccctgagcttcgagcccacagagaaaaccagcgagggctttgataagatgtactatgactacttccctgatgccgccaagatgatcccaaagtgcagcacccagctgaaggccgtgacagcccactttcagacccacacaacccccatcctgctgtccaacaatttcatcgagcctctggagatcacaaaggagatctacgacctgaacaatcctgagaaggagccaaagaagtttcagacagcctacgccaagaaaaccggcgaccagaagggctacagagaggccctgtgcaagtggatcgacttcacaagggattttctgtccaagtataccaagacaacctctatcgatctgtctagcctgcggccatcctctcagtataaggacctgggcgagtactatgccgagctgaatcccctgctgtaccacatcagcttccagagaatcgccgagaaggagatcatggatgccgtggagacaggcaagctgtacctgttccagatctataacaaggactttgccaagggccaccacggcaagcctaatctgcacacactgtattggaccggcctgttttctccagagaacctggccaagacaagcatcaagctgaatggccaggccgagctgttctaccgccctaagtccaggatgaagaggatggcacaccggctgggagagaagatgctgaacaagaagctgaaggatcagaaaaccccaatccccgacaccctgtaccaggagctgtacgactatgtgaatcacagactgtcccacgacctgtctgatgaggccagggccctgctgcccaacgtgatcaccaaggaggtgtctcacgagatcatcaaggataggcgctttaccagcgacaagttctttttccacgtgcctatcacactgaactatcaggccgccaattccccatctaagttcaaccagagggtgaatgcctacctgaaggagcaccccgagacacctatcatcggcatcgcccggggcgagagaaacctgatctatatcacagtgatcgactccaccggcaagatcctggagcagcggagcctgaacaccatccagcagtttgattaccagaagaagctggacaacagggagaaggagagggtggcagcaaggcaggcctggtctgtggtgggcacaatcaaggatctgaagcagggctatctgagccaggtcatccacgagatcgtggacctgatgatccactaccaggccgtggtggtgctggagaacctgaatttcggctttaagagcaagaggaccggcatcgccgagaaggccgtgtaccagcagttcgagaagatgctgatcgataagctgaattgcctggtgctgaaggactatccagcagagaaagtgggaggcgtgctgaacccataccagctgacagaccagttcacctcctttgccaagatgggcacccagtctggcttcctgttttacgtgcctgccccatatacatctaagatcgatcccctgaccggcttcgtggaccccttcgtgtggaaaaccatcaagaatcacgagagccgcaagcacttcctggagggcttcgactttctgcactacgacgtgaaaaccggcgacttcatcctgcactttaagatgaacagaaatctgtccttccagaggggcctgcccggctttatgcctgcatgggatatcgtgttcgagaagaacgagacacagtttgacgccaagggcacccctttcatcgccggcaagagaatcgtgccagtgatcgagaatcacagattcaccggcagataccgggacctgtatcctgccaacgagctgatcgccctgctggaggagaagggcatcgtgttcagggatggctccaacatcctgccaaagctgctggagaatgacgattctcacgccatcgacaccatggtggccctgatccgcagcgtgctgcagatgcggaactccaatgccgccacaggcgaggactatatcaacagccccgtgcgcgatctgaatggcgtgtgcttcgactcccggtttcagaacccagagtggcccatggacgccgatgccaatggcgcctaccacatcgccctgaagggccagctgctgctgaatcacctgaaggagagcaaggatctgaagctgcagaacggcatctccaatcaggactggctggcctacatccaggagctgcgcaacaaaaggccggcggccacgaaaaaggccggccaggcaaaaaagaaaaagggatcctacccatacgatgttccagattacgcttatccctacgacgtgcctgattatgcatacccatatgatgtccccgactatgccggaagcgaggccagcggttccggacgggctgacgcattggacgattttgatctggatatgctgggaagtgacgccctcgatgattttgaccttgacatgcttggttcggatgcccttgatgactttgacctcgacatgctcggcagtgacgcccttgatgatttcgacctggacatgctgattaactctagaagttccggatctccgaaaaagaaacgcaaagttggtagccagtacctgcccgacaccgacgaccggcaccggatcgaggaaaagcggaagcggacctacgagacattcaagagcatcatgaagaagtcccccttcagcggccccaccgaccctagacctccacctagaagaatcgccgtgcccagcagatccagcgccagcgtgccaaaacctgccccccagccttaccccttcaccagcagcctgagcaccatcaactacgacgagttccctaccatggtgttccccagcggccagatctctcaggcctctgctctggctccagcccctcctcaggtgctgcctcaggctcctgctcctgcaccagctccagccatggtgtctgcactggctcaggcaccagcacccgtgcctgtgctggctcctggacctccacaggctgtggctccaccagcccctaaacctacacaggccggcgagggcacactgtctgaagctctgctgcagctgcagttcgacgacgaggatctgggagccctgctgggaaacagcaccgatcctgccgtgttcaccgacctggccagcgtggacaacagcgagttccagcagctgctgaaccagggcatccctgtggcccctcacaccaccgagcccatgctgatggaataccccgaggccatcacccggctcgtgacaggcgctcagaggcctcctgatccagctcctgcccctctgggagcaccaggcctgcctaatggactgctgtctggcgacgaggacttcagctctatcgccgatatggatttctcagccttgctgggctctggcagcggcagccgggattccagggaagggatgtttttgccgaagcctgaggccggctccgctattagtgacgtgtttgagggccgcgaggtgtgccagccaaaacgaatccggccatttcatcctccaggaagtccatgggccaaccgcccactccccgccagcctcgcaccaacaccaaccggtccagtacatgagccagtcgggtcactgaccccggcaccagtccctcagccactggatccagcgcccgcagtgactcccgaggccagtcacctgttggaggatcccgatgaagagacgagccaggctgtcaaagcccttcgggagatggccgatactgtgattccccagaaggaagaggctgcaatctgtggccaaatggacctttcccatccgcccccaaggggccatctggatgagctgacaaccacacttgagtccatgaccgaggatctgaacctggactcacccctgaccccggaattgaacgagattctggataccttcctgaacgacgagtgcctcttgcatgccatgcatatcagcacaggactgtccatcttcgacacatctctgttt

SEQ ID NO: 434 - protein, 1885 aa, synthetic construct
  REGION 1..1885: note = Description of Artificial Sequence: Synthetic polypeptide
MTQFEGFTNLYQVSKTLRFELIPQGKTLKHIQEQGFIEEDKARNDHYKELKPIIDRIYKTYADQCLQLVQLDWENLSAAIDSYRKEKTEETRNALIEEQATYRNAIHDYFIGRTDNLTDAINKRHAEIYKGLFKAELFNGKVLKQLGTVTTTEHENALLRSFDKFTTYFSGFYRNRKNVFSAEDISTAIPHRIVQDNFPKFKENCHIFTRLITAVPSLREHFENVKKAIGIFVSTSIEEVFSFPFYNQLLTQTQIDLYNQLLGGISREAGTEKIKGLNEVLNLAIQKNDETAHIIASLPHRFIPLFKQILSDRNTLSFILEEFKSDEEVIQSFCKYKTLLRNENVLETAEALFNELNSIDLTHIFISHKKLETISSALCDHWDTLRNALYERRISELTGKITKSAKEKVQRSLKHEDINLQEIISAAGKELSEAFKQKTSEILSHAHAALDQPLPTTLKKQEEKEILKSQLDSLLGLYHLLDWFAVDESNEVDPEFSARLTGIKLEMEPSLSFYNKARNYATKKPYSVEKFKLNFQMPTLARGWDVNKEKNNGAILFVKNGLYYLGIMPKQKGRYKALSFEPTEKTSEGFDKMYYDYFPDAAKMIPKCSTQLKAVTAHFQTHTTPILLSNNFIEPLEITKEIYDLNNPEKEPKKFQTAYAKKTGDQKGYREALCKWIDFTRDFLSKYTKTTSIDLSSLRPSSQYKDLGEYYAELNPLLYHISFQRIAEKEIMDAVETGKLYLFQIYNKDFAKGHHGKPNLHTLYWTGLFSPENLAKTSIKLNGQAELFYRPKSRMKRMAHRLGEKMLNKKLKDQKTPIPDTLYQELYDYVNHRLSHDLSDEARALLPNVITKEVSHEIIKDRRFTSDKFFFHVPITLNYQAANSPSKFNQRVNAYLKEHPETPIIGIARGERNLIYITVIDSTGKILEQRSLNTIQQFDYQKKLDNREKERVAARQAWSVVGTIKDLKQGYLSQVIHEIVDLMIHYQAVVVLENLNFGFKSKRTGIAEKAVYQQFEKMLIDKLNCLVLKDYPAEKVGGVLNPYQLTDQFTSFAKMGTQSGFLFYVPAPYTSKIDPLTGFVDPFVWKTIKNHESRKHFLEGFDFLHYDVKTGDFILHFKMNRNLSFQRGLPGFMPAWDIVFEKNETQFDAKGTPFIAGKRIVPVIENHRFTGRYRDLYPANELIALLEEKGIVFRDGSNILPKLLENDDSHAIDTMVALIRSVLQMRNSNAATGEDYINSPVRDLNGVCFDSRFQNPEWPMDADANGAYHIALKGQLLLNHLKESKDLKLQNGISNQDWLAYIQELRNKRPAATKKAGQAKKKKGSYPYDVPDYAYPYDVPDYAYPYDVPDYAGSEASGSGRADALDDFDLDMLGSDALDDFDLDMLGSDALDDFDLDMLGSDALDDFDLDMLINSRSSGSPKKKRKVGSQYLPDTDDRHRIEEKRKRTYETFKSIMKKSPFSGPTDPRPPPRRIAVPSRSSASVPKPAPQPYPFTSSLSTINYDEFPTMVFPSGQISQASALAPAPPQVLPQAPAPAPAPAMVSALAQAPAPVPVLAPGPPQAVAPPAPKPTQAGEGTLSEALLQLQFDDEDLGALLGNSTDPAVFTDLASVDNSEFQQLLNQGIPVAPHTTEPMLMEYPEAITRLVTGAQRPPDPAPAPLGAPGLPNGLLSGDEDFSSIADMDFSALLGSGSGSRDSREGMFLPKPEAGSAISDVFEGREVCQPKRIRPFHPPGSPWANRPLPASLAPTPTGPVHEPVGSLTPAPVPQPLDPAPAVTPEASHLLEDPDEETSQAVKALREMADTVIPQKEEAAICGQMDLSHPPPRGHLDELTTTLESMTEDLNLDSPLTPELNEILDTFLNDECLLHAMHISTGLSIFDTSLF

SEQ ID NO: 435 - DNA, 5721 bp, synthetic construct
  misc_feature 1..5721: note = Description of Artificial Sequence: Synthetic polynucleotide
  source 1..5721: mol_type = other DNA
atgggcccaaagaaaaagaggaaagtcggcagtggacctaaaaagaaacgaaaggttgggtcaggtacacagttcgagggctttaccaacctgtatcaggtgagcaagacactgcggtttgagctgatcccacagggcaagaccctgaagcacatccaggagcagggcttcatcgaggaggacaaggcccgcaatgatcactacaaggagctgaagcccatcatcgatcggatctacaagacctatgccgaccagtgcctgcagctggtgcagctggattgggagaacctgagcgccgccatcgactcctatagaaaggagaaaaccgaggagacaaggaacgccctgatcgaggagcaggccacatatcgcaatgccatccacgactacttcatcggccggacagacaacctgaccgatgccatcaataagagacacgccgagatctacaagggcctgttcaaggccgagctgtttaatggcaaggtgctgaagcagctgggcaccgtgaccacaaccgagcacgagaacgccctgctgcggagcttcgacaagtttacaacctacttctccggcttttatagaaacaggaagaacgtgttcagcgccgaggatatcagcacagccatcccacaccgcatcgtgcaggacaacttccccaagtttaaggagaattgtcacatcttcacacgcctgatcaccgccgtgcccagcctgcgggagcactttgagaacgtgaagaaggccatcggcatcttcgtgagcacctccatcgaggaggtgttttccttccctttttataaccagctgctgacacagacccagatcgacctgtataaccagctgctgggaggaatctctcgggaggcaggcaccgagaagatcaagggcctgaacgaggtgctgaatctggccatccagaagaatgatgagacagcccacatcatcgcctccctgccacacagattcatccccctgtttaagcagatcctgtccgataggaacaccctgtctttcatcctggaggagtttaagagcgacgaggaagtgatccagtccttctgcaagtacaagacactgctgagaaacgagaacgtgctggagacagccgaggccctgtttaacgagctgaacagcatcgacctgacacacatcttcatcagccacaagaagctggagacaatcagcagcgccctgtgcgaccactgggatacactgaggaatgccctgtatgagcggagaatctccgagctgacaggcaagatcaccaagtctgccaaggagaaggtgcagcgcagcctgaagcacgaggatatcaacctgcaggagatcatctctgccgcaggcaaggagctgagcgaggccttcaagcagaaaaccagcgagatcctgtcccacgcacacgccgccctggatcagccactgcctacaaccctgaagaagcaggaggagaaggagatcctgaagtctcagctggacagcctgctgggcctgtaccacctgctggactggtttgccgtggatgagtccaacgaggtggaccccgagttctctgcccggctgaccggcatcaagctggagatggagccttctctgagcttctacaacaaggccagaaattatgccaccaagaagccctactccgtggagaagttcaagctgaactttcagatgcctacactggccagaggctgggacgtgaatagagagaagaacaatggcgccatcctgtttgtgaagaacggcctgtactatctgggcatcatgccaaagcagaagggcaggtataaggccctgagcttcgagcccacagagaaaaccagcgagggctttgataagatgtactatgactacttccctgatgccgccaagatgatcccaaagtgcagcacccagctgaaggccgtgacagcccactttcagacccacacaacccccatcctgctgtccaacaatttcatcgagcctctggagatcacaaaggagatctacgacctgaacaatcctgagaaggagccaaagaagtttcagacagcctacgccaagaaaaccggcgaccagaagggctacagagaggccctgtgcaagtggatcgacttcacaagggattttctgtccaagtataccaagacaacctctatcgatctgtctagcctgcggccatcctctcagtataaggacctgggcgagtactatgccgagctgaatcccctgctgtaccacatcagcttccagagaatcgccgagaaggagatcatggatgccgtggagacaggcaagctgtacctgttccagatctataacaaggactttgccaagggccaccacggcaagcctaatctgcacacactgtattggaccggcctgttttctccagagaacctggccaagacaagcatcaagctgaatggccaggccgagctgttctaccgccctaagtccaggatgaagaggatggcacaccggctgggagagaagatgctgaacaagaagctgaaggatcagaaaaccccaatccccgacaccctgtaccaggagctgtacgactatgtgaatcacagactgtcccacgacctgtctgatgaggccagggccctgctgcccaacgtgatcaccaaggaggtgtctcacgagatcatcaaggataggcgctttaccagcgacaagttctttttccacgtgcctatcacactgaactatcaggccgccaattccccatctaagttcaaccagagggtgaatgcctacctgaaggagcaccccgagacacctatcatcggcatcgcccggggcgagagaaacctgatctatatcacagtgatcgactccaccggcaagatcctggagcagcggagcctgaacaccatccagcagtttgattaccagaagaagctggacaacagggagaaggagagggtggcagcaaggcaggcctggtctgtggtgggcacaatcaaggatctgaagcagggctatctgagccaggtcatccacgagatcgtggacctgatgatccactaccaggccgtggtggtgctggagaacctgaatttcggctttaagagcaagaggaccggcatcgccgagaaggccgtgtaccagcagttcgagaagatgctgatcgataagctgaattgcctggtgctgaaggactatccagcagagaaagtgggaggcgtgctgaacccataccagctgacagaccagttcacctcctttgccaagatgggcacccagtctggcttcctgttttacgtgcctgccccatatacatctaagatcgatcccctgaccggcttcgtggaccccttcgtgtggaaaaccatcaagaatcacgagagccgcaagcacttcctggagggcttcgactttctgcactacgacgtgaaaaccggcgacttcatcctgcactttaagatgaacagaaatctgtccttccagaggggcctgcccggctttatgcctgcatgggatatcgtgttcgagaagaacgagacacagtttgacgccaagggcacccctttcatcgccggcaagagaatcgtgccagtgatcgagaatcacagattcaccggcagataccgggacctgtatcctgccaacgagctgatcgccctgctggaggagaagggcatcgtgttcagggatggctccaacatcctgccaaagctgctggagaatgacgattctcacgccatcgacacgatggtggccctgatccgcagcgtgctgcagatgcggaactccaatgccgccacaggcgaggactatatcaacagccccgtgcgcgatctgaatggcgtgtgcttcgactcccggtttcagaacccagagtggccaatggacgccgatgccaatggcgcctaccacatcgccctgaagggccagctgctgctgaatcacctgaaggagagcaaggatctgaagctgcagaacggcatctccaatcaggactggctggcctacatccaggagctgcgcaacaaaaggccggcggccacgaaaaaggccggccaggcaaaaaagaaaaagggatcctacccatacgatgttccagattacgcttatccctacgacgtgcctgattatgcatacccatatgatgtccccgactatgccggaagcgaggccagcggttccggacgggctgacgcattggacgattttgatctggatatgctgggaagtgacgccctcgatgattttgaccttgacatgcttggttcggatgcccttgatgactttgacctcgacatgctcggcagtgacgcccttgatgatttcgacctggacatgctgattaactctagaagttccggatctccgaaaaagaaacgcaaagttggtagccagtacctgcccgacaccgacgaccggcaccggatcgaggaaaagcggaagcggacctacgagacattcaagagcatcatgaagaagtcccccttcagcggccccaccgaccctagacctccacctagaagaatcgccgtgcccagcagatccagcgccagcgtgccaaaacctgccccccagccttaccccttcaccagcagcctgagcaccatcaactacgacgagttccctaccatggtgttccccagcggccagatctctcaggcctctgctctggctccagcccctcctcaggtgctgcctcaggctcctgctcctgcaccagctccagccatggtgtctgcactggctcaggcaccagcacccgtgcctgtgctggctcctggacctccacaggctgtggctccaccagcccctaaacctacacaggccggcgagggcacactgtctgaagctctgctgcagctgcagttcgacgacgaggatctgggagccctgctgggaaacagcaccgatcctgccgtgttcaccgacctggccagcgtggacaacagcgagttccagcagctgctgaaccagggcatccctgtggcccctcacaccaccgagcccatgctgatggaataccccgaggccatcacccggctcgtgacaggcgctcagaggcctcctgatccagctcctgcccctctgggagcaccaggcctgcctaatggactgctgtctggcgacgaggacttcagctctatcgccgatatggatttctcagccttgctgggctctggcagcggcagccgggattccagggaagggatgtttttgccgaagcctgaggccggctccgctattagtgacgtgtttgagggccgcgaggtgtgccagccaaaacgaatccggccatttcatcctccaggaagtccatgggccaaccgcccactccccgccagcctcgcaccaacaccaaccggtccagtacatgagccagtcgggtcactgaccccggcaccagtccctcagccactggatccagcgcccgcagtgactcccgaggccagtcacctgttggaggatcccgatgaagagacgagccaggctgtcaaagcccttcgggagatggccgatactgtgattccccagaaggaagaggctgcaatctgtggccaaatggacctttcccatccgcccccaaggggccatctggatgagctgacaaccacacttgagtccatgaccgaggatctgaacctggactcacccctgaccccggaattgaacgagattctggataccttcctgaacgacgagtgcctcttgcatgccatgcatatcagcacaggactgtccatcttcgacacatctctgttttaa

SEQ ID NO: 436 - DNA, 5574 bp, synthetic construct
  misc_feature 1..5574: note = Description of Artificial Sequence: Synthetic polynucleotide
  source 1..5574: mol_type = other DNA
atgacacagttcgagggctttaccaacctgtatcaggtgagcaagacactgcggtttgagctgatcccacagggcaagaccctgaagcacatccaggagcagggcttcatcgaggaggacaaggcccgcaatgatcactacaaggagctgaagcccatcatcgatcggatctacaagacctatgccgaccagtgcctgcagctggtgcagctggattgggagaacctgagcgccgccatcgactcctatagaaaggagaaaaccgaggagacaaggaacgccctgatcgaggagcaggccacatatcgcaatgccatccacgactacttcatcggccggacagacaacctgaccgatgccatcaataagagacacgccgagatctacaagggcctgttcaaggccgagctgtttaatggcaaggtgctgaagcagctgggcaccgtgaccacaaccgagcacgagaacgccctgctgcggagcttcgacaagtttacaacctacttctccggcttttatagaaacaggaagaacgtgttcagcgccgaggatatcagcacagccatcccacaccgcatcgtgcaggacaacttccccaagtttaaggagaattgtcacatcttcacacgcctgatcaccgccgtgcccagcctgcgggagcactttgagaacgtgaagaaggccatcggcatcttcgtgagcacctccatcgaggaggtgttttccttccctttttataaccagctgctgacacagacccagatcgacctgtataaccagctgctgggaggaatctctcgggaggcaggcaccgagaagatcaagggcctgaacgaggtgctgaatctggccatccagaagaatgatgagacagcccacatcatcgcctccctgccacacagattcatccccctgtttaagcagatcctgtccgataggaacaccctgtctttcatcctggaggagtttaagagcgacgaggaagtgatccagtccttctgcaagtacaagacactgctgagaaacgagaacgtgctggagacagccgaggccctgtttaacgagctgaacagcatcgacctgacacacatcttcatcagccacaagaagctggagacaatcagcagcgccctgtgcgaccactgggatacactgaggaatgccctgtatgagcggagaatctccgagctgacaggcaagatcaccaagtctgccaaggagaaggtgcagcgcagcctgaagcacgaggatatcaacctgcaggagatcatctctgccgcaggcaaggagctgagcgaggccttcaagcagaaaaccagcgagatcctgtcccacgcacacgccgccctggatcagccactgcctacaaccctgaagaagcaggaggagaaggagatcctgaagtctcagctggacagcctgctgggcctgtaccacctgctggactggtttgccgtggatgagtccaacgaggtggaccccgagttctctgcccggctgaccggcatcaagctggagatggagccttctctgagcttctacaacaaggccagaaattatgccaccaagaagccctactccgtggagaagttcaagctgaactttcagatgcctacactggccagaggctgggacgtgaatagagagaagaacaatggcgccatcctgtttgtgaagaacggcctgtactatctgggcatcatgccaaagcagaagggcaggtataaggccctgagcttcgagcccacagagaaaaccagcgagggctttgataagatgtactatgactacttccctgatgccgccaagatgatcccaaagtgcagcacccagctgaaggccgtgacagcccactttcagacccacacaacccccatcctgctgtccaacaatttcatcgagcctctggagatcacaaaggagatctacgacctgaacaatcctgagaaggagccaaagaagtttcagacagcctacgccaagaaaaccggcgaccagaagggctacagagaggccctgtgcaagtggatcgacttcacaagggattttctgtccaagtataccaagacaacctctatcgatctgtctagcctgcggccatcctctcagtataaggacctgggcgagtactatgccgagctgaatcccctgctgtaccacatcagcttccagagaatcgccgagaaggagatcatggatgccgtggagacaggcaagctgtacctgttccagatctataacaaggactttgccaagggccaccacggcaagcctaatctgcacacactgtattggaccggcctgttttctccagagaacctggccaagacaagcatcaagctgaatggccaggccgagctgttctaccgccctaagtccaggatgaagaggatggcacaccggctgggagagaagatgctgaacaagaagctgaaggatcagaaaaccccaatccccgacaccctgtaccaggagctgtacgactatgtgaatcacagactgtcccacgacctgtctgatgaggccagggccctgctgcccaacgtgatcaccaaggaggtgtctcacgagatcatcaaggataggcgctttaccagcgacaagttctttttccacgtgcctatcacactgaactatcaggccgccaattccccatctaagttcaaccagagggtgaatgcctacctgaaggagcaccccgagacacctatcatcggcatcgcccggggcgagagaaacctgatctatatcacagtgatcgactccaccggcaagatcctggagcagcggagcctgaacaccatccagcagtttgattaccagaagaagctggacaacagggagaaggagagggtggcagcaaggcaggcctggtctgtggtgggcacaatcaaggatctgaagcagggctatctgagccaggtcatccacgagatcgtggacctgatgatccactaccaggccgtggtggtgctggagaacctgaatttcggctttaagagcaagaggaccggcatcgccgagaaggccgtgtaccagcagttcgagaagatgctgatcgataagctgaattgcctggtgctgaaggactatccagcagagaaagtgggaggcgtgctgaacccataccagctgacagaccagttcacctcctttgccaagatgggcacccagtctggcttcctgttttacgtgcctgccccatatacatctaagatcgatcccctgaccggcttcgtggaccccttcgtgtggaaaaccatcaagaatcacgagagccgcaagcacttcctggagggcttcgactttctgcactacgacgtgaaaaccggcgacttcatcctgcactttaagatgaacagaaatctgtccttccagaggggcctgcccggctttatgcctgcatgggatatcgtgttcgagaagaacgagacacagtttgacgccaagggcacccctttcatcgccggcaagagaatcgtgccagtgatcgagaatcacagattcaccggcagataccgggacctgtatcctgccaacgagctgatcgccctgctggaggagaagggcatcgtgttcagggatggctccaacatcctgccaaagctgctggagaatgacgattctcacgccatcgacacgatggtggccctgatccgcagcgtgctgcagatgcggaactccaatgccgccacaggcgaggactatatcaacagccccgtgcgcgatctgaatggcgtgtgcttcgactcccggtttcagaacccagagtggccaatggacgccgatgccaatggcgcctaccacatcgccctgaagggccagctgctgctgaatcacctgaaggagagcaaggatctgaagctgcagaacggcatctccaatcaggactggctggcctacatccaggagctgcgcaacggtggaagcggagggagtcccaagaagaagaggaaagtcgggggttccggaggaagcgaggccagcggttccggacgggctgacgcattggacgattttgatctggatatgctgggaagtgacgccctcgatgattttgaccttgacatgcttggttcggatgcccttgatgactttgacctcgacatgctcggcagtgacgcccttgatgatttcgacctggacatgctgattaactctagaagttccggatctccgaaaaagaaacgcaaagttggtagccagtacctgcccgacaccgacgaccggcaccggatcgaggaaaagcggaagcggacctacgagacattcaagagcatcatgaagaagtcccccttcagcggccccaccgaccctagacctccacctagaagaatcgccgtgcccagcagatccagcgccagcgtgccaaaacctgccccccagccttaccccttcaccagcagcctgagcaccatcaactacgacgagttccctaccatggtgttccccagcggccagatctctcaggcctctgctctggctccagcccctcctcaggtgctgcctcaggctcctgctcctgcaccagctccagccatggtgtctgcactggctcaggcaccagcacccgtgcctgtgctggctcctggacctccacaggctgtggctccaccagcccctaaacctacacaggccggcgagggcacactgtctgaagctctgctgcagctgcagttcgacgacgaggatctgggagccctgctgggaaacagcaccgatcctgccgtgttcaccgacctggccagcgtggacaacagcgagttccagcagctgctgaaccagggcatccctgtggcccctcacaccaccgagcccatgctgatggaataccccgaggccatcacccggctcgtgacaggcgctcagaggcctcctgatccagctcctgcccctctgggagcaccaggcctgcctaatggactgctgtctggcgacgaggacttcagctctatcgccgatatggatttctcagccttgctgggctctggcagcggcagccgggattccagggaagggatgtttttgccgaagcctgaggccggctccgctattagtgacgtgtttgagggccgcgaggtgtgccagccaaaacgaatccggccatttcatcctccaggaagtccatgggccaaccgcccactccccgccagcctcgcaccaacaccaaccggtccagtacatgagccagtcgggtcactgaccccggcaccagtccctcagccactggatccagcgcccgcagtgactcccgaggccagtcacctgttggaggatcccgatgaagagacgagccaggctgtcaaagcccttcgggagatggccgatactgtgattccccagaaggaagaggctgcaatctgtggccaaatggacctttcccatccgcccccaaggggccatctggatgagctgacaaccacacttgagtccatgaccgaggatctgaacctggactcacccctgaccccggaattgaacgagattctggataccttcctgaacgacgagtgcctcttgcatgccatgcatatcagcacaggactgtccatcttcgacacatctctgttttaa

SEQ ID NO: 437 - DNA, 5637 bp, synthetic construct
  misc_feature 1..5637: note = Description of Artificial Sequence: Synthetic polynucleotide
  source 1..5637: mol_type = other DNA
atgggcccaaagaaaaagaggaaagtcggcagtggacctaaaaagaaacgaaaggttgggtcaggtacacagttcgagggctttaccaacctgtatcaggtgagcaagacactgcggtttgagctgatcccacagggcaagaccctgaagcacatccaggagcagggcttcatcgaggaggacaaggcccgcaatgatcactacaaggagctgaagcccatcatcgatcggatctacaagacctatgccgaccagtgcctgcagctggtgcagctggattgggagaacctgagcgccgccatcgactcctatagaaaggagaaaaccgaggagacaaggaacgccctgatcgaggagcaggccacatatcgcaatgccatccacgactacttcatcggccggacagacaacctgaccgatgccatcaataagagacacgccgagatctacaagggcctgttcaaggccgagctgtttaatggcaaggtgctgaagcagctgggcaccgtgaccacaaccgagcacgagaacgccctgctgcggagcttcgacaagtttacaacctacttctccggcttttatagaaacaggaagaacgtgttcagcgccgaggatatcagcacagccatcccacaccgcatcgtgcaggacaacttccccaagtttaaggagaattgtcacatcttcacacgcctgatcaccgccgtgcccagcctgcgggagcactttgagaacgtgaagaaggccatcggcatcttcgtgagcacctccatcgaggaggtgttttccttccctttttataaccagctgctgacacagacccagatcgacctgtataaccagctgctgggaggaatctctcgggaggcaggcaccgagaagatcaagggcctgaacgaggtgctgaatctggccatccagaagaatgatgagacagcccacatcatcgcctccctgccacacagattcatccccctgtttaagcagatcctgtccgataggaacaccctgtctttcatcctggaggagtttaagagcgacgaggaagtgatccagtccttctgcaagtacaagacactgctgagaaacgagaacgtgctggagacagccgaggccctgtttaacgagctgaacagcatcgacctgacacacatcttcatcagccacaagaagctggagacaatcagcagcgccctgtgcgaccactgggatacactgaggaatgccctgtatgagcggagaatctccgagctgacaggcaagatcaccaagtctgccaaggagaaggtgcagcgcagcctgaagcacgaggatatcaacctgcaggagatcatctctgccgcaggcaaggagctgagcgaggccttcaagcagaaaaccagcgagatcctgtcccacgcacacgccgccctggatcagccactgcctacaaccctgaagaagcaggaggagaaggagatcctgaagtctcagctggacagcctgctgggcctgtaccacctgctggactggtttgccgtggatgagtccaacgaggtggaccccgagttctctgcccggctgaccggcatcaagctggagatggagccttctctgagcttctacaacaaggccagaaattatgccaccaagaagccctactccgtggagaagttcaagctgaactttcagatgcctacactggccagaggctgggacgtgaatagagagaagaacaatggcgccatcctgtttgtgaagaacggcctgtactatctgggcatcatgccaaagcagaagggcaggtataaggccctgagcttcgagcccacagagaaaaccagcgagggctttgataagatgtactatgactacttccctgatgccgccaagatgatcccaaagtgcagcacccagctgaaggccgtgacagcccactttcagacccacacaacccccatcctgctgtccaacaatttcatcgagcctctggagatcacaaaggagatctacgacctgaacaatcctgagaaggagccaaagaagtttcagacagcctacgccaagaaaaccggcgaccagaagggctacagagaggccctgtgcaagtggatcgacttcacaagggattttctgtccaagtataccaagacaacctctatcgatctgtctagcctgcggccatcctctcagtataaggacctgggcgagtactatgccgagctgaatcccctgctgtaccacatcagcttccagagaatcgccgagaaggagatcatggatgccgtggagacaggcaagctgtacctgttccagatctataacaaggactttgccaagggccaccacggcaagcctaatctgcacacactgtattggaccggcctgttttctccagagaacctggccaagacaagcatcaagctgaatggccaggccgagctgttctaccgccctaagtccaggatgaagaggatggcacaccggctgggagagaagatgctgaacaagaagctgaaggatcagaaaaccccaatccccgacaccctgtaccaggagctgtacgactatgtgaatcacagactgtcccacgacctgtctgatgaggccagggccctgctgcccaacgtgatcaccaaggaggtgtctcacgagatcatcaaggataggcgctttaccagcgacaagttctttttccacgtgcctatcacactgaactatcaggccgccaattccccatctaagttcaaccagagggtgaatgcctacctgaaggagcaccccgagacacctatcatcggcatcgcccggggcgagagaaacctgatctatatcacagtgatcgactccaccggcaagatcctggagcagcggagcctgaacaccatccagcagtttgattaccagaagaagctggacaacagggagaaggagagggtggcagcaaggcaggcctggtctgtggtgggcacaatcaaggatctgaagcagggctatctgagccaggtcatccacgagatcgtggacctgatgatccactaccaggccgtggtggtgctggagaacctgaatttcggctttaagagcaagaggaccggcatcgccgagaaggccgtgtaccagcagttcgagaagatgctgatcgataagctgaattgcctggtgctgaaggactatccagcagagaaagtgggaggcgtgctgaacccataccagctgacagaccagttcacctcctttgccaagatgggcacccagtctggcttcctgttttacgtgcctgccccatatacatctaagatcgatcccctgaccggcttcgtggaccccttcgtgtggaaaaccatcaagaatcacgagagccgcaagcacttcctggagggcttcgactttctgcactacgacgtgaaaaccggcgacttcatcctgcactttaagatgaacagaaatctgtccttccagaggggcctgcccggctttatgcctgcatgggatatcgtgttcgagaagaacgagacacagtttgacgccaagggcacccctttcatcgccggcaagagaatcgtgccagtgatcgagaatcacagattcaccggcagataccgggacctgtatcctgccaacgagctgatcgccctgctggaggagaagggcatcgtgttcagggatggctccaacatcctgccaaagctgctggagaatgacgattctcacgccatcgacacgatggtggccctgatccgcagcgtgctgcagatgcggaactccaatgccgccacaggcgaggactatatcaacagccccgtgcgcgatctgaatggcgtgtgcttcgactcccggtttcagaacccagagtggccaatggacgccgatgccaatggcgcctaccacatcgccctgaagggccagctgctgctgaatcacctgaaggagagcaaggatctgaagctgcagaacggcatctccaatcaggactggctggcctacatccaggagctgcgcaacggtggaagcggagggagtcccaagaagaagaggaaagtcgggggttccggaggaagcgaggccagcggttccggacgggctgacgcattggacgattttgatctggatatgctgggaagtgacgccctcgatgattttgaccttgacatgcttggttcggatgcccttgatgactttgacctcgacatgctcggcagtgacgcccttgatgatttcgacctggacatgctgattaactctagaagttccggatctccgaaaaagaaacgcaaagttggtagccagtacctgcccgacaccgacgaccggcaccggatcgaggaaaagcggaagcggacctacgagacattcaagagcatcatgaagaagtcccccttcagcggccccaccgaccctagacctccacctagaagaatcgccgtgcccagcagatccagcgccagcgtgccaaaacctgccccccagccttaccccttcaccagcagcctgagcaccatcaactacgacgagttccctaccatggtgttccccagcggccagatctctcaggcctctgctctggctccagcccctcctcaggtgctgcctcaggctcctgctcctgcaccagctccagccatggtgtctgcactggctcaggcaccagcacccgtgcctgtgctggctcctggacctccacaggctgtggctccaccagcccctaaacctacacaggccggcgagggcacactgtctgaagctctgctgcagctgcagttcgacgacgaggatctgggagccctgctgggaaacagcaccgatcctgccgtgttcaccgacctggccagcgtggacaacagcgagttccagcagctgctgaaccagggcatccctgtggcccctcacaccaccgagcccatgctgatggaataccccgaggccatcacccggctcgtgacaggcgctcagaggcctcctgatccagctcctgcccctctgggagcaccaggcctgcctaatggactgctgtctggcgacgaggacttcagctctatcgccgatatggatttctcagccttgctgggctctggcagcggcagccgggattccagggaagggatgtttttgccgaagcctgaggccggctccgctattagtgacgtgtttgagggccgcgaggtgtgccagccaaaacgaatccggccatttcatcctccaggaagtccatgggccaaccgcccactccccgccagcctcgcaccaacaccaaccggtccagtacatgagccagtcgggtcactgaccccggcaccagtccctcagccactggatccagcgcccgcagtgactcccgaggccagtcacctgttggaggatcccgatgaagagacgagccaggctgtcaaagcccttcgggagatggccgatactgtgattccccagaaggaagaggctgcaatctgtggccaaatggacctttcccatccgcccccaaggggccatctggatgagctgacaaccacacttgagtccatgaccgaggatctgaacctggactcacccctgaccccggaattgaacgagattctggataccttcctgaacgacgagtgcctcttgcatgccatgcatatcagcacaggactgtccatcttcgacacatctctgttttaa

SEQ ID NO: 438 - DNA, 5073 bp, synthetic construct
  misc_feature 1..5073: note = Description of Artificial Sequence: Synthetic polynucleotide
  source 1..5073: mol_type = other DNA
atgggcagctcagagactggcccagtggctgtggaccccacattgagacggcggatcgagccccatgagtttgaggtattcttcgatccgagagagctccgcaaggagacctgcctgctttacgaaattaattgggggggccggcactccatttggcgacatacatcacagaacactaacaagcacgtcgaagtcaacttcatcgagaagttcacgacagaaagatatttctgtccgaacacaaggtgcagcattacctggtttctcagctggagcccatgcggcgaatgtagtagggccatcactgaattcctgtcaaggtatccccacgtcactctgtttatttacatcgcaaggctgtaccaccacgctgacccccgcaatcgacaaggcctgcgggatttgatctcttcaggtgtgactatccaaattatgactgagcaggagtcaggatactgctggagaaactttgtgaattatagcccgagtaatgaagcccactggcctaggtatccccatctgtgggtacgactgtacgttcttgaactgtactgcatcatactgggcctgcctccttgtctcaacattctgagaaggaagcagccacagctgacattctttaccatcgctcttcagtcttgtcattaccagcgactgcccccacacattctctgggccaccgggttgaaatctggtggttcttctggtggttctagcggcagcgagactcccgggacctcagagtccgccacacccgaaagttccggagggagtagcggcgggtctacacagttcgagggctttaccaacctgtatcaggtgagcaagacactgcggtttgagctgatcccacagggcaagaccctgaagcacatccaggagcagggcttcatcgaggaggacaaggcccgcaatgatcactacaaggagctgaagcccatcatcgatcggatctacaagacctatgccgaccagtgcctgcagctggtgcagctggattgggagaacctgagcgccgccatcgactcctatagaaaggagaaaaccgaggagacaaggaacgccctgatcgaggagcaggccacatatcgcaatgccatccacgactacttcatcggccggacagacaacctgaccgatgccatcaataagagacacgccgagatctacaagggcctgttcaaggccgagctgtttaatggcaaggtgctgaagcagctgggcaccgtgaccacaaccgagcacgagaacgccctgctgcggagcttcgacaagtttacaacctacttctccggcttttatgagaacaggaagaacgtgttcagcgccgaggatatcagcacagccatcccacaccgcatcgtgcaggacaacttccccaagtttaaggagaattgtcacatcttcacacgcctgatcaccgccgtgcccagcctgcgggagcactttgagaacgtgaagaaggccatcggcatcttcgtgagcacctccatcgaggaggtgttttccttccctttttataaccagctgctgacacagacccagatcgacctgtataaccagctgctgggaggaatctctcgggaggcaggcaccgagaagatcaagggcctgaacgaggtgctgaatctggccatccagaagaatgatgagacagcccacatcatcgcctccctgccacacagattcatccccctgtttaagcagatcctgtccgataggaacaccctgtctttcatcctggaggagtttaagagcgacgaggaagtgatccagtccttctgcaagtacaagacactgctgagaaacgagaacgtgctggagacagccgaggccctgtttaacgagctgaacagcatcgacctgacacacatcttcatcagccacaagaagctggagacaatcagcagcgccctgtgcgaccactgggatacactgaggaatgccctgtatgagcggagaatctccgagctgacaggcaagatcaccaagtctgccaaggagaaggtgcagcgcagcctgaagcacgaggatatcaacctgcaggagatcatctctgccgcaggcaaggagctgagcgaggccttcaagcagaaaaccagcgagatcctgtcccacgcacacgccgccctggatcagccactgcctacaaccctgaagaagcaggaggagaaggagatcctgaagtctcagctggacagcctgctgggcctgtaccacctgctggactggtttgccgtggatgagtccaacgaggtggaccccgagttctctgcccggctgaccggcatcaagctggagatggagccttctctgagcttctacaacaaggccagaaattatgccaccaagaagccctactccgtggagaagttcaagctgaactttcagatgcctacactggcctctggctgggacgtgaataaggagaagaacaatggcgccatcctgtttgtgaagaacggcctgtactatctgggcatcatgccaaagcagaagggcaggtataaggccctgagcttcgagcccacagagaaaaccagcgagggctttgataagatgtactatgactacttccctgatgccgccaagatgatcccaaagtgcagcacccagctgaaggccgtgacagcccactttcagacccacacaacccccatcctgctgtccaacaatttcatcgagcctctggagatcacaaaggagatctacgacctgaacaatcctgagaaggagccaaagaagtttcagacagcctacgccaagaaaaccggcgaccagaagggctacagagaggccctgtgcaagtggatcgacttcacaagggattttctgtccaagtataccaagacaacctctatcgatctgtctagcctgcggccatcctctcagtataaggacctgggcgagtactatgccgagctgaatcccctgctgtaccacatcagcttccagagaatcgccgagaaggagatcatggatgccgtggagacaggcaagctgtacctgttccagatctataacaaggactttgccaagggccaccacggcaagcctaatctgcacacactgtattggaccggcctgttttctccagagaacctggccaagacaagcatcaagctgaatggccaggccgagctgttctaccgccctaagtccaggatgaagaggatggcacaccggctgggagagaagatgctgaacaagaagctgaaggatcagaaaaccccaatccccgacaccctgtaccaggagctgtacgactatgtgaatcacagactgtcccacgacctgtctgatgaggccagggccctgctgcccaacgtgatcaccaaggaggtgtctcacgagatcatcaaggataggcgctttaccagcgacaagttctttttccacgtgcctatcacactgaactatcaggccgccaattccccatctaagttcaaccagagggtgaatgcctacctgaaggagcaccccgagacacctatcatcggcatcgcccggggcgagagaaacctgatctatatcacagtgatcgactccaccggcaagatcctggagcagcggagcctgaacaccatccagcagtttgattaccagaagaagctggacaacagggagaaggagagggtggcagcaaggcaggcctggtctgtggtgggcacaatcaaggatctgaagcagggctatctgagccaggtcatccacgagatcgtggacctgatgatccactaccaggccgtggtggtgctggagaacctgaatttcggctttaagagcaagaggaccggcatcgccgagaaggccgtgtaccagcagttcgagaagatgctgatcgataagctgaattgcctggtgctgaaggactatccagcagagaaagtgggaggcgtgctgaacccataccagctgacagaccagttcacctcctttgccaagatgggcacccagtctggcttcctgttttacgtgcctgccccatatacatctaagatcgatcccctgaccggcttcgtggaccccttcgtgtggaaaaccatcaagaatcacgagagccgcaagcacttcctggagggcttcgactttctgcactacgacgtgaaaaccggcgacttcatcctgcactttaagatgaacagaaatctgtccttccagaggggcctgcccggctttatgcctgcatgggatatcgtgttcgagaagaacgagacacagtttgacgccaagggcacccctttcatcgccggcaagagaatcgtgccagtgatcgagaatcacagattcaccggcagataccgggacctgtatcctgccaacgagctgatcgccctgctggaggagaagggcatcgtgttcagggatggctccaacatcctgccaaagctgctggagaatgacgattctcacgccatcgacacgatggtggccctgatccgcagcgtgctgcagatgcggaactccaatgccgccacaggcgaggactatatcaacagccccgtgcgcgatctgaatggcgtgtgcttcgactcccggtttcagaacccagagtggccaatggacgccgatgccaatggcgcctaccacatcgccctgaagggccagctgctgctgaatcacctgaaggagagcaaggatctgaagctgcagaacggcatctccaatcaggactggctggcctacatccaggagctgcgcaacaaaaggccggcggccacgaaaaaggccggccaggcaaaaaagaaaaagggatcctctggtggttctggaggatctggtggttctactaatctgtcagatattattgaaaaggagaccggtaagcaactggttatccaggaatccatcctcatgctcccagaggaggtggaagaagtcattgggaacaagccggaaagcgatatactcgtgcacaccgcctacgacgagagcaccgacgagaatgtcatgcttctgactagcgacgcccctgaatacaagccttgggctctggtcatacaggatagcaacggtgagaacaagattaagatgctctctggtggttctcccaagaagaagaggaaagtctaa

SEQ ID NO: 439 - DNA, 4836 bp, synthetic construct
  misc_feature 1..4836: note = Description of Artificial Sequence: Synthetic polynucleotide
  source 1..4836: mol_type = other DNA
atgggcagctcagagactggcccagtggctgtggaccccacattgagacggcggatcgagccccatgagtttgaggtattcttcgatccgagagagctccgcaaggagacctgcctgctttacgaaattaattgggggggccggcactccatttggcgacatacatcacagaacactaacaagcacgtcgaagtcaacttcatcgagaagttcacgacagaaagatatttctgtccgaacacaaggtgcagcattacctggtttctcagctggagcccatgcggcgaatgtagtagggccatcactgaattcctgtcaaggtatccccacgtcactctgtttatttacatcgcaaggctgtaccaccacgctgacccccgcaatcgacaaggcctgcgggatttgatctcttcaggtgtgactatccaaattatgactgagcaggagtcaggatactgctggagaaactttgtgaattatagcccgagtaatgaagcccactggcctaggtatccccatctgtgggtacgactgtacgttcttgaactgtactgcatcatactgggcctgcctccttgtctcaacattctgagaaggaagcagccacagctgacattctttaccatcgctcttcagtcttgtcattaccagcgactgcccccacacattctctgggccaccgggttgaaatctggtggttcttctggtggttctagcggcagcgagactcccgggacctcagagtccgccacacccgaaagttccggagggagtagcggcgggtctagcaagctggagaagtttacaaactgctactccctgtctaagaccctgaggttcaaggccatccctgtgggcaagacccaggagaacatcgacaataagcggctgctggtggaggacgagaagagagccgaggattataagggcgtgaagaagctgctggatcgctactatctgtcttttatcaacgacgtgctgcacagcatcaagctgaagaatctgaacaattacatcagcctgttccggaagaaaaccagaaccgagaaggagaataaggagctggagaacctggagatcaatctgcggaaggagatcgccaaggccttcaagggcaacgagggctacaagtccctgtttaagaaggatatcatcgagacaatcctgccagagttcctggacgataaggacgagatcgccctggtgaacagcttcaatggctttaccacagccttcaccggcttctttgataacagagagaatatgttttccgaggaggccaagagcacatccatcgccttcaggtgtatcaacgagaatctgacccgctacatctctaatatggacatcttcgagaaggtggacgccatctttgataagcacgaggtgcaggagatcaaggagaagatcctgaacagcgactatgatgtggaggatttctttgagggcgagttctttaactttgtgctgacacaggagggcatcgacgtgtataacgccatcatcggcggcttcgtgaccgagagcggcgagaagatcaagggcctgaacgagtacatcaacctgtataatcagaaaaccaagcagaagctgcctaagtttaagccactgtataagcaggtgctgagcgatcgggagtctctgagcttctacggcgagggctatacatccgatgaggaggtgctggaggtgtttagaaacaccctgaacaagaacagcgagatcttcagctccatcaagaagctggagaagctgttcaagaattttgacgagtactctagcgccggcatctttgtgaagaacggccccgccatcagcacaatctccaaggatatcttcggcgagtggaacgtgatccgggacaagtggaatgccgagtatgacgatatccacctgaagaagaaggccgtggtgaccgagaagtacgaggacgatcggagaaagtccttcaagaagatcggctccttttctctggagcagctgcaggagtacgccgacgccgatctgtctgtggtggagaagctgaaggagatcatcatccagaaggtggatgagatctacaaggtgtatggctcctctgagaagctgttcgacgccgattttgtgctggagaagagcctgaagaagaacgacgccgtggtggccatcatgaaggacctgctggattctgtgaagagcttcgagaattacatcaaggccttctttggcgagggcaaggagacaaacagggacgagtccttctatggcgattttgtgctggcctacgacatcctgctgaaggtggaccacatctacgatgccatccgcaattatgtgacccagaagccctactctaaggataagttcaagctgtattttcagaaccctcagttcatgggcggctgggacaaggataaggagacagactatcgggccaccatcctgagatacggctccaagtactatctggccatcatggataagaagtacgccaagtgcctgcagaagatcgacaaggacgatgtgaacggcaattacgagaagatcaactataagctgctgcccggccctaataagatgctgccaaaggtgttcttttctaagaagtggatggcctactataaccccagcgaggacatccagaagatctacaagaatggcacattcaagaagggcgatatgtttaacctgaatgactgtcacaagctgatcgacttctttaaggatagcatctcccggtatccaaagtggtccaatgcctacgatttcaacttttctgagacagagaagtataaggacatcgccggcttttacagagaggtggaggagcagggctataaggtgagcttcgagtctgccagcaagaaggaggtggataagctggtggaggagggcaagctgtatatgttccagatctataacaaggacttttccgataagtctcacggcacacccaatctgcacaccatgtacttcaagctgctgtttgacgagaacaatcacggacagatcaggctgagcggaggagcagagctgttcatgaggcgcgcctccctgaagaaggaggagctggtggtgcacccagccaactcccctatcgccaacaagaatccagataatcccaagaaaaccacaaccctgtcctacgacgtgtataaggataagaggttttctgaggaccagtacgagctgcacatcccaatcgccatcaataagtgccccaagaacatcttcaagatcaatacagaggtgcgcgtgctgctgaagcacgacgataacccctatgtgatcggcatcgccaggggcgagcgcaatctgctgtatatcgtggtggtggacggcaagggcaacatcgtggagcagtattccctgaacgagatcatcaacaacttcaacggcatcaggatcaagacagattaccactctctgctggacaagaaggagaaggagaggttcgaggcccgccagaactggacctccatcgagaatatcaaggagctgaaggccggctatatctctcaggtggtgcacaagatctgcgagctggtggagaagtacgatgccgtgatcgccctggaggacctgaactctggctttaagaatagccgcgtgaaggtggagaagcaggtgtatcagaagttcgagaagatgctgatcgataagctgaactacatggtggacaagaagtctaatccttgtgcaacaggcggcgccctgaagggctatcagatcaccaataagttcgagagctttaagtccatgtctacccagaacggcttcatcttttacatccctgcctggctgacatccaagatcgatccatctaccggctttgtgaacctgctgaaaaccaagtataccagcatcgccgattccaagaagttcatcagctcctttgacaggatcatgtacgtgcccgaggaggatctgttcgagtttgccctggactataagaacttctctcgcacagacgccgattacatcaagaagtggaagctgtactcctacggcaaccggatcagaatcttccggaatcctaagaagaacaacgtgttcgactgggaggaggtgtgcctgaccagcgcctataaggagctgttcaacaagtacggcatcaattatcagcagggcgatatcagagccctgctgtgcgagcagtccgacaaggccttctactctagctttatggccctgatgagcctgatgctgcagatgcggaacagcatcacaggccgcaccgacgtggattttctgatcagccctgtgaagaactccgacggcatcttctacgatagccggaactatgaggcccaggagaatgccatcctgccaaagaacgccgacgccaatggcgcctataacatcgccagaaaggtgctgtgggccatcggccagttcaagaaggccgaggacgagaagctggataaggtgaagatcgccatctctaacaaggagtggctggagtacgcccagaccagcgtgaagcacaaaaggccggcggccacgaaaaaggccggccaggcaaaaaagaaaaagggatcctctggtggttctggaggatctggtggttctactaatctgtcagatattattgaaaaggagaccggtaagcaactggttatccaggaatccatcctcatgctcccagaggaggtggaagaagtcattgggaacaagccggaaagcgatatactcgtgcacaccgcctacgacgagagcaccgacgagaatgtcatgcttctgactagcgacgcccctgaatacaagccttgggctctggtcatacaggatagcaacggtgagaacaagattaagatgctctctggtggttctcccaagaagaagaggaaagtctaa

SEQ ID NO: 440 - DNA, 5073 bp, synthetic construct
  misc_feature 1..5073: note = Description of Artificial Sequence: Synthetic polynucleotide
  source 1..5073: mol_type = other DNA
atgggcagctcagagactggcccagtggctgtggaccccacattgagacggcggatcgagccccatgagtttgaggtattcttcgatccgagagagctccgcaaggagacctgcctgctttacgaaattaattgggggggccggcactccatttggcgacatacatcacagaacactaacaagcacgtcgaagtcaacttcatcgagaagttcacgacagaaagatatttctgtccgaacacaaggtgcagcattacctggtttctcagctggagcccatgcggcgaatgtagtagggccatcactgaattcctgtcaaggtatccccacgtcactctgtttatttacatcgcaaggctgtaccaccacgctgacccccgcaatcgacaaggcctgcgggatttgatctcttcaggtgtgactatccaaattatgactgagcaggagtcaggatactgctggagaaactttgtgaattatagcccgagtaatgaagcccactggcctaggtatccccatctgtgggtacgactgtacgttcttgaactgtactgcatcatactgggcctgcctccttgtctcaacattctgagaaggaagcagccacagctgacattctttaccatcgctcttcagtcttgtcattaccagcgactgcccccacacattctctgggccaccgggttgaaatctggtggttcttctggtggttctagcggcagcgagactcccgggacctcagagtccgccacacccgaaagttccggagggagtagcggcgggtctacacagttcgagggctttaccaacctgtatcaggtgagcaagacactgcggtttgagctgatcccacagggcaagaccctgaagcacatccaggagcagggcttcatcgaggaggacaaggcccgcaatgatcactacaaggagctgaagcccatcatcgatcggatctacaagacctatgccgaccagtgcctgcagctggtgcagctggattgggagaacctgagcgccgccatcgactcctatagaaaggagaaaaccgaggagacaaggaacgccctgatcgaggagcaggccacatatcgcaatgccatccacgactacttcatcggccggacagacaacctgaccgatgccatcaataagagacacgccgagatctacaagggcctgttcaaggccgagctgtttaatggcaaggtgctgaagcagctgggcaccgtgaccacaaccgagcacgagaacgccctgctgcggagcttcgacaagtttacaacctacttctccggcttttatagaaacaggaagaacgtgttcagcgccgaggatatcagcacagccatcccacaccgcatcgtgcaggacaacttccccaagtttaaggagaattgtcacatcttcacacgcctgatcaccgccgtgcccagcctgcgggagcactttgagaacgtgaagaaggccatcggcatcttcgtgagcacctccatcgaggaggtgttttccttccctttttataaccagctgctgacacagacccagatcgacctgtataaccagctgctgggaggaatctctcgggaggcaggcaccgagaagatcaagggcctgaacgaggtgctgaatctggccatccagaagaatgatgagacagcccacatcatcgcctccctgccacacagattcatccccctgtttaagcagatcctgtccgataggaacaccctgtctttcatcctggaggagtttaagagcgacgaggaagtgatccagtccttctgcaagtacaagacactgctgagaaacgagaacgtgctggagacagccgaggccctgtttaacgagctgaacagcatcgacctgacacacatcttcatcagccacaagaagctggagacaatcagcagcgccctgtgcgaccactgggatacactgaggaatgccctgtatgagcggagaatctccgagctgacaggcaagatcaccaagtctgccaaggagaaggtgcagcgcagcctgaagcacgaggatatcaacctgcaggagatcatctctgccgcaggcaaggagctgagcgaggccttcaagcagaaaaccagcgagatcctgtcccacgcacacgccgccctggatcagccactgcctacaaccctgaagaagcaggaggagaaggagatcctgaagtctcagctggacagcctgctgggcctgtaccacctgctggactggtttgccgtggatgagtccaacgaggtggaccccgagttctctgcccggctgaccggcatcaagctggagatggagccttctctgagcttctacaacaaggccagaaattatgccaccaagaagccctactccgtggagaagttcaagctgaactttcagatgcctacactggccagaggctgggacgtgaatagagagaagaacaatggcgccatcctgtttgtgaagaacggcctgtactatctgggcatcatgccaaagcagaagggcaggtataaggccctgagcttcgagcccacagagaaaaccagcgagggctttgataagatgtactatgactacttccctgatgccgccaagatgatcccaaagtgcagcacccagctgaaggccgtgacagcccactttcagacccacacaacccccatcctgctgtccaacaatttcatcgagcctctggagatcacaaaggagatctacgacctgaacaatcctgagaaggagccaaagaagtttcagacagcctacgccaagaaaaccggcgaccagaagggctacagagaggccctgtgcaagtggatcgacttcacaagggattttctgtccaagtataccaagacaacctctatcgatctgtctagcctgcggccatcctctcagtataaggacctgggcgagtactatgccgagctgaatcccctgctgtaccacatcagcttccagagaatcgccgagaaggagatcatggatgccgtggagacaggcaagctgtacctgttccagatctataacaaggactttgccaagggccaccacggcaagcctaatctgcacacactgtattggaccggcctgttttctccagagaacctggccaagacaagcatcaagctgaatggccaggccgagctgttctaccgccctaagtccaggatgaagaggatggcacaccggctgggagagaagatgctgaacaagaagctgaaggatcagaaaaccccaatccccgacaccctgtaccaggagctgtacgactatgtgaatcacagactgtcccacgacctgtctgatgaggccagggccctgctgcccaacgtgatcaccaaggaggtgtctcacgagatcatcaaggataggcgctttaccagcgacaagttctttttccacgtgcctatcacactgaactatcaggccgccaattccccatctaagttcaaccagagggtgaatgcctacctgaaggagcaccccgagacacctatcatcggcatcgcccggggcgagagaaacctgatctatatcacagtgatcgactccaccggcaagatcctggagcagcggagcctgaacaccatccagcagtttgattaccagaagaagctggacaacagggagaaggagagggtggcagcaaggcaggcctggtctgtggtgggcacaatcaaggatctgaagcagggctatctgagccaggtcatccacgagatcgtggacctgatgatccactaccaggccgtggtggtgctggagaacctgaatttcggctttaagagcaagaggaccggcatcgccgagaaggccgtgtaccagcagttcgagaagatgctgatcgataagctgaattgcctggtgctgaaggactatccagcagagaaagtgggaggcgtgctgaacccataccagctgacagaccagttcacctcctttgccaagatgggcacccagtctggcttcctgttttacgtgcctgccccatatacatctaagatcgatcccctgaccggcttcgtggaccccttcgtgtggaaaaccatcaagaatcacgagagccgcaagcacttcctggagggcttcgactttctgcactacgacgtgaaaaccggcgacttcatcctgcactttaagatgaacagaaatctgtccttccagaggggcctgcccggctttatgcctgcatgggatatcgtgttcgagaagaacgagacacagtttgacgccaagggcacccctttcatcgccggcaagagaatcgtgccagtgatcgagaatcacagattcaccggcagataccgggacctgtatcctgccaacgagctgatcgccctgctggaggagaagggcatcgtgttcagggatggctccaacatcctgccaaagctgctggagaatgacgattctcacgccatcgacacgatggtggccctgatccgcagcgtgctgcagatgcggaactccaatgccgccacaggcgaggactatatcaacagccccgtgcgcgatctgaatggcgtgtgcttcgactcccggtttcagaacccagagtggccaatggacgccgatgccaatggcgcctaccacatcgccctgaagggccagctgctgctgaatcacctgaaggagagcaaggatctgaagctgcagaacggcatctccaatcaggactggctggcctacatccaggagctgcgcaacaaaaggccggcggccacgaaaaaggccggccaggcaaaaaagaaaaagggatcctctggtggttctggaggatctggtggttctactaatctgtcagatattattgaaaaggagaccggtaagcaactggttatccaggaatccatcctcatgctcccagaggaggtggaagaagtcattgggaacaagccggaaagcgatatactcgtgcacaccgcctacgacgagagcaccgacgagaatgtcatgcttctgactagcgacgcccctgaatacaagccttgggctctggtcatacaggatagcaacggtgagaacaagattaagatgctctctggtggttctcccaagaagaagaggaaagtctaa

SEQ ID NO: 441 - DNA, 5133 bp, synthetic construct
  misc_feature 1..5133: note = Description of Artificial Sequence: Synthetic polynucleotide
  source 1..5133: mol_type = other DNA
atgggcccaaagaaaaagaggaaagtcggcagtggacctaaaaagaaacgaaaggttgggtcaggtagctcagagactggcccagtggctgtggaccccacattgagacggcggatcgagccccatgagtttgaggtattcttcgatccgagagagctccgcaaggagacctgcctgctttacgaaattaattgggggggccggcactccatttggcgacatacatcacagaacactaacaagcacgtcgaagtcaacttcatcgagaagttcacgacagaaagatatttctgtccgaacacaaggtgcagcattacctggtttctcagctggagcccatgcggcgaatgtagtagggccatcactgaattcctgtcaaggtatccccacgtcactctgtttatttacatcgcaaggctgtaccaccacgctgacccccgcaatcgacaaggcctgcgggatttgatctcttcaggtgtgactatccaaattatgactgagcaggagtcaggatactgctggagaaactttgtgaattatagcccgagtaatgaagcccactggcctaggtatccccatctgtgggtacgactgtacgttcttgaactgtactgcatcatactgggcctgcctccttgtctcaacattctgagaaggaagcagccacagctgacattctttaccatcgctcttcagtcttgtcattaccagcgactgcccccacacattctctgggccaccgggttgaaatctggtggttcttctggtggttctagcggcagcgagactcccgggacctcagagtccgccacacccgaaagttccggagggagtagcggcgggtctacacagttcgagggctttaccaacctgtatcaggtgagcaagacactgcggtttgagctgatcccacagggcaagaccctgaagcacatccaggagcagggcttcatcgaggaggacaaggcccgcaatgatcactacaaggagctgaagcccatcatcgatcggatctacaagacctatgccgaccagtgcctgcagctggtgcagctggattgggagaacctgagcgccgccatcgactcctatagaaaggagaaaaccgaggagacaaggaacgccctgatcgaggagcaggccacatatcgcaatgccatccacgactacttcatcggccggacagacaacctgaccgatgccatcaataagagacacgccgagatctacaagggcctgttcaaggccgagctgtttaatggcaaggtgctgaagcagctgggcaccgtgaccacaaccgagcacgagaacgccctgctgcggagcttcgacaagtttacaacctacttctccggcttttatagaaacaggaagaacgtgttcagcgccgaggatatcagcacagccatcccacaccgcatcgtgcaggacaacttccccaagtttaaggagaattgtcacatcttcacacgcctgatcaccgccgtgcccagcctgcgggagcactttgagaacgtgaagaaggccatcggcatcttcgtgagcacctccatcgaggaggtgttttccttccctttttataaccagctgctgacacagacccagatcgacctgtataaccagctgctgggaggaatctctcgggaggcaggcaccgagaagatcaagggcctgaacgaggtgctgaatctggccatccagaagaatgatgagacagcccacatcatcgcctccctgccacacagattcatccccctgtttaagcagatcctgtccgataggaacaccctgtctttcatcctggaggagtttaagagcgacgaggaagtgatccagtccttctgcaagtacaagacactgctgagaaacgagaacgtgctggagacagccgaggccctgtttaacgagctgaacagcatcgacctgacacacatcttcatcagccacaagaagctggagacaatcagcagcgccctgtgcgaccactgggatacactgaggaatgccctgtatgagcggagaatctccgagctgacaggcaagatcaccaagtctgccaaggagaaggtgcagcgcagcctgaagcacgaggatatcaacctgcaggagatcatctctgccgcaggcaaggagctgagcgaggccttcaagcagaaaaccagcgagatcctgtcccacgcacacgccgccctggatcagccactgcctacaaccctgaagaagcaggaggagaaggagatcctgaagtctcagctggacagcctgctgggcctgtaccacctgctggactggtttgccgtggatgagtccaacgaggtggaccccgagttctctgcccggctgaccggcatcaagctggagatggagccttctctgagcttctacaacaaggccagaaattatgccaccaagaagccctactccgtggagaagttcaagctgaactttcagatgcctacactggccagaggctgggacgtgaatagagagaagaacaatggcgccatcctgtttgtgaagaacggcctgtactatctgggcatcatgccaaagcagaagggcaggtataaggccctgagcttcgagcccacagagaaaaccagcgagggctttgataagatgtactatgactacttccctgatgccgccaagatgatcccaaagtgcagcacccagctgaaggccgtgacagcccactttcagacccacacaacccccatcctgctgtccaacaatttcatcgagcctctggagatcacaaaggagatctacgacctgaacaatcctgagaaggagccaaagaagtttcagacagcctacgccaagaaaaccggcgaccagaagggctacagagaggccctgtgcaagtggatcgacttcacaagggattttctgtccaagtataccaagacaacctctatcgatctgtctagcctgcggccatcctctcagtataaggacctgggcgagtactatgccgagctgaatcccctgctgtaccacatcagcttccagagaatcgccgagaaggagatcatggatgccgtggagacaggcaagctgtacctgttccagatctataacaaggactttgccaagggccaccacggcaagcctaatctgcacacactgtattggaccggcctgttttctccagagaacctggccaagacaagcatcaagctgaatggccaggccgagctgttctaccgccctaagtccaggatgaagaggatggcacaccggctgggagagaagatgctgaacaagaagctgaaggatcagaaaaccccaatccccgacaccctgtaccaggagctgtacgactatgtgaatcacagactgtcccacgacctgtctgatgaggccagggccctgctgcccaacgtgatcaccaaggaggtgtctcacgagatcatcaaggataggcgctttaccagcgacaagttctttttccacgtgcctatcacactgaactatcaggccgccaattccccatctaagttcaaccagagggtgaatgcctacctgaaggagcaccccgagacacctatcatcggcatcgcccggggcgagagaaacctgatctatatcacagtgatcgactccaccggcaagatcctggagcagcggagcctgaacaccatccagcagtttgattaccagaagaagctggacaacagggagaaggagagggtggcagcaaggcaggcctggtctgtggtgggcacaatcaaggatctgaagcagggctatctgagccaggtcatccacgagatcgtggacctgatgatccactaccaggccgtggtggtgctggagaacctgaatttcggctttaagagcaagaggaccggcatcgccgagaaggccgtgtaccagcagttcgagaagatgctgatcgataagctgaattgcctggtgctgaaggactatccagcagagaaagtgggaggcgtgctgaacccataccagctgacagaccagttcacctcctttgccaagatgggcacccagtctggcttcctgttttacgtgcctgccccatatacatctaagatcgatcccctgaccggcttcgtggaccccttcgtgtggaaaaccatcaagaatcacgagagccgcaagcacttcctggagggcttcgactttctgcactacgacgtgaaaaccggcgacttcatcctgcactttaagatgaacagaaatctgtccttccagaggggcctgcccggctttatgcctgcatgggatatcgtgttcgagaagaacgagacacagtttgacgccaagggcacccctttcatcgccggcaagagaatcgtgccagtgatcgagaatcacagattcaccggcagataccgggacctgtatcctgccaacgagctgatcgccctgctggaggagaagggcatcgtgttcagggatggctccaacatcctgccaaagctgctggagaatgacgattctcacgccatcgacacgatggtggccctgatccgcagcgtgctgcagatgcggaactccaatgccgccacaggcgaggactatatcaacagccccgtgcgcgatctgaatggcgtgtgcttcgactcccggtttcagaacccagagtggccaatggacgccgatgccaatggcgcctaccacatcgccctgaagggccagctgctgctgaatcacctgaaggagagcaaggatctgaagctgcagaacggcatctccaatcaggactggctggcctacatccaggagctgcgcaacaaaaggccggcggccacgaaaaaggccggccaggcaaaaaagaaaaagggatcctctggtggttctggaggatctggtggttctactaatctgtcagatattattgaaaaggagaccggtaagcaactggttatccaggaatccatcctcatgctcccagaggaggtggaagaagtcattgggaacaagccggaaagcgatatactcgtgcacaccgcctacgacgagagcaccgacgagaatgtcatgcttctgactagcgacgcccctgaatacaagccttgggctctggtcatacaggatagcaacggtgagaacaagattaagatgctctctggtggttctcccaagaagaagaggaaagtctaa

SEQ ID NO: 442 - DNA, 5019 bp, synthetic construct
  misc_feature 1..5019: note = Description of Artificial Sequence: Synthetic polynucleotide
  source 1..5019: mol_type = other DNA
atgggcagctcagagactggcccagtggctgtggaccccacattgagacggcggatcgagccccatgagtttgaggtattcttcgatccgagagagctccgcaaggagacctgcctgctttacgaaattaattgggggggccggcactccatttggcgacatacatcacagaacactaacaagcacgtcgaagtcaacttcatcgagaagttcacgacagaaagatatttctgtccgaacacaaggtgcagcattacctggtttctcagctggagcccatgcggcgaatgtagtagggccatcactgaattcctgtcaaggtatccccacgtcactctgtttatttacatcgcaaggctgtaccaccacgctgacccccgcaatcgacaaggcctgcgggatttgatctcttcaggtgtgactatccaaattatgactgagcaggagtcaggatactgctggagaaactttgtgaattatagcccgagtaatgaagcccactggcctaggtatccccatctgtgggtacgactgtacgttcttgaactgtactgcatcatactgggcctgcctccttgtctcaacattctgagaaggaagcagccacagctgacattctttaccatcgctcttcagtcttgtcattaccagcgactgcccccacacattctctgggccaccgggttgaaatctggtggttcttctggtggttctagcggcagcgagactcccgggacctcagagtccgccacacccgaaagttccggagggagtagcggcgggtctacacagttcgagggctttaccaacctgtatcaggtgagcaagacactgcggtttgagctgatcccacagggcaagaccctgaagcacatccaggagcagggcttcatcgaggaggacaaggcccgcaatgatcactacaaggagctgaagcccatcatcgatcggatctacaagacctatgccgaccagtgcctgcagctggtgcagctggattgggagaacctgagcgccgccatcgactcctatagaaaggagaaaaccgaggagacaaggaacgccctgatcgaggagcaggccacatatcgcaatgccatccacgactacttcatcggccggacagacaacctgaccgatgccatcaataagagacacgccgagatctacaagggcctgttcaaggccgagctgtttaatggcaaggtgctgaagcagctgggcaccgtgaccacaaccgagcacgagaacgccctgctgcggagcttcgacaagtttacaacctacttctccggcttttatagaaacaggaagaacgtgttcagcgccgaggatatcagcacagccatcccacaccgcatcgtgcaggacaacttccccaagtttaaggagaattgtcacatcttcacacgcctgatcaccgccgtgcccagcctgcgggagcactttgagaacgtgaagaaggccatcggcatcttcgtgagcacctccatcgaggaggtgttttccttccctttttataaccagctgctgacacagacccagatcgacctgtataaccagctgctgggaggaatctctcgggaggcaggcaccgagaagatcaagggcctgaacgaggtgctgaatctggccatccagaagaatgatgagacagcccacatcatcgcctccctgccacacagattcatccccctgtttaagcagatcctgtccgataggaacaccctgtctttcatcctggaggagtttaagagcgacgaggaagtgatccagtccttctgcaagtacaagacactgctgagaaacgagaacgtgctggagacagccgaggccctgtttaacgagctgaacagcatcgacctgacacacatcttcatcagccacaagaagctggagacaatcagcagcgccctgtgcgaccactgggatacactgaggaatgccctgtatgagcggagaatctccgagctgacaggcaagatcaccaagtctgccaaggagaaggtgcagcgcagcctgaagcacgaggatatcaacctgcaggagatcatctctgccgcaggcaaggagctgagcgaggccttcaagcagaaaaccagcgagatcctgtcccacgcacacgccgccctggatcagccactgcctacaaccctgaagaagcaggaggagaaggagatcctgaagtctcagctggacagcctgctgggcctgtaccacctgctggactggtttgccgtggatgagtccaacgaggtggaccccgagttctctgcccggctgaccggcatcaagctggagatggagccttctctgagcttctacaacaaggccagaaattatgccaccaagaagccctactccgtggagaagttcaagctgaactttcagatgcctacactggccagaggctgggacgtgaatagagagaagaacaatggcgccatcctgtttgtgaagaacggcctgtactatctgggcatcatgccaaagcagaagggcaggtataaggccctgagcttcgagcccacagagaaaaccagcgagggctttgataagatgtactatgactacttccctgatgccgccaagatgatcccaaagtgcagcacccagctgaaggccgtgacagcccactttcagacccacacaacccccatcctgctgtccaacaatttcatcgagcctctggagatcacaaaggagatctacgacctgaacaatcctgagaaggagccaaagaagtttcagacagcctacgccaagaaaaccggcgaccagaagggctacagagaggccctgtgcaagtggatcgacttcacaagggattttctgtccaagtataccaagacaacctctatcgatctgtctagcctgcggccatcctctcagtataaggacctgggcgagtactatgccgagctgaatcccctgctgtaccacatcagcttccagagaatcgccgagaaggagatcatggatgccgtggagacaggcaagctgtacctgttccagatctataacaaggactttgccaagggccaccacggcaagcctaatctgcacacactgtattggaccggcctgttttctccagagaacctggccaagacaagcatcaagctgaatggccaggccgagctgttctaccgccctaagtccaggatgaagaggatggcacaccggctgggagagaagatgctgaacaagaagctgaaggatcagaaaaccccaatccccgacaccctgtaccaggagctgtacgactatgtgaatcacagactgtcccacgacctgtctgatgaggccagggccctgctgcccaacgtgatcaccaaggaggtgtctcacgagatcatcaaggataggcgctttaccagcgacaagttctttttccacgtgcctatcacactgaactatcaggccgccaattccccatctaagttcaaccagagggtgaatgcctacctgaaggagcaccccgagacacctatcatcggcatcgcccggggcgagagaaacctgatctatatcacagtgatcgactccaccggcaagatcctggagcagcggagcctgaacaccatccagcagtttgattaccagaagaagctggacaacagggagaaggagagggtggcagcaaggcaggcctggtctgtggtgggcacaatcaaggatctgaagcagggctatctgagccaggtcatccacgagatcgtggacctgatgatccactaccaggccgtggtggtgctggagaacctgaatttcggctttaagagcaagaggaccggcatcgccgagaaggccgtgtaccagcagttcgagaagatgctgatcgataagctgaattgcctggtgctgaaggactatccagcagagaaagtgggaggcgtgctgaacccataccagctgacagaccagttcacctcctttgccaagatgggcacccagtctggcttcctgttttacgtgcctgccccatatacatctaagatcgatcccctgaccggcttcgtggaccccttcgtgtggaaaaccatcaagaatcacgagagccgcaagcacttcctggagggcttcgactttctgcactacgacgtgaaaaccggcgacttcatcctgcactttaagatgaacagaaatctgtccttccagaggggcctgcccggctttatgcctgcatgggatatcgtgttcgagaagaacgagacacagtttgacgccaagggcacccctttcatcgccggcaagagaatcgtgccagtgatcgagaatcacagattcaccggcagataccgggacctgtatcctgccaacgagctgatcgccctgctggaggagaagggcatcgtgttcagggatggctccaacatcctgccaaagctgctggagaatgacgattctcacgccatcgacacgatggtggccctgatccgcagcgtgctgcagatgcggaactccaatgccgccacaggcgaggactatatcaacagccccgtgcgcgatctgaatggcgtgtgcttcgactcccggtttcagaacccagagtggccaatggacgccgatgccaatggcgcctaccacatcgccctgaagggccagctgctgctgaatcacctgaaggagagcaaggatctgaagctgcagaacggcatctccaatcaggactggctggcctacatccaggagctgcgcaactctggtggttctggaggatctggtggttctactaatctgtcagatattattgaaaaggagaccggtaagcaactggttatccaggaatccatcctcatgctcccagaggaggtggaagaagtcattgggaacaagccggaaagcgatatactcgtgcacaccgcctacgacgagagcaccgacgagaatgtcatgcttctgactagcgacgcccctgaatacaagccttgggctctggtcatacaggatagcaacggtgagaacaagattaagatgctctctggtggttctcccaagaagaagaggaaagtctaa

SEQ ID NO: 443 - DNA, 5421 bp, synthetic construct
  misc_feature 1..5421: note = Description of Artificial Sequence: Synthetic polynucleotide
  source 1..5421: mol_type = other DNA
atgagcaagctggagaagtttacaaactgctactccctgtctaagaccctgaggttcaaggccatccctgtgggcaagacccaggagaacatcgacaataagcggctgctggtggaggacgagaagagagccgaggattataagggcgtgaagaagctgctggatcgctactatctgtcttttatcaacgacgtgctgcacagcatcaagctgaagaatctgaacaattacatcagcctgttccggaagaaaaccagaaccgagaaggagaataaggagctggagaacctggagatcaatctgcggaaggagatcgccaaggccttcaagggcaacgagggctacaagtccctgtttaagaaggatatcatcgagacaatcctgccagagttcctggacgataaggacgagatcgccctggtgaacagcttcaatggctttaccacagccttcaccggcttctttgataacagagagaatatgttttccgaggaggccaagagcacatccatcgccttcaggtgtatcaacgagaatctgacccgctacatctctaatatggacatcttcgagaaggtggacgccatctttgataagcacgaggtgcaggagatcaaggagaagatcctgaacagcgactatgatgtggaggatttctttgagggcgagttctttaactttgtgctgacacaggagggcatcgacgtgtataacgccatcatcggcggcttcgtgaccgagagcggcgagaagatcaagggcctgaacgagtacatcaacctgtataatcagaaaaccaagcagaagctgcctaagtttaagccactgtataagcaggtgctgagcgatcgggagtctctgagcttctacggcgagggctatacatccgatgaggaggtgctggaggtgtttagaaacaccctgaacaagaacagcgagatcttcagctccatcaagaagctggagaagctgttcaagaattttgacgagtactctagcgccggcatctttgtgaagaacggccccgccatcagcacaatctccaaggatatcttcggcgagtggaacgtgatccgggacaagtggaatgccgagtatgacgatatccacctgaagaagaaggccgtggtgaccgagaagtacgaggacgatcggagaaagtccttcaagaagatcggctccttttctctggagcagctgcaggagtacgccgacgccgatctgtctgtggtggagaagctgaaggagatcatcatccagaaggtggatgagatctacaaggtgtatggctcctctgagaagctgttcgacgccgattttgtgctggagaagagcctgaagaagaacgacgccgtggtggccatcatgaaggacctgctggattctgtgaagagcttcgagaattacatcaaggccttctttggcgagggcaaggagacaaacagggacgagtccttctatggcgattttgtgctggcctacgacatcctgctgaaggtggaccacatctacgatgccatccgcaattatgtgacccagaagccctactctaaggataagttcaagctgtattttcagaaccctcagttcatgggcggctgggacaaggataaggagacagactatcgggccaccatcctgagatacggctccaagtactatctggccatcatggataagaagtacgccaagtgcctgcagaagatcgacaaggacgatgtgaacggcaattacgagaagatcaactataagctgctgcccggccctaataagatgctgccaaaggtgttcttttctaagaagtggatggcctactataaccccagcgaggacatccagaagatctacaagaatggcacattcaagaagggcgatatgtttaacctgaatgactgtcacaagctgatcgacttctttaaggatagcatctcccggtatccaaagtggtccaatgcctacgatttcaacttttctgagacagagaagtataaggacatcgccggcttttacagagaggtggaggagcagggctataaggtgagcttcgagtctgccagcaagaaggaggtggataagctggtggaggagggcaagctgtatatgttccagatctataacaaggacttttccgataagtctcacggcacacccaatctgcacaccatgtacttcaagctgctgtttgacgagaacaatcacggacagatcaggctgagcggaggagcagagctgttcatgaggcgcgcctccctgaagaaggaggagctggtggtgcacccagccaactcccctatcgccaacaagaatccagataatcccaagaaaaccacaaccctgtcctacgacgtgtataaggataagaggttttctgaggaccagtacgagctgcacatcccaatcgccatcaataagtgccccaagaacatcttcaagatcaatacagaggtgcgcgtgctgctgaagcacgacgataacccctatgtgatcggcatcgccaggggcgagcgcaatctgctgtatatcgtggtggtggacggcaagggcaacatcgtggagcagtattccctgaacgagatcatcaacaacttcaacggcatcaggatcaagacagattaccactctctgctggacaagaaggagaaggagaggttcgaggcccgccagaactggacctccatcgagaatatcaaggagctgaaggccggctatatctctcaggtggtgcacaagatctgcgagctggtggagaagtacgatgccgtgatcgccctggaggacctgaactctggctttaagaatagccgcgtgaaggtggagaagcaggtgtatcagaagttcgagaagatgctgatcgataagctgaactacatggtggacaagaagtctaatccttgtgcaacaggcggcgccctgaagggctatcagatcaccaataagttcgagagctttaagtccatgtctacccagaacggcttcatcttttacatccctgcctggctgacatccaagatcgatccatctaccggctttgtgaacctgctgaaaaccaagtataccagcatcgccgattccaagaagttcatcagctcctttgacaggatcatgtacgtgcccgaggaggatctgttcgagtttgccctggactataagaacttctctcgcacagacgccgattacatcaagaagtggaagctgtactcctacggcaaccggatcagaatcttccggaatcctaagaagaacaacgtgttcgactgggaggaggtgtgcctgaccagcgcctataaggagctgttcaacaagtacggcatcaattatcagcagggcgatatcagagccctgctgtgcgagcagtccgacaaggccttctactctagctttatggccctgatgagcctgatgctgcagatgcggaacagcatcacaggccgcaccgacgtggattttctgatcagccctgtgaagaactccgacggcatcttctacgatagccggaactatgaggcccaggagaatgccatcctgccaaagaacgccgacgccaatggcgcctataacatcgccagaaaggtgctgtgggccatcggccagttcaagaaggccgaggacgagaagctggataaggtgaagatcgccatctctaacaaggagtggctggagtacgcccagaccagcgtgaagcacaaaaggccggcggccacgaaaaaggccggccaggcaaaaaagaaaaagggatcctacccatacgatgttccagattacgcttatccctacgacgtgcctgattatgcatacccatatgatgtccccgactatgccggaagcgaggccagcggttccggacgggctgacgcattggacgattttgatctggatatgctgggaagtgacgccctcgatgattttgaccttgacatgcttggttcggatgcccttgatgactttgacctcgacatgctcggcagtgacgcccttgatgatttcgacctggacatgctgattaactctagaagttccggatctccgaaaaagaaacgcaaagttggtagccagtacctgcccgacaccgacgaccggcaccggatcgaggaaaagcggaagcggacctacgagacattcaagagcatcatgaagaagtcccccttcagcggccccaccgaccctagacctccacctagaagaatcgccgtgcccagcagatccagcgccagcgtgccaaaacctgccccccagccttaccccttcaccagcagcctgagcaccatcaactacgacgagttccctaccatggtgttccccagcggccagatctctcaggcctctgctctggctccagcccctcctcaggtgctgcctcaggctcctgctcctgcaccagctccagccatggtgtctgcactggctcaggcaccagcacccgtgcctgtgctggctcctggacctccacaggctgtggctccaccagcccctaaacctacacaggccggcgagggcacactgtctgaagctctgctgcagctgcagttcgacgacgaggatctgggagccctgctgggaaacagcaccgatcctgccgtgttcaccgacctggccagcgtggacaacagcgagttccagcagctgctgaaccagggcatccctgtggcccctcacaccaccgagcccatgctgatggaataccccgaggccatcacccggctcgtgacaggcgctcagaggcctcctgatccagctcctgcccctctgggagcaccaggcctgcctaatggactgctgtctggcgacgaggacttcagctctatcgccgatatggatttctcagccttgctgggctctggcagcggcagccgggattccagggaagggatgtttttgccgaagcctgaggccggctccgctattagtgacgtgtttgagggccgcgaggtgtgccagccaaaacgaatccggccatttcatcctccaggaagtccatgggccaaccgcccactccccgccagcctcgcaccaacaccaaccggtccagtacatgagccagtcgggtcactgaccccggcaccagtccctcagccactggatccagcgcccgcagtgactcccgaggccagtcacctgttggaggatcccgatgaagagacgagccaggctgtcaaagcccttcgggagatggccgatactgtgattccccagaaggaagaggctgcaatctgtggccaaatggacctttcccatccgcccccaaggggccatctggatgagctgacaaccacacttgagtccatgaccgaggatctgaacctggactcacccctgaccccggaattgaacgagattctggataccttcctgaacgacgagtgcctcttgcatgccatgcatatcagcacaggactgtccatcttcgacacatctctgttttaa

SEQ ID NO: 444 - protein, 1806 aa, synthetic construct
  REGION 1..1806: note = Description of Artificial Sequence: Synthetic polypeptide
MSKLEKFTNCYSLSKTLRFKAIPVGKTQENIDNKRLLVEDEKRAEDYKGVKKLLDRYYLSFINDVLHSIKLKNLNNYISLFRKKTRTEKENKELENLEINLRKEIAKAFKGNEGYKSLFKKDIIETILPEFLDDKDEIALVNSFNGFTTAFTGFFDNRENMFSEEAKSTSIAFRCINENLTRYISNMDIFEKVDAIFDKHEVQEIKEKILNSDYDVEDFFEGEFFNFVLTQEGIDVYNAIIGGFVTESGEKIKGLNEYINLYNQKTKQKLPKFKPLYKQVLSDRESLSFYGEGYTSDEEVLEVFRNTLNKNSEIFSSIKKLEKLFKNFDEYSSAGIFVKNGPAISTISKDIFGEWNVIRDKWNAEYDDIHLKKKAVVTEKYEDDRRKSFKKIGSFSLEQLQEYADADLSVVEKLKEIIIQKVDEIYKVYGSSEKLFDADFVLEKSLKKNDAVVAIMKDLLDSVKSFENYIKAFFGEGKETNRDESFYGDFVLAYDILLKVDHIYDAIRNYVTQKPYSKDKFKLYFQNPQFMGGWDKDKETDYRATILRYGSKYYLAIMDKKYAKCLQKIDKDDVNGNYEKINYKLLPGPNKMLPKVFFSKKWMAYYNPSEDIQKIYKNGTFKKGDMFNLNDCHKLIDFFKDSISRYPKWSNAYDFNFSETEKYKDIAGFYREVEEQGYKVSFESASKKEVDKLVEEGKLYMFQIYNKDFSDKSHGTPNLHTMYFKLLFDENNHGQIRLSGGAELFMRRASLKKEELVVHPANSPIANKNPDNPKKTTTLSYDVYKDKRFSEDQYELHIPIAINKCPKNIFKINTEVRVLLKHDDNPYVIGIARGERNLLYIVVVDGKGNIVEQYSLNEIINNFNGIRIKTDYHSLLDKKEKERFEARQNWTSIENIKELKAGYISQVVHKICELVEKYDAVIALEDLNSGFKNSRVKVEKQVYQKFEKMLIDKLNYMVDKKSNPCATGGALKGYQITNKFESFKSMSTQNGFIFYIPAWLTSKIDPSTGFVNLLKTKYTSIADSKKFISSFDRIMYVPEEDLFEFALDYKNFSRTDADYIKKWKLYSYGNRIRIFRNPKKNNVFDWEEVCLTSAYKELFNKYGINYQQGDIRALLCEQSDKAFYSSFMALMSLMLQMRNSITGRTDVDFLISPVKNSDGIFYDSRNYEAQENAILPKNADANGAYNIARKVLWAIGQFKKAEDEKLDKVKIAISNKEWLEYAQTSVKHKRPAATKKAGQAKKKKGSYPYDVPDYAYPYDVPDYAYPYDVPDYAGSEASGSGRADALDDFDLDMLGSDALDDFDLDMLGSDALDDFDLDMLGSDALDDFDLDMLINSRSSGSPKKKRKVGSQYLPDTDDRHRIEEKRKRTYETFKSIMKKSPFSGPTDPRPPPRRIAVPSRSSASVPKPAPQPYPFTSSLSTINYDEFPTMVFPSGQISQASALAPAPPQVLPQAPAPAPAPAMVSALAQAPAPVPVLAPGPPQAVAPPAPKPTQAGEGTLSEALLQLQFDDEDLGALLGNSTDPAVFTDLASVDNSEFQQLLNQGIPVAPHTTEPMLMEYPEAITRLVTGAQRPPDPAPAPLGAPGLPNGLLSGDEDFSSIADMDFSALLGSGSGSRDSREGMFLPKPEAGSAISDVFEGREVCQPKRIRPFHPPGSPWANRPLPASLAPTPTGPVHEPVGSLTPAPVPQPLDPAPAVTPEASHLLEDPDEETSQAVKALREMADTVIPQKEEAAICGQMDLSHPPPRGHLDELTTTLESMTEDLNLDSPLTPELNEILDTFLNDECLLHAMHISTGLSIFDTSLF

SEQ ID NO: 445 - DNA, 5130 bp, synthetic construct
  misc_feature 1..5130: note = Description of Artificial Sequence: Synthetic polynucleotide
  source 1..5130: mol_type = other DNA
atgggcccaaagaaaaagaggaaagtcggcagtggacctaaaaagaaacgaaaggttgggtcaggtagctcagagactggcccagtggctgtggaccccacattgagacggcggatcgagccccatgagtttgaggtattcttcgatccgagagagctccgcaaggagacctgcctgctttacgaaattaattgggggggccggcactccatttggcgacatacatcacagaacactaacaagcacgtcgaagtcaacttcatcgagaagttcacgacagaaagatatttctgtccgaacacaaggtgcagcattacctggtttctcagctggagcccatgcggcgaatgtagtagggccatcactgaattcctgtcaaggtatccccacgtcactctgtttatttacatcgcaaggctgtaccaccacgctgacccccgcaatcgacaaggcctgcgggatttgatctcttcaggtgtgactatccaaattatgactgagcaggagtcaggatactgctggagaaactttgtgaattatagcccgagtaatgaagcccactggcctaggtatccccatctgtgggtacgactgtacgttcttgaactgtactgcatcatactgggcctgcctccttgtctcaacattctgagaaggaagcagccacagctgacattctttaccatcgctcttcagtcttgtcattaccagcgactgcccccacacattctctgggccaccgggttgaaatctggtggttcttctggtggttctagcggcagcgagactcccgggacctcagagtccgccacacccgaaagttccggagggagtagcggcgggtctacacagttcgagggctttaccaacctgtatcaggtgagcaagacactgcggtttgagctgatcccacagggcaagaccctgaagcacatccaggagcagggcttcatcgaggaggacaaggcccgcaatgatcactacaaggagctgaagcccatcatcgatcggatctacaagacctatgccgaccagtgcctgcagctggtgcagctggattgggagaacctgagcgccgccatcgactcctatagaaaggagaaaaccgaggagacaaggaacgccctgatcgaggagcaggccacatatcgcaatgccatccacgactacttcatcggccggacagacaacctgaccgatgccatcaataagagacacgccgagatctacaagggcctgttcaaggccgagctgtttaatggcaaggtgctgaagcagctgggcaccgtgaccacaaccgagcacgagaacgccctgctgcggagcttcgacaagtttacaacctacttctccggcttttatgagaacaggaagaacgtgttcagcgccgaggatatcagcacagccatcccacaccgcatcgtgcaggacaacttccccaagtttaaggagaattgtcacatcttcacacgcctgatcaccgccgtgcccagcctgcgggagcactttgagaacgtgaagaaggccatcggcatcttcgtgagcacctccatcgaggaggtgttttccttccctttttataaccagctgctgacacagacccagatcgacctgtataaccagctgctgggaggaatctctcgggaggcaggcaccgagaagatcaagggcctgaacgaggtgctgaatctggccatccagaagaatgatgagacagcccacatcatcgcctccctgccacacagattcatccccctgtttaagcagatcctgtccgataggaacaccctgtctttcatcctggaggagtttaagagcgacgaggaagtgatccagtccttctgcaagtacaagacactgctgagaaacgagaacgtgctggagacagccgaggccctgtttaacgagctgaacagcatcgacctgacacacatcttcatcagccacaagaagctggagacaatcagcagcgccctgtgcgaccactgggatacactgaggaatgccctgtatgagcggagaatctccgagctgacaggcaagatcaccaagtctgccaaggagaaggtgcagcgcagcctgaagcacgaggatatcaacctgcaggagatcatctctgccgcaggcaaggagctgagcgaggccttcaagcagaaaaccagcgagatcctgtcccacgcacacgccgccctggatcagccactgcctacaaccctgaagaagcaggaggagaaggagatcctgaagtctcagctggacagcctgctgggcctgtaccacctgctggactggtttgccgtggatgagtccaacgaggtggaccccgagttctctgcccggctgaccggcatcaagctggagatggagccttctctgagcttctacaacaaggccagaaattatgccaccaagaagccctactccgtggagaagttcaagctgaactttcagatgcctacactggcctctggctgggacgtgaataaggagaagaacaatggcgccatcctgtttgtgaagaacggcctgtactatctgggcatcatgccaaagcagaagggcaggtataaggccctgagcttcgagcccacagagaaaaccagcgagggctttgataagatgtactatgactacttccctgatgccgccaagatgatcccaaagtgcagcacccagctgaaggccgtgacagcccactttcagacccacacaacccccatcctgctgtccaacaatttcatcgagcctctggagatcacaaaggagatctacgacctgaacaatcctgagaaggagccaaagaagtttcagacagcctacgccaagaaaaccggcgaccagaagggctacagagaggccctgtgcaagtggatcgacttcacaagggattttctgtccaagtataccaagacaacctctatcgatctgtctagcctgcggccatcctctcagtataaggacctgggcgagtactatgccgagctgaatcccctgctgtaccacatcagcttccagagaatcgccgagaaggagatcatggatgccgtggagacaggcaagctgtacctgttccagatctataacaaggactttgccaagggccaccacggcaagcctaatctgcacacactgtattggaccggcctgttttctccagagaacctggccaagacaagcatcaagctgaatggccaggccgagctgttctaccgccctaagtccaggatgaagaggatggcacaccggctgggagagaagatgctgaacaagaagctgaaggatcagaaaaccccaatccccgacaccctgtaccaggagctgtacgactatgtgaatcacagactgtcccacgacctgtctgatgaggccagggccctgctgcccaacgtgatcaccaaggaggtgtctcacgagatcatcaaggataggcgctttaccagcgacaagttctttttccacgtgcctatcacactgaactatcaggccgccaattccccatctaagttcaaccagagggtgaatgcctacctgaaggagcaccccgagacacctatcatcggcatcgcccggggcgagagaaacctgatctatatcacagtgatcgactccaccggcaagatcctggagcagcggagcctgaacaccatccagcagtttgattaccagaagaagctggacaacagggagaaggagagggtggcagcaaggcaggcctggtctgtggtgggcacaatcaaggatctgaagcagggctatctgagccaggtcatccacgagatcgtggacctgatgatccactaccaggccgtggtggtgctggagaacctgaatttcggctttaagagcaagaggaccggcatcgccgagaaggccgtgtaccagcagttcgagaagatgctgatcgataagctgaattgcctggtgctgaaggactatccagcagagaaagtgggaggcgtgctgaacccataccagctgacagaccagttcacctcctttgccaagatgggcacccagtctggcttcctgttttacgtgcctgccccatatacatctaagatcgatcccctgaccggcttcgtggaccccttcgtgtggaaaaccatcaagaatcacgagagccgcaagcacttcctggagggcttcgactttctgcactacgacgtgaaaaccggcgacttcatcctgcactttaagatgaacagaaatctgtccttccagaggggcctgcccggctttatgcctgcatgggatatcgtgttcgagaagaacgagacacagtttgacgccaagggcacccctttcatcgccggcaagagaatcgtgccagtgatcgagaatcacagattcaccggcagataccgggacctgtatcctgccaacgagctgatcgccctgctggaggagaagggcatcgtgttcagggatggctccaacatcctgccaaagctgctggagaatgacgattctcacgccatcgacacgatggtggccctgatccgcagcgtgctgcagatgcggaactccaatgccgccacaggcgaggactatatcaacagccccgtgcgcgatctgaatggcgtgtgcttcgactcccggtttcagaacccagagtggccaatggacgccgatgccaatggcgcctaccacatcgccctgaagggccagctgctgctgaatcacctgaaggagagcaaggatctgaagctgcagaacggcatctccaatcaggactggctggcctacatccaggagctgcgcaacaaaaggccggcggccacgaaaaaggccggccaggcaaaaaagaaaaagggatcctctggtggttctggaggatctggtggttctactaatctgtcagatattattgaaaaggagaccggtaagcaactggttatccaggaatccatcctcatgctcccagaggaggtggaagaagtcattgggaacaagccggaaagcgatatactcgtgcacaccgcctacgacgagagcaccgacgagaatgtcatgcttctgactagcgacgcccctgaatacaagccttgggctctggtcatacaggatagcaacggtgagaacaagattaagatgctctctggtggttctcccaagaagaagaggaaagtc

SEQ ID NO: 446 - protein, 1710 aa, synthetic construct
  REGION 1..1710: note = Description of Artificial Sequence: Synthetic polypeptide
MGPKKKRKVGSGPKKKRKVGSGSSETGPVAVDPTLRRRIEPHEFEVFFDPRELRKETCLLYEINWGGRHSIWRHTSQNTNKHVEVNFIEKFTTERYFCPNTRCSITWFLSWSPCGECSRAITEFLSRYPHVTLFIYIARLYHHADPRNRQGLRDLISSGVTIQIMTEQESGYCWRNFVNYSPSNEAHWPRYPHLWVRLYVLELYCIILGLPPCLNILRRKQPQLTFFTIALQSCHYQRLPPHILWATGLKSGGSSGGSSGSETPGTSESATPESSGGSSGGSTQFEGFTNLYQVSKTLRFELIPQGKTLKHIQEQGFIEEDKARNDHYKELKPIIDRIYKTYADQCLQLVQLDWENLSAAIDSYRKEKTEETRNALIEEQATYRNAIHDYFIGRTDNLTDAINKRHAEIYKGLFKAELFNGKVLKQLGTVTTTEHENALLRSFDKFTTYFSGFYENRKNVFSAEDISTAIPHRIVQDNFPKFKENCHIFTRLITAVPSLREHFENVKKAIGIFVSTSIEEVFSFPFYNQLLTQTQIDLYNQLLGGISREAGTEKIKGLNEVLNLAIQKNDETAHIIASLPHRFIPLFKQILSDRNTLSFILEEFKSDEEVIQSFCKYKTLLRNENVLETAEALFNELNSIDLTHIFISHKKLETISSALCDHWDTLRNALYERRISELTGKITKSAKEKVQRSLKHEDINLQEIISAAGKELSEAFKQKTSEILSHAHAALDQPLPTTLKKQEEKEILKSQLDSLLGLYHLLDWFAVDESNEVDPEFSARLTGIKLEMEPSLSFYNKARNYATKKPYSVEKFKLNFQMPTLASGWDVNKEKNNGAILFVKNGLYYLGIMPKQKGRYKALSFEPTEKTSEGFDKMYYDYFPDAAKMIPKCSTQLKAVTAHFQTHTTPILLSNNFIEPLEITKEIYDLNNPEKEPKKFQTAYAKKTGDQKGYREALCKWIDFTRDFLSKYTKTTSIDLSSLRPSSQYKDLGEYYAELNPLLYHISFQRIAEKEIMDAVETGKLYLFQIYNKDFAKGHHGKPNLHTLYWTGLFSPENLAKTSIKLNGQAELFYRPKSRMKRMAHRLGEKMLNKKLKDQKTPIPDTLYQELYDYVNHRLSHDLSDEARALLPNVITKEVSHEIIKDRRFTSDKFFFHVPITLNYQAANSPSKFNQRVNAYLKEHPETPIIGIARGERNLIYITVIDSTGKILEQRSLNTIQQFDYQKKLDNREKERVAARQAWSVVGTIKDLKQGYLSQVIHEIVDLMIHYQAVVVLENLNFGFKSKRTGIAEKAVYQQFEKMLIDKLNCLVLKDYPAEKVGGVLNPYQLTDQFTSFAKMGTQSGFLFYVPAPYTSKIDPLTGFVDPFVWKTIKNHESRKHFLEGFDFLHYDVKTGDFILHFKMNRNLSFQRGLPGFMPAWDIVFEKNETQFDAKGTPFIAGKRIVPVIENHRFTGRYRDLYPANELIALLEEKGIVFRDGSNILPKLLENDDSHAIDTMVALIRSVLQMRNSNAATGEDYINSPVRDLNGVCFDSRFQNPEWPMDADANGAYHIALKGQLLLNHLKESKDLKLQNGISNQDWLAYIQELRNKRPAATKKAGQAKKKKGSSGGSGGSGGSTNLSDIIEKETGKQLVIQESILMLPEEVEEVIGNKPESDILVHTAYDESTDENVMLLTSDAPEYKPWALVIQDSNGENKIKMLSGGSPKKKRKV

SEQ ID NO: 447 - DNA, 5130 bp, synthetic construct
  misc_feature 1..5130: note = Description of Artificial Sequence: Synthetic polynucleotide
  source 1..5130: mol_type = other DNA
atgggcccaaagaaaaagaggaaagtcggcagtggacctaaaaagaaacgaaaggttgggtcaggtagctcagagactggcccagtggctgtggaccccacattgagacggcggatcgagccccatgagtttgaggtattcttcgatccgagagagctccgcaaggagacctgcctgctttacgaaattaattgggggggccggcactccatttggcgacatacatcacagaacactaacaagcacgtcgaagtcaacttcatcgagaagttcacgacagaaagatatttctgtccgaacacaaggtgcagcattacctggtttctcagctggagcccatgcggcgaatgtagtagggccatcactgaattcctgtcaaggtatccccacgtcactctgtttatttacatcgcaaggctgtaccaccacgctgacccccgcaatcgacaaggcctgcgggatttgatctcttcaggtgtgactatccaaattatgactgagcaggagtcaggatactgctggagaaactttgtgaattatagcccgagtaatgaagcccactggcctaggtatccccatctgtgggtacgactgtacgttcttgaactgtactgcatcatactgggcctgcctccttgtctcaacattctgagaaggaagcagccacagctgacattctttaccatcgctcttcagtcttgtcattaccagcgactgcccccacacattctctgggccaccgggttgaaatctggtggttcttctggtggttctagcggcagcgagactcccgggacctcagagtccgccacacccgaaagttccggagggagtagcggcgggtctacacagttcgagggctttaccaacctgtatcaggtgagcaagacactgcggtttgagctgatcccacagggcaagaccctgaagcacatccaggagcagggcttcatcgaggaggacaaggcccgcaatgatcactacaaggagctgaagcccatcatcgatcggatctacaagacctatgccgaccagtgcctgcagctggtgcagctggattgggagaacctgagcgccgccatcgactcctatagaaaggagaaaaccgaggagacaaggaacgccctgatcgaggagcaggccacatatcgcaatgccatccacgactacttcatcggccggacagacaacctgaccgatgccatcaataagagacacgccgagatctacaagggcctgttcaaggccgagctgtttaatggcaaggtgctgaagcagctgggcaccgtgaccacaaccgagcacgagaacgccctgctgcggagcttcgacaagtttacaacctacttctccggcttttatgccaacaggaagaacgtgttcagcgccgaggatatcagcacagccatcccacaccgcatcgtgcaggacaacttccccaagtttaaggagaattgtcacatcttcacacgcctgatcaccgccgtgcccagcctgcgggagcactttgagaacgtgaagaaggccatcggcatcttcgtgagcacctccatcgaggaggtgttttccttccctttttataaccagctgctgacacagacccagatcgacctgtataaccagctgctgggaggaatctctcgggaggcaggcaccgagaagatcaagggcctgaacgaggtgctgaatctggccatccagaagaatgatgagacagcccacatcatcgcctccctgccacacagattcatccccctgtttaagcagatcctgtccgataggaacaccctgtctttcatcctggaggagtttaagagcgacgaggaagtgatccagtccttctgcaagtacaagacactgctgagaaacgagaacgtgctggagacagccgaggccctgtttaacgagctgaacagcatcgacctgacacacatcttcatcagccacaagaagctggagacaatcagcagcgccctgtgcgaccactgggatacactgaggaatgccctgtatgagcggagaatctccgagctgacaggcaagatcaccaagtctgccaaggagaaggtgcagcgcagcctgaagcacgaggatatcaacctgcaggagatcatctctgccgcaggcaaggagctgagcgaggccttcaagcagaaaaccagcgagatcctgtcccacgcacacgccgccctggatcagccactgcctacaaccctgaagaagcaggaggagaaggagatcctgaagtctcagctggacagcctgctgggcctgtaccacctgctggactggtttgccgtggatgagtccaacgaggtggaccccgagttctctgcccggctgaccggcatcaagctggagatggagccttctctgagcttctacaacaaggccagaaattatgccaccaagaagccctactccgtggagaagttcaagctgaactttcagatgcctacactggccgccggctgggacgtgaataaggccaagaacaatggcgccatcctgtttgtgaagaacggcctgtactatctgggcatcatgccaaagcagaagggcaggtataaggccctgagcttcgagcccacagagaaaaccagcgagggctttgataagatgtactatgactacttccctgatgccgccaagatgatcccaaagtgcagcacccagctgaaggccgtgacagcccactttcagacccacacaacccccatcctgctgtccaacaatttcatcgagcctctggagatcacaaaggagatctacgacctgaacaatcctgagaaggagccaaagaagtttcagacagcctacgccaagaaaaccggcgaccagaagggctacagagaggccctgtgcaagtggatcgacttcacaagggattttctgtccaagtataccaagacaacctctatcgatctgtctagcctgcggccatcctctcagtataaggacctgggcgagtactatgccgagctgaatcccctgctgtaccacatcagcttccagagaatcgccgagaaggagatcatggatgccgtggagacaggcaagctgtacctgttccagatctataacaaggactttgccaagggccaccacggcaagcctaatctgcacacactgtattggaccggcctgttttctccagagaacctggccaagacaagcatcaagctgaatggccaggccgagctgttctaccgccctaagtccaggatgaagaggatggcacaccggctgggagagaagatgctgaacaagaagctgaaggatcagaaaaccccaatccccgacaccctgtaccaggagctgtacgactatgtgaatcacagactgtcccacgacctgtctgatgaggccagggccctgctgcccaacgtgatcaccaaggaggtgtctcacgagatcatcaaggataggcgctttaccagcgacaagttctttttccacgtgcctatcacactgaactatcaggccgccaattccccatctaagttcaaccagagggtgaatgcctacctgaaggagcaccccgagacacctatcatcggcatcgcccggggcgagagaaacctgatctatatcacagtgatcgactccaccggcaagatcctggagcagcggagcctgaacaccatccagcagtttgattaccagaagaagctggacaacagggagaaggagagggtggcagcaaggcaggcctggtctgtggtgggcacaatcaaggatctgaagcagggctatctgagccaggtcatccacgagatcgtggacctgatgatccactaccaggccgtggtggtgctggagaacctgaatttcggctttaagagcaagaggaccggcatcgccgagaaggccgtgtaccagcagttcgagaagatgctgatcgataagctgaattgcctggtgctgaaggactatccagcagagaaagtgggaggcgtgctgaacccataccagctgacagaccagttcacctcctttgccaagatgggcacccagtctggcttcctgttttacgtgcctgccccatatacatctaagatcgatcccctgaccggcttcgtggaccccttcgtgtggaaaaccatcaagaatcacgagagccgcaagcacttcctggagggcttcgactttctgcactacgacgtgaaaaccggcgacttcatcctgcactttaagatgaacagaaatctgtccttccagaggggcctgcccggctttatgcctgcatgggatatcgtgttcgagaagaacgagacacagtttgacgccaagggcacccctttcatcgccggcaagagaatcgtgccagtgatcgagaatcacagattcaccggcagataccgggacctgtatcctgccaacgagctgatcgccctgctggaggagaagggcatcgtgttcagggatggctccaacatcctgccaaagctgctggagaatgacgattctcacgccatcgacacgatggtggccctgatccgcagcgtgctgcagatgcggaactccaatgccgccacaggcgaggactatatcaacagccccgtgcgcgatctgaatggcgtgtgcttcgactcccggtttcagaacccagagtggccaatggacgccgatgccaatggcgcctaccacatcgccctgaagggccagctgctgctgaatcacctgaaggagagcaaggatctgaagctgcagaacggcatctccaatcaggactggctggcctacatccaggagctgcgcaacaaaaggccggcggccacgaaaaaggccggccaggcaaaaaagaaaaagggatcctctggtggttctggaggatctggtggttctactaatctgtcagatattattgaaaaggagaccggtaagcaactggttatccaggaatccatcctcatgctcccagaggaggtggaagaagtcattgggaacaagccggaaagcgatatactcgtgcacaccgcctacgacgagagcaccgacgagaatgtcatgcttctgactagcgacgcccctgaatacaagccttgggctctggtcatacaggatagcaacggtgagaacaagattaagatgctctctggtggttctcccaagaagaagaggaaagtc

SEQ ID NO: 448 - protein, 1710 aa, synthetic construct
  REGION 1..1710: note = Description of Artificial Sequence: Synthetic polypeptide
MGPKKKRKVGSGPKKKRKVGSGSSETGPVAVDPTLRRRIEPHEFEVFFDPRELRKETCLLYEINWGGRHSIWRHTSQNTNKHVEVNFIEKFTTERYFCPNTRCSITWFLSWSPCGECSRAITEFLSRYPHVTLFIYIARLYHHADPRNRQGLRDLISSGVTIQIMTEQESGYCWRNFVNYSPSNEAHWPRYPHLWVRLYVLELYCIILGLPPCLNILRRKQPQLTFFTIALQSCHYQRLPPHILWATGLKSGGSSGGSSGSETPGTSESATPESSGGSSGGSTQFEGFTNLYQVSKTLRFELIPQGKTLKHIQEQGFIEEDKARNDHYKELKPIIDRIYKTYADQCLQLVQLDWENLSAAIDSYRKEKTEETRNALIEEQATYRNAIHDYFIGRTDNLTDAINKRHAEIYKGLFKAELFNGKVLKQLGTVTTTEHENALLRSFDKFTTYFSGFYRNRKNVFSAEDISTAIPHRIVQDNFPKFKENCHIFTRLITAVPSLREHFENVKKAIGIFVSTSIEEVFSFPFYNQLLTQTQIDLYNQLLGGISREAGTEKIKGLNEVLNLAIQKNDETAHIIASLPHRFIPLFKQILSDRNTLSFILEEFKSDEEVIQSFCKYKTLLRNENVLETAEALFNELNSIDLTHIFISHKKLETISSALCDHWDTLRNALYERRISELTGKITKSAKEKVQRSLKHEDINLQEIISAAGKELSEAFKQKTSEILSHAHAALDQPLPTTLKKQEEKEILKSQLDSLLGLYHLLDWFAVDESNEVDPEFSARLTGIKLEMEPSLSFYNKARNYATKKPYSVEKFKLNFQMPTLARGWDVNREKNNGAILFVKNGLYYLGIMPKQKGRYKALSFEPTEKTSEGFDKMYYDYFPDAAKMIPKCSTQLKAVTAHFQTHTTPILLSNNFIEPLEITKEIYDLNNPEKEPKKFQTAYAKKTGDQKGYREALCKWIDFTRDFLSKYTKTTSIDLSSLRPSSQYKDLGEYYAELNPLLYHISFQRIAEKEIMDAVETGKLYLFQIYNKDFAKGHHGKPNLHTLYWTGLFSPENLAKTSIKLNGQAELFYRPKSRMKRMAHRLGEKMLNKKLKDQKTPIPDTLYQELYDYVNHRLSHDLSDEARALLPNVITKEVSHEIIKDRRFTSDKFFFHVPITLNYQAANSPSKFNQRVNAYLKEHPETPIIGIARGERNLIYITVIDSTGKILEQRSLNTIQQFDYQKKLDNREKERVAARQAWSVVGTIKDLKQGYLSQVIHEIVDLMIHYQAVVVLENLNFGFKSKRTGIAEKAVYQQFEKMLIDKLNCLVLKDYPAEKVGGVLNPYQLTDQFTSFAKMGTQSGFLFYVPAPYTSKIDPLTGFVDPFVWKTIKNHESRKHFLEGFDFLHYDVKTGDFILHFKMNRNLSFQRGLPGFMPAWDIVFEKNETQFDAKGTPFIAGKRIVPVIENHRFTGRYRDLYPANELIALLEEKGIVFRDGSNILPKLLENDDSHAIDTMVALIRSVLQMRNSNAATGEDYINSPVRDLNGVCFDSRFQNPEWPMDADANGAYHIALKGQLLLNHLKESKDLKLQNGISNQDWLAYIQELRNKRPAATKKAGQAKKKKGSSGGSGGSGGSTNLSDIIEKETGKQLVIQESILMLPEEVEEVIGNKPESDILVHTAYDESTDENVMLLTSDAPEYKPWALVIQDSNGENKIKMLSGGSPKKKRKV

SEQ ID NO: 449 - DNA, 24 bp, synthetic construct
  misc_feature 1..24: note = Description of Artificial Sequence: Synthetic oligonucleotide
  modified_base 4: mod_base = OTHER; note = a, c, t, g, unknown or other
  source 1..24: mol_type = other DNA
tttnctgatggtccatgtctgtta

SEQ ID NO: 450 - DNA, 24 bp, synthetic construct
  misc_feature 1..24: note = Description of Artificial Sequence: Synthetic oligonucleotide
  source 1..24: mol_type = other DNA
tttcctgatggtccatgtctgaat

SEQ ID NO: 451 - DNA, 24 bp, synthetic construct
  misc_feature 1..24: note = Description of Artificial Sequence: Synthetic oligonucleotide
  source 1..24: mol_type = other DNA
tttcctgatggtccatgtctgtta

SEQ ID NO: 452 - DNA, 24 bp, synthetic construct
  misc_feature 1..24: note = Description of Artificial Sequence: Synthetic oligonucleotide
  source 1..24: mol_type = other DNA
tttcctgatggtccacatctgtta

SEQ ID NO: 453 - DNA, 24 bp, synthetic construct
  misc_feature 1..24: note = Description of Artificial Sequence: Synthetic oligonucleotide
  source 1..24: mol_type = other DNA
tttcctgatggtccatatctgtgg

SEQ ID NO: 454 - DNA, 24 bp, synthetic construct
  misc_feature 1..24: note = Description of Artificial Sequence: Synthetic oligonucleotide
  source 1..24: mol_type = other DNA
tttcctgatggtccatacctgtta

SEQ ID NO: 455 - DNA, 24 bp, synthetic construct
  misc_feature 1..24: note = Description of Artificial Sequence: Synthetic oligonucleotide
  source 1..24: mol_type = other DNA
tttcctgatggtccacgcctgtta

SEQ ID NO: 456 - DNA, 24 bp, synthetic construct
  misc_feature 1..24: note = Description of Artificial Sequence: Synthetic oligonucleotide
  source 1..24: mol_type = other DNA
gttcctgatggtccacatctgtta

SEQ ID NO: 457 - DNA, 24 bp, synthetic construct
  misc_feature 1..24: note = Description of Artificial Sequence: Synthetic oligonucleotide
  source 1..24: mol_type = other DNA
ttttgtgatgtttcatgtgtccta

SEQ ID NO: 458 - DNA, 24 bp, synthetic construct
  misc_feature 1..24: note = Description of Artificial Sequence: Synthetic oligonucleotide
  modified_base 4: mod_base = OTHER; note = a, c, t, g, unknown or other
  source 1..24: mol_type = other DNA
tttngctcagcaggcacctgcctc

SEQ ID NO: 459 - DNA, 24 bp, synthetic construct
  misc_feature 1..24: note = Description of Artificial Sequence: Synthetic oligonucleotide
  source 1..24: mol_type = other DNA
cttagctcagcaggcacctgccca

SEQ ID NO: 460 - DNA, 24 bp, synthetic construct
  misc_feature 1..24: note = Description of Artificial Sequence: Synthetic oligonucleotide
  source 1..24: mol_type = other DNA
tttggctcagcaggcacctgcctc

SEQ ID NO: 461 - DNA, 24 bp, synthetic construct
  misc_feature 1..24: note = Description of Artificial Sequence: Synthetic oligonucleotide
  source 1..24: mol_type = other DNA
agcagctcagcaggcacctgcctt

SEQ ID NO: 462 - DNA, 24 bp, synthetic construct
  misc_feature 1..24: note = Description of Artificial Sequence: Synthetic oligonucleotide
  source 1..24: mol_type = other DNA
aacagctcagcagacacctgccaa

SEQ ID NO: 463 - DNA, 24 bp, synthetic construct
  misc_feature 1..24: note = Description of Artificial Sequence: Synthetic oligonucleotide
  source 1..24: mol_type = other DNA
tttagctcagctgacacctgccca

SEQ ID NO: 464 - DNA, 24 bp, synthetic construct
  misc_feature 1..24: note = Description of Artificial Sequence: Synthetic oligonucleotide
  source 1..24: mol_type = other DNA
tccagctcagcagacaccagcctc

SEQ ID NO: 465 - DNA, 24 bp, synthetic construct
  misc_feature 1..24: note = Description of Artificial Sequence: Synthetic oligonucleotide
  source 1..24: mol_type = other DNA
ttcccctcagcagacacctgccat

SEQ ID NO: 466 - DNA, 24 bp, synthetic construct
  misc_feature 1..24: note = Description of Artificial Sequence: Synthetic oligonucleotide
  source 1..24: mol_type = other DNA
ttcccctcagcagacacctgccat

SEQ ID NO: 467 - DNA, 24 bp, synthetic construct
  misc_feature 1..24: note = Description of Artificial Sequence: Synthetic oligonucleotide
  source 1..24: mol_type = other DNA
ttcccctcagcagacacctgccat

SEQ ID NO: 468 - DNA, 24 bp, synthetic construct
  misc_feature 1..24: note = Description of Artificial Sequence: Synthetic oligonucleotide
  source 1..24: mol_type = other DNA
ttcccctcagcggacacctgccat

SEQ ID NO: 469 - DNA, 24 bp, synthetic construct
  misc_feature 1..24: note = Description of Artificial Sequence: Synthetic oligonucleotide
  modified_base 4: mod_base = OTHER; note = a, c, t, g, unknown or other
  source 1..24: mol_type = other DNA
tttngattgaaggaaaagttacaa

SEQ ID NO: 470 - DNA, 24 bp, synthetic construct
  misc_feature 1..24: note = Description of Artificial Sequence: Synthetic oligonucleotide
  source 1..24: mol_type = other DNA
tttagattgaaggaaaagttacaa

SEQ ID NO: 471 - DNA, 24 bp, synthetic construct
  misc_feature 1..24: note = Description of Artificial Sequence: Synthetic oligonucleotide
  source 1..24: mol_type = other DNA
tttagattaatggaaaagttacaa

SEQ ID NO: 472 - DNA, 24 bp, synthetic construct
  misc_feature 1..24: note = Description of Artificial Sequence: Synthetic oligonucleotide
  source 1..24: mol_type = other DNA
tttagacttaaagaaaagttacaa

SEQ ID NO: 473 - DNA, 24 bp, synthetic construct
  misc_feature 1..24: note = Description of Artificial Sequence: Synthetic oligonucleotide
  source 1..24: mol_type = other DNA
cttggattaaaggaaaagctacaa

SEQ ID NO: 474 - DNA, 24 bp, synthetic construct
  misc_feature 1..24: note = Description of Artificial Sequence: Synthetic oligonucleotide
  modified_base 4: mod_base = OTHER; note = a, c, t, g, unknown or other
  source 1..24: mol_type = other DNA
tttnggatgccactaaaagggaaa

SEQ ID NO: 475 - DNA, 24 bp, synthetic construct
  misc_feature 1..24: note = Description of Artificial Sequence: Synthetic oligonucleotide
  source 1..24: mol_type = other DNA
tttaggatgccactaaaagggaaa

SEQ ID NO: 476 - DNA, 24 bp, synthetic construct
  misc_feature 1..24: note = Description of Artificial Sequence: Synthetic oligonucleotide
  source 1..24: mol_type = other DNA
tttagaatgccactaaaaaaagag

SEQ ID NO: 477 - DNA, 24 bp, synthetic construct
  misc_feature 1..24: note = Description of Artificial Sequence: Synthetic oligonucleotide
  source 1..24: mol_type = other DNA
ttttgtataccactaaaagggaaa

SEQ ID NO: 478 - DNA, 24 bp, synthetic construct
  misc_feature 1..24: note = Description of Artificial Sequence: Synthetic oligonucleotide
  modified_base 4: mod_base = OTHER; note = a, c, t, g, unknown or other
  source 1..24: mol_type = other DNA
attntgatgagcctttagagagaa

SEQ ID NO: 479 - DNA, 24 bp, synthetic construct
  misc_feature 1..24: note = Description of Artificial Sequence: Synthetic oligonucleotide
  source 1..24: mol_type = other DNA
attctgatgagcctttagagagaa

SEQ ID NO: 480 - DNA, 24 bp, synthetic construct
  misc_feature 1..24: note = Description of Artificial Sequence: Synthetic oligonucleotide
  source 1..24: mol_type = other DNA
tttgtgatgagcgttgagagaaag

SEQ ID NO: 481 - DNA, 24 bp, synthetic construct
  misc_feature 1..24: note = Description of Artificial Sequence: Synthetic oligonucleotide
  source 1..24: mol_type = other DNA
tttttgatgagcctttagagtact

SEQ ID NO: 482 - DNA, 24 bp, synthetic construct
  misc_feature 1..24: note = Description of Artificial Sequence: Synthetic oligonucleotide
  source 1..24: mol_type = other DNA
aatgtgatgacccattagagagaa

SEQ ID NO: 483 - DNA, 24 bp, synthetic construct
  misc_feature 1..24: note = Description of Artificial Sequence: Synthetic oligonucleotide
  source 1..24: mol_type = other DNA
tttatgatgagtctttagagtttt

SEQ ID NO: 484 - DNA, 24 bp, synthetic construct
  misc_feature 1..24: note = Description of Artificial Sequence: Synthetic oligonucleotide
  source 1..24: mol_type = other DNA
tttatgatgtacctttagaaagca

SEQ ID NO: 485 - DNA, 24 bp, synthetic construct
  misc_feature 1..24: note = Description of Artificial Sequence: Synthetic oligonucleotide
  modified_base 4: mod_base = OTHER; note = a, c, t, g, unknown or other
  source 1..24: mol_type = other DNA
attnaccgagcaggagtgagggaa

SEQ ID NO: 486 - DNA, 24 bp, synthetic construct
  misc_feature 1..24: note = Description of Artificial Sequence: Synthetic oligonucleotide
  source 1..24: mol_type = other DNA
attcaccgagcaggagtgagggaa

SEQ ID NO: 487 - DNA, 24 bp, synthetic construct
  misc_feature 1..24: note = Description of Artificial Sequence: Synthetic oligonucleotide
  source 1..24: mol_type = other DNA
tttacttgagcagaagtgagggag

SEQ ID NO: 488 - DNA, 24 bp, synthetic construct
  misc_feature 1..24: note = Description of Artificial Sequence: Synthetic oligonucleotide
  source 1..24: mol_type = other DNA
tttgactgagcaggattgagggaa

SEQ ID NO: 489 - DNA, 24 bp, synthetic construct
  misc_feature 1..24: note = Description of Artificial Sequence: Synthetic oligonucleotide
  source 1..24: mol_type = other DNA
tttcctagagcaggagtgaggata

SEQ ID NO: 490 - DNA, 24 bp, synthetic construct
  misc_feature 1..24: note = Description of Artificial Sequence: Synthetic oligonucleotide
  modified_base 4: mod_base = OTHER; note = a, c, t, g, unknown or other
  source 1..24: mol_type = other DNA
cttnttgggtcagctgttaacatc

SEQ ID NO: 491 - DNA, 24 bp, synthetic construct
  misc_feature 1..24: note = Description of Artificial Sequence: Synthetic oligonucleotide
  source 1..24: mol_type = other DNA
cttattgggtcagctgttaacatc

SEQ ID NO: 492 - DNA, 24 bp, synthetic construct
  misc_feature 1..24: note = Description of Artificial Sequence: Synthetic oligonucleotide
  source 1..24: mol_type = other DNA
cattttgggtcagcacgtgacatt

SEQ ID NO: 493 - DNA, 24 bp, synthetic construct
  misc_feature 1..24: note = Description of Artificial Sequence: Synthetic oligonucleotide
  modified_base 4: mod_base = OTHER; note = a, c, t, g, unknown or other
  source 1..24: mol_type = other DNA
cttnacccaggttcataacaatgt

SEQ ID NO: 494 - DNA, 24 bp, synthetic construct
  misc_feature 1..24: note = Description of Artificial Sequence: Synthetic oligonucleotide
  source 1..24: mol_type = other DNA
cttcacccaggttcataacaatgt

SEQ ID NO: 495 - DNA, 24 bp, synthetic construct
  misc_feature 1..24: note = Description of Artificial Sequence: Synthetic oligonucleotide
  modified_base 4: mod_base = OTHER; note = a, c, t, g, unknown or other
  source 1..24: mol_type = other DNA
gttnatttgtccagaggaaaccac

SEQ ID NO: 496 - DNA, 24 bp, synthetic construct
  misc_feature 1..24: note = Description of Artificial Sequence: Synthetic oligonucleotide
  source 1..24: mol_type = other DNA
gttcatttgtccagaggaaaccac

SEQ ID NO: 497 - DNA, 24 bp, synthetic construct
  misc_feature 1..24: note = Description of Artificial Sequence: Synthetic oligonucleotide
  source 1..24: mol_type = other DNA
ttaattttgtccaaaggaaaccac

SEQ ID NO: 498 - DNA, 24 bp, synthetic construct
  misc_feature 1..24: note = Description of Artificial Sequence: Synthetic oligonucleotide
  source 1..24: mol_type = other DNA
ttccatttgtccacaggaaacctc

SEQ ID NO: 499 - DNA, 24 bp, synthetic construct
  misc_feature 1..24: note = Description of Artificial Sequence: Synthetic oligonucleotide
  source 1..24: mol_type = other DNA
tttcatttgaccaaagaaaaccca

SEQ ID NO: 500 - DNA, 24 bp, synthetic construct
  misc_feature 1..24: note = Description of Artificial Sequence: Synthetic oligonucleotide
  source 1..24: mol_type = other DNA
gccaatttgtcctgaggaaaccac

SEQ ID NO: 501 - DNA, 24 bp, synthetic construct
  misc_feature 1..24: note = Description of Artificial Sequence: Synthetic oligonucleotide
  source 1..24: mol_type = other DNA
cctcatttgtccagaggaaactac

SEQ ID NO: 502 - DNA, 24 bp, synthetic construct
  misc_feature 1..24: note = Description of Artificial Sequence: Synthetic oligonucleotide
  source 1..24: mol_type = other DNA
tttgctttgtacagaggaaaccat

SEQ ID NO: 503 - DNA, 24 bp, synthetic construct
  misc_feature 1..24: note = Description of Artificial Sequence: Synthetic oligonucleotide
  source 1..24: mol_type = other DNA
agtcatctgtcctgaggaaaccac

SEQ ID NO: 504 - DNA, 24 bp, synthetic construct
  misc_feature 1..24: note = Description of Artificial Sequence: Synthetic oligonucleotide
  source 1..24: mol_type = other DNA
attgatttttccagagaaaaccac

SEQ ID NO: 505 - DNA, 24 bp, synthetic construct
  misc_feature 1..24: note = Description of Artificial Sequence: Synthetic oligonucleotide
  source 1..24: mol_type = other DNA
tttcattactccagaagaaaccac

SEQ ID NO: 506 - DNA, 24 bp, synthetic construct
  misc_feature 1..24: note = Description of Artificial Sequence: Synthetic oligonucleotide
  modified_base 4: mod_base = OTHER; note = a, c, t, g, unknown or other
  source 1..24: mol_type = other DNA
gttnccttagcactctgccactta

SEQ ID NO: 507 - DNA, 24 bp, synthetic construct
  misc_feature 1..24: note = Description of Artificial Sequence: Synthetic oligonucleotide
  source 1..24: mol_type = other DNA
gttcccttagcactctgccactta

SEQ ID NO: 508 - DNA, 24 bp, synthetic construct
  misc_feature 1..24: note = Description of Artificial Sequence: Synthetic oligonucleotide
  source 1..24: mol_type = other DNA
ttccccttagccatctgccaccta

SEQ ID NO: 509 - DNA, 24 bp, synthetic construct
  misc_feature 1..24: note = Description of Artificial Sequence: Synthetic oligonucleotide
  source 1..24: mol_type = other DNA
tttgccccagcactctgccactta

SEQ ID NO: 510 - DNA, 24 bp, synthetic construct
  misc_feature 1..24: note = Description of Artificial Sequence: Synthetic oligonucleotide
  modified_base 4: mod_base = OTHER; note = a, c, t, g, unknown or other
  source 1..24: mol_type = other DNA
gttncctgtcttgtttgtgagagg

SEQ ID NO: 511 - DNA, 24 bp, synthetic construct
  misc_feature 1..24: note = Description of Artificial Sequence: Synthetic oligonucleotide
  source 1..24: mol_type = other DNA
gttccctgtcttgtttgtgagagg

SEQ ID NO: 512 - DNA, 24 bp, synthetic construct
  misc_feature 1..24: note = Description of Artificial Sequence: Synthetic oligonucleotide
  source 1..24: mol_type = other DNA
attacctgtcttgtttgggagaga

SEQ ID NO: 513 - DNA, 24 bp, synthetic construct
  misc_feature 1..24: note = Description of Artificial Sequence: Synthetic oligonucleotide
  source 1..24: mol_type = other DNA
tttgcctgtcctgtgtgtgagatg

SEQ ID NO: 514 - DNA, 24 bp, synthetic construct
  misc_feature 1..24: note = Description of Artificial Sequence: Synthetic oligonucleotide
  source 1..24: mol_type = other DNA
tttgcctgtcttgttaatgagaaa

SEQ ID NO: 515 - DNA, 24 bp, synthetic construct
  misc_feature 1..24: note = Description of Artificial Sequence: Synthetic oligonucleotide
  source 1..24: mol_type = other DNA
tttccctgtcttcattgtgagaga

SEQ ID NO: 516 - DNA, 24 bp, synthetic construct
  misc_feature 1..24: note = Description of Artificial Sequence: Synthetic oligonucleotide
  modified_base 4: mod_base = OTHER; note = a, c, t, g, unknown or other
  source 1..24: mol_type = other DNA
tatngcctctccctgctcagaatc

SEQ ID NO: 517 - DNA, 24 bp, synthetic construct
  misc_feature 1..24: note = Description of Artificial Sequence: Synthetic oligonucleotide
  source 1..24: mol_type = other DNA
tatcgcctctccctgctcagaatc

SEQ ID NO: 518 - DNA, 24 bp, synthetic construct
  misc_feature 1..24: note = Description of Artificial Sequence: Synthetic oligonucleotide
  modified_base 4: mod_base = OTHER; note = a, c, t, g, unknown or other
  source 1..24: mol_type = other DNA
tatnaacctgggtgaagtcccaac

SEQ ID NO: 519 - DNA, 24 bp, synthetic construct
  misc_feature 1..24: note = Description of Artificial Sequence: Synthetic oligonucleotide
  source 1..24: mol_type = other DNA
tatgaacctgggtgaagtcccaac

SEQ ID NO: 520 - DNA, 24 bp, synthetic construct
  misc_feature 1..24: note = Description of Artificial Sequence: Synthetic oligonucleotide
  source 1..24: mol_type = other DNA
tttgcacctgggtgaagtcccaaa

SEQ ID NO: 521 - DNA, 24 bp, synthetic construct
  misc_feature 1..24: note = Description of Artificial Sequence: Synthetic oligonucleotide
  modified_base 4: mod_base = OTHER; note = a, c, t, g, unknown or other
  source 1..24: mol_type = other DNA
ttcntgatggtccatgtctgttac

SEQ ID NO: 522 - DNA, 24 bp, synthetic construct
  misc_feature 1..24: note = Description of Artificial Sequence: Synthetic oligonucleotide
  source 1..24: mol_type = other DNA
tttctgatggtccatacctgttac

SEQ ID NO: 523 - DNA, 24 bp, synthetic construct
  misc_feature 1..24: note = Description of Artificial Sequence: Synthetic oligonucleotide
  source 1..24: mol_type = other DNA
ttcctgatggtccatgtctgttac

SEQ ID NO: 524 - DNA, 24 bp, synthetic construct
  misc_feature 1..24: note = Description of Artificial Sequence: Synthetic oligonucleotide
  source 1..24: mol_type = other DNA
ttcctgatggtccatgtctgaatt

SEQ ID NO: 525 - DNA, 24 bp, synthetic construct
  misc_feature 1..24: note = Description of Artificial Sequence: Synthetic oligonucleotide
  source 1..24: mol_type = other DNA
cttctgatggtccatatctgttaa

SEQ ID NO: 526 - DNA, 24 bp, synthetic construct
  misc_feature 1..24: note = Description of Artificial Sequence: Synthetic oligonucleotide
  source 1..24: mol_type = other DNA
ttcctgatggtccacatctgttaa

SEQ ID NO: 527 - DNA, 24 bp, synthetic construct
  misc_feature 1..24: note = Description of Artificial Sequence: Synthetic oligonucleotide
  source 1..24: mol_type = other DNA
ttcctgatggtccacatctgttaa

SEQ ID NO: 528 - DNA, 24 bp, synthetic construct
  misc_feature 1..24: note = Description of Artificial Sequence: Synthetic oligonucleotide
  source 1..24: mol_type = other DNA
ttcctgatggtccatacctgttaa

SEQ ID NO: 529 - DNA, 24 bp, synthetic construct
  misc_feature 1..24: note = Description of Artificial Sequence: Synthetic oligonucleotide
  source 1..24: mol_type = other DNA
tttgtgatgtttcatgtgtcctag

SEQ ID NO: 530 - DNA, 24 bp, synthetic construct
  misc_feature 1..24: note = Description of Artificial Sequence: Synthetic oligonucleotide
  source 1..24: mol_type = other DNA
ttcctgatggtccatatctgtggc

SEQ ID NO: 531 - DNA, 30 bp, synthetic construct
  misc_feature 1..30: note = Description of Artificial Sequence: Synthetic oligonucleotide
  source 1..30: mol_type = other DNA
ctttcttctcccctctgctggatacctctg

SEQ ID NO: 532 - DNA, 30 bp, synthetic construct
  misc_feature 1..30: note = Description of Artificial Sequence: Synthetic oligonucleotide
  source 1..30: mol_type = other DNA
ctttatccgtgttccttgactctgggcaac

SEQ ID NO: 533 - DNA, 30 bp, synthetic construct
  misc_feature 1..30: note = Description of Artificial Sequence: Synthetic oligonucleotide
  source 1..30: mol_type = other DNA
gtttctcatctgtgcccctccctccctggc

SEQ ID NO: 534 - DNA, 30 bp, synthetic construct
  misc_feature 1..30: note = Description of Artificial Sequence: Synthetic oligonucleotide
  source 1..30: mol_type = other DNA
ttttccgagcttctggcggtctcaagcact

SEQ ID NO: 535 - DNA, 30 bp, synthetic construct
  misc_feature 1..30: note = Description of Artificial Sequence: Synthetic oligonucleotide
  source 1..30: mol_type = other DNA
gtttccctcactcctgctcggtgaatttgg

SEQ ID NO: 536 - DNA, 30 bp, synthetic construct
  misc_feature 1..30: note = Description of Artificial Sequence: Synthetic oligonucleotide
  source 1..30: mol_type = other DNA
gtttcagcctcacccctctagccctacatc

SEQ ID NO: 537 - DNA, 30 bp, synthetic construct
  misc_feature 1..30: note = Description of Artificial Sequence: Synthetic oligonucleotide
  source 1..30: mol_type = other DNA
gtttgtggttgcccaccctagtcattggag

SEQ ID NO: 538 - DNA, 30 bp, synthetic construct
  misc_feature 1..30: note = Description of Artificial Sequence: Synthetic oligonucleotide
  source 1..30: mol_type = other DNA
ctttggtcggcatggccccattcgcacggc

SEQ ID NO: 539 - DNA, 23 bp, synthetic construct
  misc_feature 1..23: note = Description of Artificial Sequence: Synthetic oligonucleotide
  source 1..23: mol_type = other DNA
ggaatcccttctgcagcacctgg

SEQ ID NO: 540 - DNA, 23 bp, synthetic construct
  misc_feature 1..23: note = Description of Artificial Sequence: Synthetic oligonucleotide
  source 1..23: mol_type = other DNA
ctgatggtccatgtctgttactc

SEQ ID NO: 541 - protein, 21 aa, Acidaminococcus sp.
SFDKFTTYFSGFYENRKNVFS

SEQ ID NO: 542 - protein, 21 aa, Lachnospiraceae bacterium
SFNGFTTAFTGFFDNRENMFS

SEQ ID NO: 543 - protein, 21 aa, Francisella tularensis
SFKGWTTYFKGFHENRKNVYS

SEQ ID NO: 544 - protein, 21 aa, Moraxella bovoculi
HFEKFSTYFTGFHDNRKNMYS

SEQ ID NO: 545 - protein, 21 aa, Thiomicrospira sp.
TFNNFTTYFTGFHENRKNIYS

SEQ ID NO: 546 - protein, 21 aa, Moraxella bovoculi
HFEKFSTYFTGFHDNRKNMYS

SEQ ID NO: 547 - protein, 22 aa, Acidaminococcus sp.
NFQMPTLASGWDVNKEKNNGAI

SEQ ID NO: 548 - protein, 22 aa, Lachnospiraceae bacterium
YFQNPQFMGGWDKDKETDYRAT

SEQ ID NO: 549 - protein, 22 aa, Francisella tularensis
NFENSTLANGWDKNKEPDNTAI

SEQ ID NO: 550 - protein, 22 aa, Moraxella bovoculi
NFGNPTLLNGWDLNKEKDNFGV

SEQ ID NO: 551 - protein, 22 aa, Thiomicrospira sp.
NFDNNTLLSGWDANKETANASI

SEQ ID NO: 552 - protein, 22 aa, Moraxella bovoculi
NFGNPTLLNGWDLNKEKDNFGV

SEQ ID NO: 553 - DNA, 24 bp, Acidaminococcus sp.
  source 1..24: mol_type = other DNA
tttccctcactcctgctcggtgaa

SEQ ID NO: 554 - DNA, 20 bp, Acidaminococcus sp.
  source 1..20: mol_type = other DNA
cctcactcctgctcggtgaa

SEQ ID NO: 555 - DNA, 20 bp, synthetic construct
  misc_feature 1..20: note = Description of Artificial Sequence: Synthetic oligonucleotide
  source 1..20: mol_type = other DNA
cctcactgctgctcggtgaa

SEQ ID NO: 556 - DNA, 20 bp, synthetic construct
  misc_feature 1..20: note = Description of Artificial Sequence: Synthetic oligonucleotide
  source 1..20: mol_type = other DNA
cctcactcgtgctcggtgaa

SEQ ID NO: 557 - DNA, 24 bp, Acidaminococcus sp.
  source 1..24: mol_type = other DNA
tttcctgatggtccatgtctgtta

SEQ ID NO: 558 - DNA, 20 bp, Acidaminococcus sp.
  source 1..20: mol_type = other DNA
ctgatggtccatgtctgtta

SEQ ID NO: 559 - DNA, 20 bp, synthetic construct
  misc_feature 1..20: note = Description of Artificial Sequence: Synthetic oligonucleotide
  source 1..20: mol_type = other DNA
ctgatggaccatgtctgtta

SEQ ID NO: 560 - DNA, 20 bp, synthetic construct
  misc_feature 1..20: note = Description of Artificial Sequence: Synthetic oligonucleotide
  source 1..20: mol_type = other DNA
ctgatggtgcatgtctgtta

SEQ ID NO: 561 - protein, 6 aa, Lachnospiraceae bacterium
MSKLEK

SEQ ID NO: 562 - protein, 6 aa, synthetic construct
  REGION 1..6: note = Description of Artificial Sequence: Synthetic 6xHis tag
HHHHHH

SEQ ID NO: 563 - protein, 7 aa, Acidaminococcus sp.
GLFKAEL

SEQ ID NO: 564 - protein, 21 aa, Acidaminococcus sp.
SFDKFTTYFSGFYENRKNVFS

SEQ ID NO: 565 - protein, 22 aa, Acidaminococcus sp.
NFQMPTLASGWDVNKEKNNGAI

SEQ ID NO: 566 - protein, 22 aa, Acidaminococcus sp.
YDYFPDAAKMIPKCSTQLKAVT

SEQ ID NO: 567 - protein, 5 aa, Acidaminococcus sp.
LSNNF

SEQ ID NO: 568 - protein, 9 aa, Acidaminococcus sp.
SKYTKTTSI

SEQ ID NO: 569 - protein, 7 aa, Lachnospiraceae bacterium
SLFKKDI

SEQ ID NO: 570 - protein, 21 aa, Lachnospiraceae bacterium
SFNGFTTAFTGFFDNRENMFS

SEQ ID NO: 571 - protein, 22 aa, Lachnospiraceae bacterium
YFQNPQFMGGWDKDKETDYRAT

SEQ ID NO: 572 - protein, 22 aa, Lachnospiraceae bacterium
YKLLPGPNKMLPKVFFSKKWMA

SEQ ID NO: 573 - protein, 5 aa, Lachnospiraceae bacterium
FSKKW

SEQ ID NO: 574 - protein, 9 aa, Lachnospiraceae bacterium
SRYPKWSNA

SEQ ID NO: 575 - protein, 7 aa, Lachnospiraceae bacterium
SLFKKDI

SEQ ID NO: 576 - protein, 21 aa, Lachnospiraceae bacterium
SFNGFTTAFTGFFDNRENMFS

SEQ ID NO: 577 - protein, 22 aa, Lachnospiraceae bacterium
YFQNPQFMGGWDKDKETDYRAT

SEQ ID NO: 578 - protein, 22 aa, Lachnospiraceae bacterium
YKLLPGPNKMLPKVFFSKKWMA

SEQ ID NO: 579 - protein, 5 aa, Lachnospiraceae bacterium
FSKKW

SEQ ID NO: 580 - protein, 9 aa, Lachnospiraceae bacterium
SRYPKWSNA

SEQ ID NO: 581 - protein, 6 aa, Francisella tularensis
LKQSKD

SEQ ID NO: 582 - protein, 21 aa, Francisella tularensis
SFKGWTTYFKGFHENRKNVYS

SEQ ID NO: 583 - protein, 22 aa, Francisella tularensis
NFENSTLANGWDKNKEPDNTAI

SEQ ID NO: 584 - protein, 22 aa, Francisella tularensis
YKLLPGANKMLPKVFFSAKSIK

SEQ ID NO: 585 - protein, 5 aa, Francisella tularensis
RIRNH

SEQ ID NO: 586 - protein, 9 aa, Francisella tularensis
SKHPEWKDF